European Patent Specification EP 3 667 323 B1, published November 13, 2024. Title: METHODS, COMPOSITIONS AND DEVICES FOR TREATING CANCER WITH ILLUDOFULVENES. Applicant: Kelner, Michael J. The sequence listing filed with the application follows.

SEQUENCE LISTING (926 sequences)

SEQ ID NO: 1 - DNA, 1962 bp, Homo sapiens
gctgttccagtcccgcccctgagctctgtcatggcgacgtccagtgctccagccggtgtgaggacacgatatgctggggtttttgtccgcacgccaaacgggtttggaggaccctcttcgccttcggagagcagagtcaacacggagagttttgggactggaattaaataaagacagagatgttgaaagaatccacggcggtggaattaacacccttgacattgaacctgttgaagggagatacatgttatcaggtggttcagatggtgtgattgtactttatgaccttgagaactccagcagacaatcttattacacatgtaaagcagtgtgttccattggcagagatcatcctgatgttcacagatacagtgtggagactgtacagtggtatcctcatgacactggcatgttcacatcaagctcatttgataaaactctgaaagtatgggatacaaatacattacaattggtactagaggacccaaagtacaactttgtgacttgaagtctggatcctgttctcacattctacagggtcacagacaagaaatattagcagtttcctggtctccacgttatgactatatcttggcaacagcaagtgctgacagtagagtaaaattatgggatgtgagaagagcatcaggatgtttgattactcttgatcaacataatgggaaaaagtcacaagctgttgaatcagcaaacactgctcataatgggaaagttaatggcttatgttttacaagtgatggacttcacctcctcactgttggtacagataatcgaatgaggctctggaatagttccaatggagaaaacacacttgtgaactatggaaaagtttgtaataacagtaaaaaaggattgaaattcactgtctcctgtggctgcagttcagaatttgtttttgtaccatatggtagcaccattgctgtttatacagtttactcaggagaacagataactatgcttaagggacattataaaactgttgactgctgtgtatttcagtcaaatttccaggaactttatagtggtagcagagactgcaacattctggcttgggttccatccttatatgaaccagttcctgatgatgatgagactacaacaaaatcacaattaaatccggcctttgaagatgcctggagcagcagtgatgaagaaggatgaatatcatctttagtacctttttgtctctgctgaaactttttaaatgagactgtgtttttttcaactgtatggtctattcctgacagctaaattagccctaaatgtgggtaatatttttcctcatgttttaaaatgaggttaatatttgcataaaatcctaaaacagacttctgtatagtttatttagtcaaaatgtgttccttgatcccagatgttgtggcctgggaaagccctcattgctacagtacaagtaacacaagtcgttgtacctcagttgtgaccttcagcagattttatgaactataagatgcagtctcagaggatcagcaagtggaggccatcagtattgactttctcttacttgctgtactatcagcctgctcgtttccacctttaagaatgattttgccaagaatgattatatcaaaaatagtagttgaaatggtaacatcaaaattattttattctttcttcttcatgtattcacatttttcagtggtttcatttaattaaccatgctttatgttaaacattttggggctcaatgtctcctactatccaaaatgtgcatcacaggaggcttttaactttgtgaaaatcccatgtttgctttattttattttaatgtcagaaggcagtttgcgctaatgcttgaactctttttctgtgaaactcattaaggtatgaccaaatcctgcctcattaattcaagcagaaaatatcctggcagggaatctggcttaaacatgaaatgctgtaataaaatttctatgttattgtctc

SEQ ID NO: 2 - protein, 396 aa, Homo sapiens
MLGFLSARQTGLEDPLRLRRAESTRRVLGLELNKDRDVERIHGGGINTLDIEPVEGRYMLSGGSDGVIVLYDLENSSRQSYYTCKAVCSIGRDHPDVHRYSVETVQWYPHDTGMFTSSSFDKTLKVWDTNTLQTADVFNFEETVYSHHMSPVSTKHCLVAVGTRGPKVQLCDLKSGSCSHILQGHRQEILAVSWSPRYDYILATASADSRVKLWDVRRASGCLITLDQHNGKKSQAVESANTAHNGKVNGLCFTSDGLHLLTVGTDNRMRLWNSSNGENTLVNYGKVCNNSKKGLKFTVSCGCSSEFVFVPYGSTIAVYTVYSGEQITMLKGHYKTVDCCVFQSNFQELYSGSRDCNILAWVPSLYEPVPDDDETTTKSQLNPAFEDAWSSSDEEG

SEQ ID NO: 3 - DNA, 3590 bp, Homo sapiens
gcgccacgggcctccccgcaccagcagaagtcggagtcgctgttgggggcggtgtctatggttgagctgagggcgcaggcgccacggcccgtcgagctgggttccaaggcggctggcggcggtagcgtctctgtttccttgtgggcgctcgcgcggccctgggtagtctgtagagaatgccaaatgagggaatcccccactcaagtcaaactcaggagcaagactgtttacagagtcaacctgtcagtaataatgaagaaatggcaatcaagcaagaaagtggtggtgatggggaggtggaggagtacctctcctttcgttctgtgggtgacgggctgtccacctctgctgtggggtgcgcatcagcagctccgaggagagggccagccctgctgcacatcgaccgacatcagatccaggcagtagagcctagcgcccaggcccttgagctgcagggtttgggtgtggacgtctatgaccaggacgtgctggaacagggagtgcttcagcaggtggacaatgccatccatgaggccagccgtgcctcccagctcgttgacgtggagaaggagtatcggtcggtcctggatgacctcacgtcatgtacgacatccctaaggcaaatcaataaaattattgaacagcttagccctcaagctgccaccagcagagacatcaacaggaaactagattctgtaaaacgacagaagtataataaggaacaacagctaaaaaagatcactgcaaaacaaaagcatctccaggccatccttggaggagcagaggtgaaaattgaactagatcacgccagtctggaggaggatgcagagccggggccatccagtcttggcagcatgctcatgcctgtccaggagactgcctgggaagagctcatccgcactggccagatgacaccttttggtacccagatccctcagaaacaggagaaaaagcccagaaaaatcatgcttaatgaagcatcaggcttcgaaaagtatttggcagatcaagcaaaactgtcttttgaaaggaagaagcaaggttgtaataaaagagcagctagaaaagctccagccccagtcacgcctccagccccagtgcaaaataaaaacaaaccaaacaagaaagccagagttctgtccaaaaaagaggagcgtttgaaaaagcacatcaagaaactccagaagagggctttgcagttccaggggaaagtgggattgccaaaggcaaggagaccttgggagtcagacatgaggccagaggcagagggagactctgagggtgaagagtctgagtatttccccacagaggaggaggaagaggaggaagatgacgaggtggagggggcagaggcggacctgtctggagatggtactgactatgagctgaagcctctgcccaagggcgggaaacggcagaagaaagtgccagtgcaggagattgatgatgactttttcccaagttctggggaagaagctgaagctgcttctgtaggagaaggaggaggaggaggtcggaaagtgggaagataccgagatgatggagatgaagattattataagcagcggttaagtcccaagatgcctcgaacactaagtttacatgaaataactgaccttttagagacagatgacagcatagaagcaagtgctatagtgatacaaccacctgaaaatgctacagcacctgtttctgatgaggaatcaggagatgaagaaggtggaacaataaataatctgccaggttctttgttgcacacagctgcgtatcttattcaagatggctctgatgctgagtctgactcagatgatccctcatacgcacctaaagatgactctcctgatgaagttccatctacgtttactgtgcagcaacctccaccatcaaggaggaggaaaatgacaaaaattctttgcaaatggaaaaaagccgacctaactgtacaacccgtagcaggtagagttacagcaccaccaaacgatttcttcaccgtaatgagaactcccacagaaattcttgaactttttcttgatgacgaggtcattgaactcattgtcaagtactccaacttatatgcttgcagtaaaggtgtacatcttggcttgactagctctgaattcaaatgttttctgggaattatttttctgagtggttatgtctcagttcctagaaggcgtatgttttgggaacaaagaacagatgtgcataatgtactggttagtgctgccatgagacgtgaccggtttgaaactatattttctaatttgcatgttgctgacaatgcaaatttggatccagtggacaaattttccaaattgcgacctctcataagcaaacttaatgagagatgcatgaaatttgttccaaatgaaacatatttcagctttgatgaattcatggttccttattttggtcgtcacgggtgcaaacaatttattcggggaaagcccattcggtttggctataagttttggtgtggtgccacctgtctgggctacatttgctggtttcagccgtatcagggtaaaaacccaaatactaaacatgaggaatatggtgtcggtgcgtcacttgtccttcagtttagtgaggcacttacagaggcacaccctggacaataccattttgtattcaataactttttcaccagtattgcacttcttgataagctcagttcaatgggacatcaggcaacaggtacagtgagaaaggatcacattgacagagttccactggaatcagatgtagctttaaagaaaaaagaaagaggcacatttgattatcgaattgatggcaaaggcaatattgtctgcagatggaatgataacagtgttgtcactgttgcctcatctggtgctggtatccatcccctgtgtcttgtcagtcgttactcccagaaactgaaaaagaagatacaagttcagcagccaaacatgatcaaagtgtataaccagttcatgggaggcgtagacagagctgatgaaaacattgataagtatcgggcatcaatccgtggaaagaaatggtattcaagccctcttttgttctgtttcgaactggtcttacaaaatgcttggcaattgcataaaacatatgatgagaaaccagtggattttctggagtttcgtcgacgtgtggtatgccattatctggagacccatggtcatcctccagaacctggccaaaaaggaagacctcagaagcgtaacattgactcacgttatgatggcataaatcatgtgatagtcaaacagggaaagcaaacgcgatgcgctgaatgtcataagaacacaacttttcgatgtgaaaaatgtgatgttgccttacatgtgaagtgttccgttgaatatcacactgaatagcaggtgtcaccacctcctgagataagaaacatagttttatacattatgtacagtgtagcagtggttttgcctagtgttccaattttggaacgtcacataacaatggaacataataaatttttttttctcttcaaatttttgttccttgaatttttctaggtaacatatatgaatttcatgcaaaaattcaaaaaattgtaacctcagacataaatgggttaaagatgt

SEQ ID NO: 4 - protein, 1493 aa, Homo sapiens
MPNEGIPHSSQTQEQDCLQSQPVSNNEEMAIKQESGGDGEVEEYLSFRSVGDGLSTSAVGCASAAPRRGPALLHIDRHQIQAVEPSAQALELQGLGVDVYDQDVLEQGVLQQVDNAIHEASRASQLVDVEKEYRSVLDDLTSCTTSLRQINKIIEQLSPQAATSRDINRKLDSVKRQKYNKEQQLKKITAKQKHLQAILGGAEVKIELDHASLEEDAEPGPSSLGSMLMPVQETAWEELIRTGQMTPFGTQIPQKQEKKPRKIMLNEASGFEKYLADQAKLSFERKKQGCNKRAARKAPAPVTPPAPVQNKNKPNKKARVLSKKEERLKKHIKKLQKRALQFQGKVGLPKARRPWESDMRPEAEGDSEGEESEYFPTEEEEEEEDDEVEGAEADLSGDGTDYELKPLPKGGKRQKKVPVQEIDDDFFPSSGEEAEAASVGEGGGGGRKVGRYRDDGDEDYYKQRLRRWNKLRLQDKEKRLKLEDDSEESDAEFDEGFKVPGFLFKKLFKYQQTGVRWLWELHCQQAGGILGDEMGLGKTIQIIAFLAGLSYSKIRTRGSNYRFEGLGPTVIVCPTTVMHQWVKEFHTWWPPFRVAILHETGSYTHKKEKLIRDVAHCHGILITSYSYIRLMQDDISRYDWHYVILDEGHKIRNPNAAVTLACKQFRTPHRIILSGSPMQNNLRELWSLFDFIFPGKLGTLPVFMEQFSVPITMGGYSNASPVQVKTAYKCACVLRDTINPYLLRRMKSDVKMSLSLPDKNEQVLFCRLTDEQHKVYQNFVDSKEVYRILNGEMQIFSGLIALRKICNHPDLFSGGPKNLKGLPDDELEEDQFGYWKRSGKMIVVESLLKIWHKQGQRVLLFSQSRQMLDILEVFLRAQKYTYLKMDGTTTIASRQPLITRYNEDTSIFVFLLTTRVGGLGVNLTGANRVVIYDPDWNPSTDTQARERAWRIGQKKQVTVYRLLTAGTIEEKIYHRQIFKQFLTNRVLKDPKQRRFFKSNDLYELFTLTSPDASQSTETSAIFAGTGSDVQTPKCHLKRRIQPAFGADHDVPKRKKFPASNISVNDATSSEEKSEAKGAEVNAVTSNRSDPLKDDPHMSSNVTSNDRLGEETNAVSGPEELSVISGNGECSNSSGTGKTSMPSGDESIDEKLGLSYKRERPSQAQTEAFWENKQMENNFYKHKSKTKHHSVAEEETLEKHLRPKQKPKNSKHCRDAKFEGTRIPHLVKKRRYQKQDSENKSEAKEQSNDDYVLEKLFKKSVGVHSVMKHDAIMDGASPDYVLVEAEANRVAQDALKALRLSRQRCLGAVSGVPTWTGHRGISGAPAGKKSRFGKKRNSNFSVQHPSSTSPTEKCQDGIMKKEGKDNVPEHFSGRAEDADSSSGPLASSSLLAKMRARNHLILPERLESESGHLQEASALLPTTEHDDLLVEMRNFIAFQAHTDGQASTREILQEFESKLSASQSCVFRELLRNLCTFHRTSGGEGIWKLKPEYC

SEQ ID NO: 5 - DNA, 3515 bp, Homo sapiens
ctccttccgcgtggtccctccccctcaggccgcggtcgcgattacgctctctacggcctgcgaccgcagggccgttgcgggctggagacacggcgccgactggaaccggaggagctctaggccaaatggttgggccagccaggatcccaggacccttcgccgctcgagaccggagagaggaaacgaaacaggcgggaacccgtgggggagggagggaactagcggaaggtgtcatggcggccgcgctcttgagtcacgtgcccagggcccgccttgctacttccggtcacgtgccctcagactcctcgcagccagcgatggaggcgagaccccctagtaacagaggcggtggctactgctgcggccactgggtttcggcctcttcccagcagcggctctaagaagcgcagcggaactcgaccggatccaacccagttagttacttcctgtctagagttgtagcttccacctgagttctcctgggaagaagtgtttgccactcaaggaatacactcaagaaaaacctggaaatcacagaaggcattgtaagatagctacagtgattctgttaaacctcctgaaattggtccttgaacaattaagaggtgctacagatgaccaggaaaatttaccaggcaaattagctgtgagacaattgaccatttgtgcccaatgttcgcaccttctagccaccatggcaacctcatctgaagaagttttgctgattgtaaagaaagtgcgtcaaaagaagcaggatggagctctgtacctcatggcagaaagaattgcttgggcacctgaaggcaaagatagatttacaatcagccatatgtatgcagatattaaatgccagaaaattagtccagaaggaaaagctaaaattcagcttcagctggtcctacatgcaggggacacaactaacttccatttttccaatgaaagcacagcagtgaaagagcgagatgcagtaaaagaccttcttcagcagctgctgcccaaattcaagaggaaagcaaataaagaactggaagagaagaacagaatgctgcaagaagatcctgttttgtttcagctttataaagaccttgttgtgagtcaagtgatcagtgctgaggaattctgggccaatcgtttaaatgtgaatgcaacagatagttcttccacatccaatcataagcaggatgttggcatttctgctgcatttctggctgatgtccggccccaaactgatggctgtaacggtctaagatataatttaacttctgatatcattgagtccatatttaggacctatccagcagtaaaaatgaaatatgcagaaaatgttccccacaacatgacagagaaggaattctggacacgttttttccagtcccattattttcacagggatcggctgaatacagggtcaaaggatctctttgcagaatgtgccaaaatagatgaaaaaggcctaaaaacaatggtttcattaggagtgaaaaacccactactagatttaacagctttggaagataaaccattagatgagggctatggcatttcctctgtgccatctgcttccaattctaaatccataaaagagaatagtaatgctgccatcatcaagagatttaaccatcacagtgccatggtcctggcagctggactcagaaaacaagaagcacaaaatgaacaaactagtgagcccagcaacatggatggaaattccggagatgcagactgctttcagccagcagtcaaaagggcgaaattacaagagtccattgaatatgaagacttggggaaaaataattctgtaaaaacgattgcactaaacctcaagaagtcagataggtattatcatggtccaactccaatccagtcactacagtatgcaacaagtcaggacattattaattcttttcaaagtattagacaagaaatggaagcttatacacccaagttaactcaggttctctcaagtagtgctgccagtagtaccatcacagcactgtcacctggaggggcacttatgcagggaggaacacagcaagccataaaccagatggtgccaaatgatattcaatctgaattgaaacacttatatgtagctgttggagaacttctacgacatttctggtcctgctttcctgttaatacgccattcctagaagaaaaggtagtgaaaatgaaaagtaatttggaacgattccaagttacgaagctctgtccattccaagaaaagattcggagacagtatttaagcacaaatttggtaagtcacatagaagagatgctccagacagcctacaacaagctccacacatggcagtcacggcgtctgatgaagaaaacgtgaggtggccatgatgcttacaggttttgtgagattgagagaactatgacctgcagcaactctggaaacctggcctgacagacaagcagatgacctcacaggagtgataagaaacatctgctccacgccaactcccagagctgatgctattgtacttgcacattggagactgaaaggaaagaagggactaaatgctggggaggtaaattaagacagaaccaaatgagctaagttgcaaatatatatatatacacacacacacatatatgtacatgtgtatgtacatatatattttaaaagactgtttactgcagttgctcaggaactgcttttgattcacattaagctgctttcagaaattaaaaaaacactttttaaagggtgcattgataaaatctgaggttttttggttgtcgtttttttctgtgtacatttttttcctaagtttatggcacagggtagaccttaagtattcctcctccatccttcattcttcaccctccattggatcctcaagttttaatgaattccaattataccttacatcagcaagttaaaaaaagtactttaaaataaagcaaagggagactgttgctcaaccatcaggaaacagttgtcagaagacatcattggttctgtgtttcctacggaaataagaaacgataaatattgcactgaatgtttgtggtttggagtccctgaataataaagagggaatatatttgcagaaagtcgcatagggttttttaatgcagaattttgtcagaagacaatggcgctgcatgtttttctttgagtgcaaatgtacattgctaagatttttttaagatggcatgtgctttgaaaagaagatattgcatttttaagagtttaaaaatcttatgagtgagaaatattaaaaaaatcttattttcacctctttagaagaaataaaagatgtttctcctatctccttttctctagtatttgactgttactgtccttggcgaatcgataatcattgcatagtgactgaaaagcctaagtgcaaaaaaaaaaaaaaaagatgttcttgtttctgaacttcgtgccatattttgttcctgatgggatcaacttaatgtttaagactttagatgtcttgtattaaaaattacacaaaaaaagtaaaactttttatacttacccttttaactct

SEQ ID NO: 6 - protein, 548 aa, Homo sapiens
MATSSEEVLLIVKKVRQKKQDGALYLMAERIAWAPEGKDRFTISHMYADIKCQKISPEGKAKIQLQLVLHAGDTTNFHFSNESTAVKERDAVKDLLQQLLPKFKRKANKELEEKNRMLQEDPVLFQLYKDLVVSQVISAEEFWANRLNVNATDSSSTSNHKQDVGISAAFLADVRPQTDGCNGLRYNLTSDIIESIFRTYPAVKMKYAENVPHNMTEKEFWTRFFQSHYFHRDRLNTGSKDLFAECAKIDEKGLKTMVSLGVKNPLLDLTALEDKPLDEGYGISSVPSASNSKSIKENSNAAIIKRFNHHSAMVLAAGLRKQEAQNEQTSEPSNMDGNSGDADCFQPAVKRAKLQESIEYEDLGKNNSVKTIALNLKKSDRYYHGPTPIQSLQYATSQDIINSFQSIRQEMEAYTPKLTQVLSSSAASSTITALSPGGALMQGGTQQAINQMVPNDIQSELKHLYVAVGELLRHFWSCFPVNTPFLEEKVVKMKSNLERFQVTKLCPFQEKIRRQYLSTNLVSHIEEMLQTAYNKLHTWQSRRLMKKT

SEQ ID NO: 7 - DNA, 1951 bp, Homo sapiens
ccttctagcggcgccggtgagtccgcgtgtggaagtctgtgaggcgcagaggtggggcaggccgtctggctagctaggcggctgggagcgttttcgtggcggggaacggaggttgaattgccctgcctgggctcatagggaaggaggatgtgaaggagcttgtgaaggcagaggaagattattgaataataaaatacagttttgaaaaaaatggatgaagaacctgaaagaactaagcgatgggaaggaggctatgaaagaacatgggagattcttaaagaagatgaatctggatcacttaaagctacaatagaagacattctattcaaggcaaagagaaaaagagtatttgagcaccatggacaagttcgacttggaatgatgcgccacctttatgtggtagtagatggatcaagaacaatggaagaccaagatttaaagcctaatagactgacgtgtactttaaagttgttggaatactttgtagaggaatattttgatcaaaatcctattagtcagattggaataattgtaactaagagtaaaagagctgaaaaattgactgaactttcaggaaacccaagaaaacatataacgtctttgaagaaagctgtggatatgacctgccatggagagccatctctttataattccctaagcatagctatgcagactctaaaacacatgcctggacatacaagtcgagaagtactaatcatctttagcagccttacaacttgcgatccatctaatatttatgatctaatcaagaccctaaaggcagctaaaattagagtatctgttattggattgtctgcagaagttcgcgtttgcactgtacttgctcgtgaaactggtggcacgtaccatgttattttagatgaaagccattacaaagagttgctcacacatcatgttagtcctcctcctgctagctcaagttctgaatgctcacttattcgtatgggatttcctcagcacaccattgcttctttatctgaccaggatgcaaaaccctctttcagcatggcgcatttggatggcaatactgagccagggcttacattaggaggctatttctgcccacagtgtcgggcaaagtactgtgagctacctgttgagtgtaaaatctgtggtcttactttggtgtctgctccccacttggcacggtcttaccatcatttgtttcctttggatgcttttcaagaaattcccctagaagaatataatggagaaagattttgttatggatgtcagggggaattgaaagaccaacatgtttatgtttgtgctgtgtgccaaaatgttttctgtgtggactgtgatgtttttgttcatgattctctacactgttgccctggctgtattcataagattccagctccttcaggtgtttgattccagcatgtagtatacattgtatgtgttaaaaagaaatttgcaactgtgaataaaaggacttctttagaagaagcttcatttaaaacatgaaaggataatctgacttaagaaactttttgctaagaaaaggtaatattttattaaattttaaatttgtgttgtcacagaaatacctgaaattcagtagtacttcattcaattaattttgttttctattattttgagttatactgttttcaaagtcattatgcagtatgtataaacttataagaattaaattgatgtgataattttatgtttttataattaaatatagaatctttatgatttatgttaattcattaatttagtgtaagaagaaagttaagtctgaatgtaaattcagtgtaagatgaaaatttatcaatacttatgaaattaggctgggcgctgtggctcacacctgtaatcccaacactttgggaggctgaggtgggcagatcacctgaggtcaggagttcgagaccagcctggccaacatggtgaaaccccgtcactactaaaaatacaa

SEQ ID NO: 8 - protein, 395 aa, Homo sapiens
MDEEPERTKRWEGGYERTWEILKEDESGSLKATIEDILFKAKRKRVFEHHGQVRLGMMRHLYVVVDGSRTMEDQDLKPNRLTCTLKLLEYFVEEYFDQNPISQIGIIVTKSKRAEKLTELSGNPRKHITSLKKAVDMTCHGEPSLYNSLSIAMQTLKHMPGHTSREVLIIFSSLTTCDPSNIYDLIKTLKAAKIRVSVIGLSAEVRVCTVLARETGGTYHVILDESHYKELLTHHVSPPPASSSSECSLIRMGFPQHTIASLSDQDAKPSFSMAHLDGNTEPGLTLGGYFCPQCRAKYCELPVECKICGLTLVSAPHLARSYHHLFPLDAFQEIPLEEYNGERFCYGCQGELKDQHVYVCAVCQNVFCVDCDVFVHDSLHCCPGCIHKIPAPSGV

SEQ ID NO: 9 - DNA, 3434 bp, Homo sapiens
gggggctggcacgagtcacagcacctcgtgcgtcacttggcggcgccggacgttgggctgcgcaggatttgagacgctcccctgaccaccacttgctctgcgctgaggtgctgggacagccatggtttcagacgaagatgaattgaatcttctggttattgtagttgatgccaacccaatttggtggggaaagcaagcattaaaggaatctcagttcactttatccaaatgcatagatgccgtgatggtgctgggaaattcgcatttattcatgaatcgttccaacaaacttgctgtgatagcaagtcacattcaagaaagccgattcttatatcctggaaagaatggcagacttggagacttcttcggagaccctggcaaccctcctgaatttaatccctctgggagtaaagatggaaaatacgaacttttaacctcagcaaatgaagttattgttgaagagattaaagatctaatgaccaaaagtgacataaagggtcaacatacagaaactttgctggcaggatccctggccaaagccctttgctacattcatagaatgaacaaggaagttaaagacaatcaggaaatgaaatcaaggatattggtgattaaggctgcagaagacagtgcgttgcagtatatgaacttcatgaatgtcatctttgcagcacagaaacagaatattttgattgatgcctgtgttttagactccgactcagggctcctccaacaggcttgtgacatcacgggaggactgtacctgaaggtgcctcagatgccttctcttctgcagtatttgctgtgggtgtttcttcccgatcaagatcagagatctcagttaatcctcccacccccagttcatgttgactacagggctgcttgcttctgtcatcgaaatctcattgaaattggttatgtctgttctgtgtgtttgtcaatattctgcaatttcagccccatttgtactacgtgcgagacagcctttaaaatttctctgcctccagtgctgaaagccaagaaaaagaaactgaaagtgtctgcctgaggataaaatattttccccatcttttagagctgttaatagaaattatatagcagattctttgttgggaagactgaaaaaaataaagataggtataggataatttttaatatggtgaccttacagaaaatatttcccaaacatccttttcatcctgtgcttctggaggactgatttgtttgagggaatcattctatgcattatatcctaaaatattctatgactggtttctgtccatgtttgtggctttcatttttttaatgggatgactattagtcaaagtcagcttgtcatgactcatcataggctttctaacctactccctgaatccgggtcctcattgtgaaatgcatgccatacgaaatttgaacgtagctttggaaaaagggactatttgtggagtaatggcattaatcaacatagaacatcttatttgaatcaacagttaacttcagtagtcatgtgaataaaattcttattgtctaaattgagacagcctcagatatttgcagatatttactttttgtctgatatcagtacatatttggacaaagtcatctaaataatagtttgtcaccaaataactacaaaatctcattttaaatgagtaaggagaacgtgtacagaagcaaattttcttcaaaatagttgtgggaagagcttatatgtgaaagcttatgactggttttgagggagaacttactggagaaaatggactctatgttaagtatggttttcagatagaattctttccttttttaatgaggaaaaaaaatccacattaatattgaaactgcacctgtaatcccagcactttgggaggctgaggacagaggattgcttgagcccaggagttcgagagcagcctgggcagcaaagtgagaccccatctctactaaaaatttaaatgtatttattaaaactgttctctagaagctttggactgaatcccaaaagtgtttataagttcaaaagcaaaagtatttgtaatttcaacaacaaaaaatgtatttctttatgtaatcttgaaattattaaaagtccttttagcttctagcacatatttgtacaaagagtttaaggaatggtggctggtttggtttgttttttaaaaatgtttactgacgaggccgggcgtggtggctcacccctgcaatcccagcactttgggaggccgaggcaggcagatcacaaggtcaggagttcaagatcagcctggccagtatggtgaaaccctgtctctactaaaaatagaaaaattagccatgcgaagtagcaggtgcctgtagttccagctactcgggaggctgaggcaagagaattgcttgaatccaggaggcagaggttgcagtgagccaagatagcgcctctgtactccagcctgggtgacagagcgagactctgtatcaaaaaaaaaaaagatcgggcacgttggctcacgcctgtaatcccagcactttgggaggccaaggtgggtggatcacgaggtcaggagtgatcaggctgggtttctgttttgttttgttttgtgagacagagtctcgctctgttgcccaggctggggtgcagtggtgcaagctcggctctctgcaagctctgtctcctgggttcacgccattctcctgcctcagcctcccaagtagctgggattactactctactgaacccatgaggcagaaatttgagaccatcctgcccaacgtggtgaaaacatggtgaaaccctgtctctactaaaaatacaaaaattagctgggcgtggtggcaggtgcctgtaatcccagctactcaggagactgaggcaggagaattgcttgaacccaggaggtggaggttgcagtgagccaagatcaagattgcgccattgcactccagcctgggcgacaagaacaaaactctgtctcaaaaaaaaaaaaaaaaaaaaagtctgtactgataaaacccattgtgtacaaaactttgtatgtaaggaagattttaattttctctttatacaagctgagtcatatttaaataatttgatgttggcttagataatttcagatagattttatattctggatttgtgtttttgttaacaaatatacaaagactttggtgatcactttgcaaatatttgttaatccttgagtttgagaacctgtcttttaaaaataatattttgtatactaattaagtgtaatggaaatcacaattttaagtctaggaaataaagtattatatatactttcaaacaagctagcaaggcttttattattacttttttatttgaaatatcttatatatttggttagttctgtttaacttgtttttaactgttgcccttatgagttattttatataaatttttacaataaaataatttgattttcaaaaaaaaaaaaaaaaaa

SEQ ID NO: 10 - protein, 308 aa, Homo sapiens
MVSDEDELNLLVIVVDANPIWWGKQALKESQFTLSKCIDAVMVLGNSHLFMNRSNKLAVIASHIQESRFLYPGKNGRLGDFFGDPGNPPEFNPSGSKDGKYELLTSANEVIVEEIKDLMTKSDIKGQHTETLLAGSLAKALCYIHRMNKEVKDNQEMKSRILVIKAAEDSALQYMNFMNVIFAAQKQNILIDACVLDSDSGLLQQACDITGGLYLKVPQMPSLLQYLLWVFLPDQDQRSQLILPPPVHVDYRAACFCHRNLIEIGYVCSVCLSIFCNFSPICTTCETAFKISLPPVLKAKKKKLKVSA

SEQ ID NO: 11 - DNA, 1736 bp, Homo sapiens
cttttccactcctccccttacctcccttctcttctgaattctccattctgggctcttgcctgtgaaatctttctttgctttccccatcttttcctcgcattttttcaccatctttccctcaatctccaggagccaatgcgagactttggctccgattaagcgacggcccgagactcggggtgcgcgaggaggatcgacagagtggtgatggagagcaccccttcaaggggactgaaccgagtacacctacaatgcaggaatctgcaggaattcttagggggcctgagccctggggtattggaccgattgtatgggcaccctgccacatgtctggctgtcttcagggagctcccatccttggctaagaactgggtgatgcggatgctctttctggagcagcctttgccacaggctgctgtagctctgtgggtaaagaaggaattcagcaaggctcaggaggaaagtacagggctgctgagcggcctccggatctggcacacacagctgctcccaggcgggctccagggcctcatcctcaaccccattttccgccagaacctccgcattgcccttctgggtggggggaaggcctggtctgatgacacaagtcagctgggaccagacaagcatgcccgggacgttccctcccttgacaagtacgccgaggagcgatgggaggtggtcttgcacttcatggtgggctcccccagtgcagctgtcagccaggacttggctcagctcctcagccaggctgggctcatgaagagtactgaacctggagagccgccctgcattacttccgctggcttccagttcctgttgctggacaccccggctcagctctggtactttatgttgcagtatttgcagacagcccagagccggggcatggacctggtagagattctctccttcctcttccagctcagcttctctactctgggcaaggattactctgtggaaggtatgagtgattctctgttgaacttcctgcaacatctgcgtgagtttgggcttgttttccagaggaagaggaaatctcggcgttactaccccacacgcctggccatcaatctctcatcaggtgtctctggagctgggggcactgtgcatcagccaggtttcattgtcgtggaaaccaattaccgactgtatgcctacacggagtcggagctgcagattgccctcattgccctcttctctgagatgctctatcggttccccaacatggtggtggcgcaggtgacccgggagagtgtgcagcaggcaatcgccagtggcatcacagcccagcagataatccatttcctaaggacaagagcccacccagtgatgctcaaacagacacctgtgctgccccccaccatcaccgaccagatccggctctgggagctggaaagggacagactccggttcactgagggtgtcctgtataaccagttcctgtcgcaagtggactttgagctgctgctggcccacgcgcgggagctgggcgtgctcgtgttcgagaactcggccaagcggctcatggtggtgaccccggccgggcacagcgacgtcaagcgcttttggaagcggcagaaacatagctcctgagagcgcgggacttggacacggacctcggcgggcgggactgggcggggcggggcatcagaactcaggtgttttttatttacgcgtcagggcttttcttgtttaataaagttatgatagctaaaaaaaaaaaaaaaaaaaaa

SEQ ID NO: 12 - protein, 462 aa, Homo sapiens
MESTPSRGLNRVHLQCRNLQEFLGGLSPGVLDRLYGHPATCLAVFRELPSLAKNWVMRMLFLEQPLPQAAVALWVKKEFSKAQEESTGLLSGLRIWHTQLLPGGLQGLILNPIFRQNLRIALLGGGKAWSDDTSQLGPDKHARDVPSLDKYAEERWEVVLHFMVGSPSAAVSQDLAQLLSQAGLMKSTEPGEPPCITSAGFQFLLLDTPAQLWYFMLQYLQTAQSRGMDLVEILSFLFQLSFSTLGKDYSVEGMSDSLLNFLQHLREFGLVFQRKRKSRRYYPTRLAINLSSGVSGAGGTVHQPGFIVVETNYRLYAYTESELQIALIALFSEMLYRFPNMVVAQVTRESVQQAIASGITAQQIIHFLRTRAHPVMLKQTPVLPPTITDQIRLWELERDRLRFTEGVLYNQFLSQVDFELLLAHARELGVLVFENSAKRLMVVTPAGHSDVKRFWKRQKHSS

SEQ ID NO: 13 - DNA, 7503 bp, Homo sapiens
ggcgcactctgccggcaacgccgaggcgcttctgcatctgtgggccgagcattcttcaggtcatctgaaccttctgagaaaacatggtcaacgtcttgaaaggagtgcttatagaatgtgatcctgccatgaagcagtttctgctgtacttggatgagtccaatgccctggggaagaagttcatcattcaagacattgatgacactcacgtctttgtaatagcagaattggttaatgtcctccaggagcgagtgggtgaattaatggaccaaaatgctttttcccttacccagaaatgaaaatactcaatatggaccatttaggaattataagcagcaactgtgaaagacttgccactcaatatcttaggtgactgattagacatagagggttgttttaggagcatgccacgggaaagactgagggatcatgatcatttgttcagaaaaaaagcccctgaactgattttgttaccatagaatttaaaaaaaaaaaaagctttaacagttggctgtaatttggcttttattatcctttattaaaatacaaatgtcaatgcttttcctgcctttttaataccatgtcagtgtaacataggtatttattttgctcatccctgtgatctgtgcatttttgctgcgtggatgtgattgtttggtttcagttagaaacgtcatagatttgctgtttgaatatgccaaggtggggacttagacattatgtacgtctcacaaatcctacctgcataccagtcagctctattgaggaagacaatgtaaaactaatgtaaactacagtttgcatttccctgaaaacagaatattgtttttaagagggttagaaacaaccagtgggaaaggcacatgctgctttgtttagtttttccttgttcaaactttgttggtcacattttcccatctgtattcttttttattaagaaaacagcttagggaggctgaggtgggaggattgcttgagcccaggagtccgaggttgctacaaaaacaccattgcactctggcctggacaacagagagaccctgcctcaaaaaaaaaaaaaaaaaaaaaaaaaattctacttgtaccttattccctatgagaatacttatcaaacttatctaaaaaagaaaaataggaacagccatatgcaaagtcagcccaacaggaaaggacatattagattaaaatacattgcggcctgggcttagtggctcacacctgtaatcccagcactttgggaggctgaggcaggcagatcgcttgagtccaggagtcgaaaccctgtctctacaaaaaaaaaaatacaaaaatctgcctgttgtcccagccactggggaggctgaggtaggaggtcaaggctgcagtgaaccttgatcattgctactgccactccagcctaggtgacagagtgagaccctgtctccaaaaaaaaaagtgtatatgtatgtgtgtatatatagcaagagagagttctgtgatcaattgaaggcaaaaacagtaacactgagaggggctttgcttcccttcctgaagatcatgtcattggggtgggttcctgtaaagggaattttccaagagaaaagagaattttcatgacctgtagactcttacaaatccattttacctgcttccttatggtatgtttattcaaagcacctgtgtaccatatttattcacttacacagcattactgaatctggaaattttcagttaggtatattttacataattcccacccatataactcagtccatacagttcacagttttcattccctcatagcaatgcaaaaaattttgatgagttactactactaaaactagttaagtaaaagatgattcttaagaatttccaggctgggcacggtggctcacgcctgtaatcccagcactttgggaggctgaggcaggcagctcacgaggtcaggagatcgagaccatcctgctcggtgaaaccccatctctattaaaaatacaaaaaattagccgggcctggtggcgggtgcctgtagtcccatctactcaggaggctgaggcaggagaatggcgtgaacccgggaggcggagcttgcagtaagctgagattgtgccactgcactccagcctgggcgacagagggagactccatctcaaaaaaaaaaaaaaaaaaaaatgaatttccagctataccaaaatgttactaatgtatcttatatttcaggcatgtctaaatcaacttttagtatgcctcaggcatttgtcaccaaccttttatattaacatgaaacttagaaaatttttgatagaatcccagagttcaaaaggtattaggatttttgccactgaagtaaaaaagagaaaaaaagatatttatgagaaaactattgaacagtgactgtgttgtacccgagcaagttagaggaacgccacactttgagacgaatttaaaagtcctttatttagctggcagccaagaggtggctcacacttggaattctctcagctccgaggaaggggcttgattttcctttatactttggtttaggaaggggacgggagctcagttgcaacaattctacagaagtaaaaacatgcaaaaaattaaaaagacaaatggttacagagaaacaaacagttccaggtgcaggggctctaaatctatcataagatgtcaggtgtgggggctctgccagacacaaactcaaggctttatggtgtatctcttgagcgaaatcctgggaacttcgtacattgcttgcttcagtaccttatgagttaattggactctttgatatgttgagagtcagcttacacaagttaactccttgaggaaagggggtgggtaaggagtccttgatgtcctgtaaatgaaggaaccaaatggagttcctccggctttctcagctaagggagagcttattcacatggaaacaaggctaggtgattaagggagaaagggacagtctgaaaacaaggttagtaaaaacaaggttaggtattagaactgcaaagagtattaagtgaaataagtgaaggaaaatatgagctcttatttttaaaaagttgtgttggggcaaatgttaaatatctttctttctctggacattattaagaaagatagagtgatgtgaatgataggaagcccacctgtaaccacttagctgacatgtccaactatgggtgaacaggaaataagcgacattcacctaggctgtttattggaatctgactagcattatttgatttggcatactttacatgtccagaacaaggctgttggtgcttggcaccaagaaatttatgactttttttttttttttaaataaagtcctaaaggtagcattaaaatgacttaactggaggcaggaggatcactgaagcccaggagtttgaagctgcagtaagctaagaaggtgccactgcactgcagcctggatgacagagtgaaactttgtctcttaatagaactatggactgaagttgtgatattgagtgttatatttctcaataaaggttttttcttttaatactgtattaggtcaaattcaaggtcttaattccttgaattccaatttccttgtgaaatttcatgtgattaatttaaaattccagggatcctatctaacatcacagttgatggatataacaatgtattttgagaaatcagttttggtgaacagtaacagcattactgataataggcaacaaacactactgcattttatttctgataggcattataggtggtaatccaaatgattaatgattttattgctctttacattttctagaacaggtgatttgacataattgtacttttttctgagaagttggtagtgtacttactactctattttgcagttatacaataaatcttacttagctgacaactaggagtaaaagctctgacaaaaagcctctgctgtaactaaaatactgagatcattctatcttaacaaacttaacagatggggaaggggtatattttaaagatggagaaatgatgcagtttgcaaatatagtcaataaatattctcaagtgtacgtagctcaatttcatttgcagcaaagataacactgaaatgtctatggatgagattattggataaacttttttaaaaacactgttctcaagataggcaagtgattaagagcactgactgggccgggcgcggtggctcacgtctataatcctagcactttgggaggccgaggcgggcaaatcacaaggtcaggagatcaaaacaatcctggctaacaaggtgaaaccccgtctctactaaaaatacaaaaaaattagctgggcatggtggtggacgcctgtagtcccagctactcgggaggctgaggcaggagaatggtgtaatcccgggaggtggaggttgcagtgagccgagatcgtgccactgcactccagccggggtgacagagcgagactcccacccatctcaaaaaaaataaaaatgaaaagcactgattgaatctagattccttgagtccaagtgtcagatctctgcttactagctctgggatctcagatgtttcgttgattggatttctttgtgctcatttgtgtaaacaggaatgcccgtctttaaagactattaaaatgaatgtgagttaacacacaagaggtcttcaaaaagttgatggaaaatgcatattatgaaaaaaattatgcatagatttcaaaaatctttgcagcaaaataaactcatcattataacatgtctgaacaggatctagtttgaggcactaagaaggatatcagtttaaatagagcccctgtcagaacaatatgaattctgctaaaactgaagcaagaacaaacatcaaatttatggcaaagcttaggtggaagaatggtgcaatcattgatgctttgcaaaaagtttatgggaacaacgccccaaggaaatcagtttacaaatggataattcattttaagaaaggacaagacaatgttgaagatgaaacctacagcagcagaccatgccacttcgtgaggaaaaaattatctcattcatgccctacttgaagaggaccaatgattaacagcagaaacgatagccaacacaatatgctcctcagttggttcagcttttataaatctgactgaaaaattaaagttgagcacactttccactcaatggataccaaaaccatccagcccaggtcagctgcagacaaaagcagagctttcgatggaaatgtcaaacaagtgagatcaagatcctgaagcatttcttcaaagaattgtagcaaaaacagacttttaaaaccttgaattcagagacaggtataaagactgcttggtgattttgaaaggactgagatcattttgggagagatcatcttcagaaaatgaccagatacaacaagaatttaacatggcagccaaaccaacccactaacacacatttaaataagatacccaaatgcagaaagaaaagcacagtcgtcatgcaaaatagtcactactcattcaaaaactctatagttgtctgagtcgttatgctcaaaatatccaataatatttcttttgctgagctgtaaaataattattttgcaaacataaaagaaaaaaaaaagaattgtaacagaaacatggctttaccagtatgaccctcaagacaaaatacaaaacaatggctaccaagaggtggaagtggcccagtcacagcaagagcagattgatcaagagcaaaggtcatggtaacagttttttggatcctcaagtcattttgcttgttgactttttggagggccaaataaagatatcatctgcttattatgagagtgtttcgagagaaatccaaagcttagcagagaaacgcctgggaaagcttcaccagagggtcttccaccgtgacagttcccctgcgcattcctctcataaagcaagggcagtttagctagaatttctatcaaaaatcattaggtatccatctcccagtcctgatttggctccttctgacttctttttgtttcccaatcttaaaaaaatccctgaagggcacctgtttttcttcagctaataaaaaagacatggttaatttcccaggaccctcagttctttagggatagactgaatggctggtatcattgcttgaacttaatggagcttatgttgagaaataaaagaaattatattttatttttatcttttaattctatttttccatgaactttttgaagtcccctcagatataaagcagaacgttatgaaactgagttaccttgaatctagaagagtacaatgataaaggggaagatagaaacacacacatatgcgttgttttccccactttcacaatgccgtgcagaaactaacagatgaaggaggagaatccctaaaaacagagcattgggtagctagtccaccagcggtctgatgctttcattgatctcaaaactgtctctgagtaactctaccaggaaagttgtctggagggttaacatttctgaaaccatttttatctttgccttcattcttgaatgataattagtctcgaatgtttggatcacaatccattgaaagactaggctattttttcactgtcctcagacatttactgagtccagtttggactttattttattttattttttttgaaacaagatctcgctctgttgctcaggctgaagtgcaatagcgcaaactcggctcactgcaacctcccaggttcaagcaattctcgtgcctcagccatccctataggcatgcgccaccacactttgctaatcttgtatttttggtagagacggggtttgcaccatgttggccaggctggtctcgaactcccaacctcaagtaatctggcctcccaaagtggtgggattacaggcgtgagccagcgcgcccggcctggacttaacttctgaagaactctttctgtttagattgcaggagcgttctctcggctcatctcttgttttctcacccagctgttcttcttctagttggccatcattcttcatccctccctccctttcctgcagttaattatttctttgaaattttaaaacttcttaatgttgcctggaatacatgagtcttcctgatctcttcaaacggggtttgttttgttttgctttggggagaattcttttgacgtttttgaataagctgttaacaactttaatacctgtcttgtttgttttcttcagaaatttgttaattctccatgattagcacctttatgtggttatctcattattttcattcctttttaattctctgttttaggaatgcttgtcaaattcgtcactaaaattgatttactttcttgaaaacctgtttctgctgctcccaacatgatttaatcttggctactgagcttttggttacgttgcactccctttaaaattactccgtttaagtacagtgttcactctttgggtaatgtgtacaatagaagcccaatccccacctatacccaatatatccatgggacaagcatgtacatgcaccccctgagtctaaaataaaaattttaaaaaaactaaaaaaaaaaaaaaaaaa

SEQ ID NO: 14 - protein, 71 aa, Homo sapiens
MVNVLKGVLIECDPAMKQFLLYLDESNALGKKFIIQDIDDTHVFVIAELVNVLQERVGELMDQNAFSLTQK

SEQ ID NO: 15 - DNA, 5831 bp, Homo sapiens
gacatttcacgccgccgccattttgagagcgagccgagccgagctgccgggcgccgcgtccgctgccggagccccgacgacgacgccgaggaggcggaggccgcggctctcggaacgcggccggcccgtcgcccgcccgctccgccgctcccgccggccccagggcccgcaggcccgccgcggccggccaggcctcccgtccgccgcgcccggcccgaggcggggctgactccgcggcccccgaccggccgccctccgcccccggccggcccgcggccccgcagccccggccccggccccggcggcgggaggcgggccccgcggcggcggcggcggcggccgcagcgagcgacgaggccgcccggcccggcccgccggccgcccgcccgcctcggcgccgagattgggcgaatcgcgagcaagtacgtgcgcgtctccctgccgccgccgccgcccgccgcgggccgccccggggccgccgtcgccgacgacgcgcgggaggaggaggaggaggccgccccgccgccgccgccgccgccgccgccccggctcgccgccgcccgcccgccgggctcgcagccccggcccccggccgcaggcgaggcccaggccgcggccgacatgaaccaccagcagcagcagcagcagcagaaagcgggcgagcagcagttgagcgagcccgaggacatggagatggaagcgggagatacagatgacccaccaagaattactcagaaccctgtgatcaatgggaatgtggccctgagtgatggacacaacaccgcggaggaggacatggaggatgacaccagttggcgctccgaggcaacctttcagttcactgtggagcgcttcagcagactgagtgagtcggtccttagccctccgtgttttgtgcgaaatctgccatggaagattatggtgatgccacgcttttatccagacagaccacaccaaaaaagcgtaggattctttctccagtgcaatgctgaatctgattccacgtcatggtcttgccatgcacaagcagtgctgaagataataaattacagagatgatgaaaagtcgttcagtcgtcgtattagtcatttgttcttccataaagaaaatgattggggattttccaattttatggcctggagtgaagtgaccgatcctgagaaaggatttatagatgatgacaaagttacctttgaagtctttgtacaggcggatgctccccatggagttgcgtgggattcaaagaagcacacaggctacgtcggcttaaagaatcagggagcgacttgttacatgaacagcctgctacagacgttatttttcacgaatcagctacgaaaggctgtgtacatgatgccaaccgagggggatgattcgtctaaaagcgtccctttagcattacaaagagtgttctatgaattacagcatagtgataaacctgtaggaacaaaaaagttaacaaagtcatttgggtgggaaactttagatagcttcatgcaacatgatgttcaggagctttgtcgagtgttgctcgataatgtggaaaataagatgaaaggcacctgtgtagagggcaccatacccaaattattccgcggcaaaatggtgtcctatatccagtgtaaagaagtagactatcggtctgatagaagagaagattattatgatatccagctaagtatcaaaggaaagaaaaatatatttgaatcatttgtggattatgtggcagtagaacagctcgatggggacaataaatacgacgctggggaacatggcttacaggaagcagagaaaggtgtgaaattcctaacattgccaccagtgttacatctacaactgatgagatttatgtatgaccctcagacggaccaaaatatcaagatcaatgataggtttgaattcccagagcagttaccacttgatgaatttttgcaaaaaacagatcctaaggaccctgcaaattatattcttcatgcagtcctggttcatagtggagataatcatggtggacattatgtggtttatctaaaccccaaaggggatggcaaatggtgtaaatttgatgacgacgtggtgtcaaggtgtactaaagaggaagcaattgagcacaattatgggggtcacgatgacgacctgtctgttcgacactgcactaatgcttacatgttagtctacatcagggaatcaaaactgagtgaagttttacaggcggtcaccgaccatgatattcctcagcagttggtggagcgattacaagaagagaaaaggatcgaggctcagaagcggaaggagcggcaggaagcccatctctatatgcaagtgcagatagtcgcagaggaccagttttgtggccaccaagggaatgacatgtacgatgaagaaaaagtgaaatacactgtgttcaaagtattgaagaactcctcgcttgctgagtttgttcagagcctctctcagaccatgggatttccacaagatcaaattcgattgtggcccatgcaagcaaggagtaatggaacaaaacgaccagcaatgttagataatgaagccgacggcaataaaacaatgattgagctcagtgataatgaaaacccttggacaatattcctggaaacagttgatcccgagctggctgctagtggagcgaccttacccaagtttgataaagatcatgatgtaatgttatttttgaagatgtatgatcccaaaacgcggagcttgaattactgtgggcatatctacacaccaatatcctgtaaaatacgtgacttgctcccagttatgtgtgacagagcaggatttattcaagatactagccttatcctctatgaggaagttaaaccgaatttaacagagagaattcaggactatgacgtgtctcttgataaagcccttgatgaactaatggatggtgacatcatagtatttcagaaggatgaccctgaaaatgataacagtgaattacccaccgcaaaggagtatttccgagatctctaccaccgcgttgatgtcattttctgtgataaaacaatccctaatgatcctggatttgtggttacgttatcaaatagaatgaattattttcaggttgcaaagacagttgcacagaggctcaacacagatccaatgttgctgcagtttttcaagtctcaaggttatagggatggcccaggtaatcctcttagacataattatgaaggtactttaagagatcttctacagttcttcaagcctagacaacctaagaaactttactatcagcagcttaagatgaaaatcacagactttgagaacaggcgaagttttaaatgtatatggttaaacagccaatttagggaagaggaaataacactatatccagacaagcatgggtgtgtccgggacctgttagaagaatgtaaaaaggccgtggagcttggggagaaagcatcagggaaacttaggctgctagaaattgtaagctacaaaatcattggtgttcatcaagaagatgaactattagaatgtttatctcctgcaacgagccggacgtttcgaatagaggaaatccctttggaccaggtggacatagacaaagagaatgagatgcttgtcacagtggcgcatttccacaaagaggtcttcggaacgttcggaatcccgtttttgctgaggatacaccagggcgagcattttcgagaagtgatgaagcgaatccagagcctgctggacatccaggagaaggagtttgagaagtttaaatttgcaattgtaatgatgggccgacaccagtacataaatgaagacgagtatgaagtaaatttgaaagactttgagccacagcccggtaatatgtctcatcctcggccttggctagggctcgaccacttcaacaaagccccaaagaggagtcgctacacttaccttgaaaaggccattaaaatccataactgatttccaagctggtgtgttcaaggcgaggacggtgtgtgggtggccccttaacagcctagaactttggtgcacgtgccctctagccgaagtcttcagcaagaggattcgctgctggtgttaattttattttattgaggctgttcagtttggcttctctgtatctattgactgccctttttgagcaaaatgaagatgtttttataaagcttggatgccaatgagagttattttatggtaaccacagtgcaaggcaactgtcagcgcaatgggggagaagaggttagtggatcgggggtccctggctcaaggtctctgggctgtccctagtgggcacgagtggctcggctgccttcctggggtcccgtgcaccagccctgcagctagcaagtcttgtgtttaggctcgtctgacctatttccttcagttatactttcaatgaccttttgtgcatctgttaaggcaaaacagagaaactcacaacctaataaatagcgctcttcccttcattgtgtgcattgtcggcccttcctcgggttctcctcctccagctgcctgggggctttttaataaacttgtctcacctcgtcagccactactgtctgcagcccctttgcaaagtggatgcactgaatacagtccggacagacattgtgggggtctttttattaaatcaagaacattgttaaattcaattaaggtttactctgctgccttggcagacttacgatctcaacagttcatacgagcaggtgaaaggattataaatagaatttcgttaaagtggaacagacgacaagaaagccttttagcaagagggcatgctcactagtggttagtaagctgtcgactttgtaaaaaagttaaaaatgaaaaaaaaaggaaaaatgaattgtatatttaatgaatgaacatgtacaatttgccactgggaggaggttcctttttgttgggtgagtctgcaagtgaatttcactgatgttgatattcattgtgtgtagttttatttcggtcccagccccgtttccttttattttggagctaatgccagctgcgtgtctagttttgagtgcagtaaaatagaatcagcaaatcactcttatttttcatccttttccggtattttttgggttgtttctgtgggagcagtgtacaccaactcttcctgtatattgcctttttgctggaaaatgttgtatgttgaataaaattttctataaaaattataattcagtgagttacgtggaagtggaggaagatttctactctccctggaaacaggcctgggaaaccttggcatttgtaacaaggtttcactgagatgtacttttccttctaattccgttttgcgggggcagggtctcttgtttctttttttttttttttttttttttagcctctaactagtcacatttactcttaagaaatgaaaggttttccaggagagaactgtgtacaaataaggtgactggagatgtgacctgatgtgtcacgaggcccttcggggcggcaggcgctatcgtgggcgtggtccttgcaccgtcccatcggccttgccttccagctccgtggcacggtttcctggtctttgggccagtgtgtaccttggagtgacttcctttctcaacttccactgcagtgtgtgtgccttctgctctgagagctgccttgtgacccgtgtgatagaaagcagggagtgagggtccccgcggacctggcccttccctccttcctcccccagaaagaggagttagagcaggggtgcgagagccgttcgctgtgggtttgtctttgaacaaacattaaggtgtcttgtttttgttctgggctgggggttggctgtagtcttaggtaactgaaagttcctactctcccttaaggtattaaatgactctttttccaaa

SEQ ID NO: 16 - protein, 1102 aa, Homo sapiens
MNHQQQQQQQKAGEQQLSEPEDMEMEAGDTDDPPRITQNPVINGNVALSDGHNTAEEDMEDDTSWRSEATFQFTVERFSRLSESVLSPPCFVRNLPWKIMVMPRFYPDRPHQKSVGFFLQCNAESDSTSWSCHAQAVLKIINYRDDEKSFSRRISHLFFHKENDWGFSNFMAWSEVTDPEKGFIDDDKVTFEVFVQADAPHGVAWDSKKHTGYVGLKNQGATCYMNSLLQTLFFTNQLRKAVYMMPTEGDDSSKSVPLALQRVFYELQHSDKPVGTKKLTKSFGWETLDSFMQHDVQELCRVLLDNVENKMKGTCVEGTIPKLFRGKMVSYIQCKEVDYRSDRREDYYDIQLSIKGKKNIFESFVDYVAVEQLDGDNKYDAGEHGLQEAEKGVKFLTLPPVLHLQLMRFMYDPQTDQNIKINDRFEFPEQLPLDEFLQKTDPKDPANYILHAVLVHSGDNHGGHYVVYLNPKGDGKWCKFDDDVVSRCTKEEAIEHNYGGHDDDLSVRHCTNAYMLVYIRESKLSEVLQAVTDHDIPQQLVERLQEEKRIEAQKRKERQEAHLYMQVQIVAEDQFCGHQGNDMYDEEKVKYTVFKVLKNSSLAEFVQSLSQTMGFPQDQIRLWPMQARSNGTKRPAMLDNEADGNKTMIELSDNENPWTIFLETVDPELAASGATLPKFDKDHDVMLFLKMYDPKTRSLNYCGHIYTPISCKIRDLLPVMCDRAGFIQDTSLILYEEVKPNLTERIQDYDVSLDKALDELMDGDIIVFQKDDPENDNSELPTAKEYFRDLYHRVDVIFCDKTIPNDPGFVVTLSNRMNYFQVAKTVAQRLNTDPMLLQFFKSQGYRDGPGNPLRHNYEGTLRDLLQFFKPRQPKKLYYQQLKMKITDFENRRSFKCIWLNSQFREEEITLYPDKHGCVRDLLEECKKAVELGEKASGKLRLLEIVSYKIIGVHQEDELLECLSPATSRTFRIEEIPLDQVDIDKENEMLVTVAHFHKEVFGTFGIPFLLRIHQGEHFREVMKRIQSLLDIQEKEFEKFKFAIVMMGRHQYINEDEYEVNLKDFEPQPGNMSHPRPWLGLDHFNKAPKRSRYTYLEKAIKIHN

SEQ ID NO: 17 - DNA, 4674 bp, Homo sapiens
gccagggcgtgtcccgtgtgcccgagagcgccggcggcggggccggagggcgggccctgggccgagtgacaggccgcagccccccgagcaccgtcgaagccggcgcgcccgcccggtgcagccgctgtgcgagagcgaccccgcggtccaagcctcgcgtggccctgccgggccccttctttccccgagtagggcgcagcttcccagcctccgccccggcctcgcctggcgcttccttccgggtccttcggcctttccctggcggtgcggcaggccctcgcctcatcccaccaggcacgccgcggtgctcggccctgggtatccgggcaggctgcctccgttagggccgcccctgctctccggacgcgacttttcattggtctcagaatttcttggctcctcttggcctctgcagccttgctggaggctgccctgcggaatctgaatatggatcagaaactttcgaagttggtagaagagctcacaacttcaggagaaccccgactaaatcctgagaaaatgaaggaactgaagaaaatttgcaagtcttcagaggagcagctgagccgcgcctaccgcctgctgatagcacagctgacccaggagcacgccgagatccgtctctcagccttccagattgtggaggaactcttcgtcaggtctcaccagttccggatgctggttgtttccaacttccaggagttcctggagctcacgctgggcacagaccccgcacagcctctgccgccccccagggaggcggcacagaggctgaggcaggcgaccacccgggccgtggaagggtggaatgagaagtttggggaggcctacaagaagcttgccttgggctaccacttcttaagacacaacaaaaaggtggattttcaagacacgaatgctcggagtctggcagaaaggaagagagaagaggagaagcagaagcacttggataaaatttatcaagaaagagccagccaggcggagagggagatgcaagaaatgtctggagaaattgaatcctgcttgacggaggtagagagctgctttaggctgctggtgccttttgactttgacccgaacccggagacggaatcccttggcatggcttctggcatgtccgatgcccttcgctcctcctgcgcgggccaggtgggcccctgccggtctggcacccctgacccccgggacggggagcagccctgctgcagtagagacctgcctgcctctgcaggccaccccagagcgggcggcggggcacagccatcccagacagccacaggtgacccctcagatgaggacgaggacagcgacctcgaggagtttgtgcggagccacgggctgggctcgcacaagtacacgctggatgtggagctctgctcagagggcctgaaggtgcaggagaacgaggacaaccttgctctcatccacgccgcccgcgacacactcaagctcatccggaacaagttcctgccggctgtgtgctcgtggatccagcgcttcacccgcgtcgggacccacggtggatgtttaaagcgtgccattgacctgaaggctgaattggagctcgtactgagaaaatacaaggagctggacatcgagcctgagggaggggaaaggcgcaggacagaagccctgggggatgcggaggaagatgaggacgatgaggactttgtggaggtccctgagaaggaggggtatgagccacacatccccgaccacttgcggcctgagtatgggctggaggcagcaccagagaaagacacagttgtgcggtgcttgcggacgaggacgaggatggacgaggaggtgtcggaccccacctctgcggctgctcagctgcggcagctccgggaccacttgcctccaccctcatctgccagcccctccagagcgttgccagagccacaggaggcccagaagctggcagcagagcgggcccgggcgcctgtggtgccctacggcgtggacctgcactactggggccaggagctccccacagccgggaagattgtcaagtctgactcccagcaccgcttctggaagcccagcgaggtggaggaggaagtggtcaatgccgacatctccgagatgctccggagccgccacatcacttttgccgggaagtttgagcctgtgcagcactggtgccgtgccccgaggccagacggccggctctgtgagcgccaagaccggctgaagtgccctttccatgggaagattgttccacgggacgacgaaggacggccgctcgacccggaagacagggctcgtgagcagcggcggcagctgcagaagcaggagcgcccggaatggcaggaccctgagttgatgagagacgtggaagcagccacagggcaggatctcggctcatccaggtacagcgggaaaggcagggggaagaagaggaggtaccccagcctcaccaacctgaaggctcaggctgataccgcccgcgctcgcattgggagaaaagtcttcgccaaggcagctgtgcggagggtagtggcagccatgaaccggatggaccagaagaagcacgagaagttttcaaaccagtttaactacgcactgaactagagagcggggcccagtgcactggccatcagcactttctccctctgccagtgtctcaggacagcagagtgggcgtgggtctgggcagtaaccatgctttgtctattactgtgtttgatgtaaagaaatggtgtgttgcaatgccctgaaggtacggccgctctgctgctacagggttcggcatcgtctggtgatgggtctggcctcgcagaagaggccctcgggcctggagatgtgaacacaggcagcgaccctgttccagagggcttctgcgagtcctcgtgagaccagtgcttgtcgtggtgtggggttcagcacggacggaatgtgtgtgcagctcagccttcagagcgtgcattccccagccaggaggcgaccactcagaggaactctgggaaacccacttttgtgcaaatgctgtttttaacacaaacacaaaggctagtgaaccgttcagtcatctgctttctgtttctggatgtgccttttcatacatgtgtcctcttgtccctggcttcttacacttggcgttgtttttaaggtttatccatgcagttcccctccaatgtataaaacaaaggaggtgaaaacctgtccatgcggaagcttgtgcacccatgttcacagcagcattggagaaggataccgaacatcttctcgtgggcttactggccatttgtgtatctcctttggagaggagtctattcaaacctcttgcctatttttaattgaatgatttatcttgagttgtaacagttgttttttttgtttttccttttagagatgggcttttgctcttacccaggctgagtgcagtggcagaatcatagctcagtgcagcctcaaactcctgggctcaagccatccttccacgtcagcctcccaggtagctgggactacaggcacacaccacaacacctggctaattttttaaattttttgtagagatgaggtctcactgtgttgcccacggtgatctcgaactcctagcctcaagcgatcctcctgcttcggtctcccaaagtgttgggattacaggcatgagccaccactcctggccaggagtttatatgtatactgtggatactagatcctcatgtgatttgcaaaaactttatttatttatttatttatttttgaaatggaatcttgctctgtcgccaggctggagtgcaatggcgtgatctcggctcactgcaactaccacctcctgggttcaagcgattcgcctgcgtcagcgtcctgagtagctgggactacaggcgcgcaccaccacgcccagctaatttttgtatttttagtagagacgggatttcactgtgttggctgggatggtcttgatctcttgacctcgtgatccacccacctcggcctcccatagtgctgggattacaggtgtgagccaccgcactcagctgatttgcaaaaactttcttccatactgttgtttcactttctggatagtgtcctctgaagcacaaaagttaattttgatgaagtacagcaatttatctgtttttttcttttgttgcttatgcttttgctgtcacatttcagaagccatcacctaatccaagatcacagagatttacacctagtttctaataagcattttataatttcagctcttatgtgtagatctttgatccattgtgaattaagttttgtgtgtggtgtaagagcccacattcttttgcatgtggatatccagttgtcccagcaccatttgttgaaaacattatttttccccattgaattatcttcgcaccattattgataatcagttgaccaaaaatgtacaggcttatttctgggcacttgactctattccattgacctgtttaaccttatgccagtgccacagtgccttgatcagtgctgctttgttgtgagaagttttactttgttctgcttcaaggctgttttgactcttctgcatctcttgcatttccaaatgaattttaggatccactcatcagtttcttcaaaaaaaaaaaaaaagcagctgagatttttgataggaattacattaaatctagagattgctttggaatgtattaccgtcttaatattaaatcttctgagtcatgaaaaaaaaaa

SEQ ID NO: 18 - protein, 709 aa, Homo sapiens
MDQKLSKLVEELTTSGEPRLNPEKMKELKKICKSSEEQLSRAYRLLIAQLTQEHAEIRLSAFQIVEELFVRSHQFRMLVVSNFQEFLELTLGTDPAQPLPPPREAAQRLRQATTRAVEGWNEKFGEAYKKLALGYHFLRHNKKVDFQDTNARSLAERKREEEKQKHLDKIYQERASQAEREMQEMSGEIESCLTEVESCFRLLVPFDFDPNPETESLGMASGMSDALRSSCAGQVGPCRSGTPDPRDGEQPCCSRDLPASAGHPRAGGGAQPSQTATGDPSDEDEDSDLEEFVRSHGLGSHKYTLDVELCSEGLKVQENEDNLALIHAARDTLKLIRNKFLPAVCSWIQRFTRVGTHGGCLKRAIDLKAELELVLRKYKELDIEPEGGERRRTEALGDAEEDEDDEDFVEVPEKEGYEPHIPDHLRPEYGLEAAPEKDTVVRCLRTRTRMDEEVSDPTSAAAQLRQLRDHLPPPSSASPSRALPEPQEAQKLAAERARAPVVPYGVDLHYWGQELPTAGKIVKSDSQHRFWKPSEVEEEVVNADISEMLRSRHITFAGKFEPVQHWCRAPRPDGRLCERQDRLKCPFHGKIVPRDDEGRPLDPEDRAREQRRQLQKQERPEWQDPELMRDVEAATGQDLGSSRYSGKGRGKKRRYPSLTNLKAQADTARARIGRKVFAKAAVRRVVAAMNRMDQKKHEKFSNQFNYALN

SEQ ID NO: 19 - DNA, 2947 bp, Homo sapiens
tgctgtagctgccatgggcaaaagagaccgagcggaccgcggtgagacgttgcgcgggcacgctcagccacgactgcccttgccggccctgccccccgctctgcctcggagctgctccgggcctctgcgccggccgaccctgctggccctcccgcgcgcaccccgttgggacaggcctttgggcgggagagatgctggacctgggcgcagcccagcgaactcggcctaggggagacgggtgaggggcgcaacgcctgcgggatgcaggtggctcttagctaggagtttgcggcggcgcagacaagaagaaatccaggaagcggcactatgaggatgaagaggatgatgaagaggacgccccggggaacgaccctcaggaagcggttccctcggcggcggggaagcaggtggatgagtcaggcaccaaagtggatgaatatggagccaaggactacaggctgcaaatgccgctgaaggacgaccacacctccaggcccctctgggtggctcccgatggccatatcttcttggaagccttctctccagtttacaaatatgcccaagacttcttggtggctattgcagagccagtgtgccgaccaacccatgtgcatgagtacaaactaactgcctactccttgtatgcagctgtcagcgttgggctgcaaaccagtgacatcaccgagtacctcaggaagctcagcaagactggagtccctgatggaattatgcagtttattaagttgtgtactgtcagctatggaaaagtcaagctggtcttgaagcacaacagatacttcgttgaaagttgccaccctgatgtaatccagcatcttctccaggaccccgtgatccgagaatgccgcttaagaaactctgaaggggaggccactgagctcatcacagagactttcacaagcaaatctgccatttctaagactgctgaaagcagtggtgggccctccacttcccgagtgacagatccacagggtaaatctgacatccccatggacctgtttgacttctatgagcaaatggacaaggatgaagaagaagaagaagagacacagacagtgtcttttgaagtcaagcaggaaatgattgaggaactccagaaacgttgcatccacctggagtaccctctgttggcagaatatgacttccggaatgattctgtcaaccctgatatcaacattgacctaaagcccacagctgtcctcagaccctatcaggagaagagcttgcgaaagatgtttggaaacgggcgtgcacgttcgggggtcattgttcttccctgcggtgctggaaagtccctggttggtgtgactgctgcatgcactgtcagaaaacgctgtctggtgctgggcaactcagctgtttctgtggagcagtggaaagcccagttcaagatgtggtccaccattgacgacagccagatctgccggttcacctccgatgccaaggacaagcccatcggctgctccgttgccattagcacctactccatgctgggccacaccaccaaaaggtcctgggaggccgagcgagtcatggagtggctcaagacccaggagtggggcctcatgatcctggatgaagtgcacaccataccagccaagatgttccgaagggtgctcaccatcgtgcaggcccactgtaagctgggtttgactgcgaccctcgtccgcgaagatgacaaaattgtggatttaaattttctgattgggcctaagctctacgaagccaactggatggagctgcagaataatggctacatcgccaaagtccagtgtgctgaggtctggtgccctatgtctcctgaattttaccgggaatatgtggcaatcaaaaccaagaaacgaatcttgctgtacaccatgaaccccaacaaatttagagcttgccagtttctgatcaagtttcatgaaaggaggaatgacaagattattgtctttgctgacaatgtgtttgccctaaaggaatatgccattcgactgaacaaaccctatatctacggacctacgtctcagggggaaaggatgcaaattctccagaatttcaagcacaaccccaaaattaacaccatcttcatatccaaggtaggtgacacttcgtttgatctgccggaagcaaatgtcctcattcagatctcatcccatggtggctccaggcgtcaggaagcccaaaggctagggcgggtgcttcgagctaaaaaagggatggttgcagaagagtacaatgcctttttctactcactggtatcccaggacacacaggaaatggcttactcaaccaagcggcagagattcttggtagatcaaggttatagcttcaaggtgatcacgaaactcgctggcatggaggaggaagacttggcgttttcgacaaaagaagagcaacagcagctcttacagaaagtcctggcagccactgacctggatgccgaggaggaggtggtggctggggaatttggctccagatccagccaggcatctcggcgctttggcaccatgagttctatgtctggggccgacgacactgtgtacatggagtaccactcatcgcggagcaaggcgcccagcaaacatgtacacccgctcttcaagcgctttaggaaatgatgcttaggcagggtacttcgttcaagaccggcgcttggcacccttgttggaaagggattttcagcataacattttccttccacctctttgaccttccctccagcgttggccaaattgtgctgaggaagatgcatcaagggcttggctgtgccttcataggtcatctagggttttataaaggaggaggagacaatattttttcaaactttttggggagtggggtcatttctgtatataaaaaatgttaatatttaaggtgtatttatgttaccgttctgaataaacagaatggaccattgaaccagtaaaaaaaaaaaaaaaaaaaa

SEQ ID NO: 20 - protein, 718 aa, Homo sapiens
MPLKDDHTSRPLWVAPDGHIFLEAFSPVYKYAQDFLVAIAEPVCRPTHVHEYKLTAYSLYAAVSVGLQTSDITEYLRKLSKTGVPDGIMQFIKLCTVSYGKVKLVLKHNRYFVESCHPDVIQHLLQDPVIRECRLRNSEGEATELITETFTSKSAISKTAESSGGPSTSRVTDPQGKSDIPMDLFDFYEQMDKDEEEEEETQTVSFEVKQEMIEELQKRCIHLEYPLLAEYDFRNDSVNPDINIDLKPTAVLRPYQEKSLRKMFGNGRARSGVIVLPCGAGKSLVGVTAACTVRKRCLVLGNSAVSVEQWKAQFKMWSTIDDSQICRFTSDAKDKPIGCSVAISTYSMLGHTTKRSWEAERVMEWLKTQEWGLMILDEVHTIPAKMFRRVLTIVQAHCKLGLTATLVREDDKIVDLNFLIGPKLYEANWMELQNNGYIAKVQCAEVWCPMSPEFYREYVAIKTKKRILLYTMNPNKFRACQFLIKFHERRNDKIIVFADNVFALKEYAIRLNKPYIYGPTSQGERMQILQNFKHNPKINTIFISKVGDTSFDLPEANVLIQISSHGGSRRQEAQRLGRVLRAKKGMVAEEYNAFFYSLVSQDTQEMAYSTKRQRFLVDQGYSFKVITKLAGMEEEDLAFSTKEEQQQLLQKVLAATDLDAEEEVVAGEFGSRSSQASRRFGTMSSMSGADDTVYMEYHSSRSKAPSKHVHPLFKRFRK

SEQ ID NO: 21 - DNA, 2568 bp, Homo sapiens
ttcatgagggaggcgggtcgaccccgctgcacagtccggccggcgccatgaagctcaacgtggacgggctcctggtctacttcccgtacgactacatctaccccgagcagttctcctacatgcgggagctcaaacgcacgctggacgccaagggtcatggagtcctggagatgccctcaggcaccgggaagacagtatccctgttggccctgatcatggcataccagagagcatatccgctggaggtgaccaaactcatctactgctcaagaactgtgccagagattgagaaggtgattgaagagcttcgaaagttgctcaacttctatgagaagcaggagggcgagaagctgccgtttctgggactggctctgagctcccgcaaaaacttgtgtattcaccctgaggtgacacccctgcgctttgggaaggacgtcgatgggaaatgccacagcctcacagcctcctatgtgcgggcgcagtaccagcatgacaccagcctgccccactgccgattctatgaggaatttgatgcccatgggcgtgaggtgcccctccccgctggcatctacaacctggatgacctgaaggccctggggcggcgccagggctggtgcccatacttccttgctcgatactcaatcctgcatgccaatgtggtggtttatagctaccactacctcctggaccccaagattgcagacctggtgtccaaggaactggcccgcaaggccgtcgtggtcttcgacgaggcccacaacattgacaacgtctgcatcgactccatgagcgtcaacctcacccgccggacccttgaccggtgccagggcaacctggagaccctgcagaagacggtgctcaggatcaaagagacagacgagcagcgcctgcgggacgagtaccggcgtctggtggaggggctgcgggaggccagcgccgcccgggagacggacgcccacctggccaaccccgtgctgcccgacgaagtgctgcaggaggcagtgcctggctccatccgcacggccgagcatttcctgggcttcctgaggcggctgctggagtacgtgaagtggcggctgcgtgtgcagcatgtggtgcaggagagcccgcccgccttcctgagcggcctggcccagcgcgtgtgcatccagcgcaagcccctcagattctgtgctgaacgcctccggtccctgctgcatactctggagatcaccgaccttgctgacttctccccgctcaccctccttgctaactttgccacccttgtcagcacctacgccaaaggcttcaccatcatcatcgagccctttgacgacagaaccccgaccattgccaaccccatcctgcacttcagctgcatggacgcctcgctggccatcaaacccgtatttgagcgtttccagtctgtcatcatcacatctgggacactgtccccgctggacatctaccccaagatcctggacttccaccccgtcaccatggcaaccttcaccatgacgctggcacgggtctgcctctgccctatgatcatcggccgtggcaatgaccaggtggccatcagctccaaatttgagacccgggaggatattgctgtgatccggaactatgggaacctcctgctggagatgtccgctgtggtccctgatggcatcgtggccttcttcaccagctaccagtacatggagagcaccgtggcctcctggtatgagcaggggatccttgagaacatccagaggaacaagctgctctttattgagacccaggatggtgccgaaaccagtgtcgccctggagaagtaccaggaggcctgcgagaatggccgcggggccatcctgctgtcagtggcccggggcaaagtgtccgagggaatcgactttgtgcaccactacgggcgggccgtcatcatgtttggcgtcccctacgtctacacacagagccgcattctcaaggcgcggctggaatacctgcgggaccagttccagattcgtgagaatgactttcttaccttcgatgccatgcgccacgcggcccagtgtgtgggtcgggccatcaggggcaagacggactacggcctcatggtctttgccgacaagcggtttgcccgtggggacaagcgggggaagctgccccgctggatccaggagcacctcacagatgccaacctcaacctgaccgtggacgagggtgtccaggtggccaagtacttcctgcggcagatggcacagcccttccaccgggaggatcagctgggcctgtccctgctcagcctggagcagctagaatcagaggagacgctgaagaggatagagcagattgctcagcagctctgagtggggcgggtggggccataaacggttcctggtgactcctgagtcttgcctggccctggttcccagcggcggtggtgctagaaggtcttatgaagtcaggtgacatttctcactgtcacgtccacagcctttaatcgcaggagaaggcagctatccaccaggtacccagaggcaagggggggccaggagatgatagaccccctctcaccccaccagcccatccctcctgcactgttcc

SEQ ID NO: 22 - protein, 760 aa, Homo sapiens
MKLNVDGLLVYFPYDYIYPEQFSYMRELKRTLDAKGHGVLEMPSGTGKTVSLLALIMAYQRAYPLEVTKLIYCSRTVPEIEKVIEELRKLLNFYEKQEGEKLPFLGLALSSRKNLCIHPEVTPLRFGKDVDGKCHSLTASYVRAQYQHDTSLPHCRFYEEFDAHGREVPLPAGIYNLDDLKALGRRQGWCPYFLARYSILHANVVVYSYHYLLDPKIADLVSKELARKAVVVFDEAHNIDNVCIDSMSVNLTRRTLDRCQGNLETLQKTVLRIKETDEQRLRDEYRRLVEGLREASAARETDAHLANPVLPDEVLQEAVPGSIRTAEHFLGFLRRLLEYVKWRLRVQHVVQESPPAFLSGLAQRVCIQRKPLRFCAERLRSLLHTLEITDLADFSPLTLLANFATLVSTYAKGFTIIIEPFDDRTPTIANPILHFSCMDASLAIKPVFERFQSVIITSGTLSPLDIYPKILDFHPVTMATFTMTLARVCLCPMIIGRGNDQVAISSKFETREDIAVIRNYGNLLLEMSAVVPDGIVAFFTSYQYMESTVASWYEQGILENIQRNKLLFIETQDGAETSVALEKYQEACENGRGAILLSVARGKVSEGIDFVHHYGRAVIMFGVPYVYTQSRILKARLEYLRDQFQIRENDFLTFDAMRHAAQCVGRAIRGKTDYGLMVFADKRFARGDKRGKLPRWIQEHLTDANLNLTVDEGVQVAKYFLRQMAQPFHREDQLGLSLLSLEQLESEETLKRIEQIAQQL

SEQ ID NO: 23 - DNA, 6765 bp, Homo sapiens
agagcttccatggagtcagggcagccggctcgacggattgccatggcgccgctgctggagtacgagcgacagctggtgctggaactgctcgacactgacgggctagtagtgtgcgcccgcgggctcggcgcggaccggctcctctaccactttctccagctgcactgccacccagcctgcctggtgctggtgctcaacacgcagccggccgaggaggagtattttatcaatcagctgaagatagaaggagttgaacacctccctcgccgtgtaacaaatgaaatcacaagcaacagtcgctatgaagtttacacacaaggtggtgttatatttgcgacaagtaggatacttgtggttgacttcttgactgatagaataccttcagatttaattactggcatcttggtgtatagagcccacagaataatcgagtcttgtcaagaagcattcatcttgcgcctctttcgccagaaaaacaaacgtggttttattaaagctttcacagacaatgctgttgcctttgatactggtttttgtcatgtggaaagagtgatgagaaatctttttgtgaggaaactgtatctgtggccaaggttccatgtagcagtaaactcatttttagaacagcacaaacctgaagttgtagaaatccatgtttctatgacacctaccatgcttgctatacagactgctatactggacattttaaatgcatgtctaaaggaactaaaatgccataacccatcgcttgaagtggaagatttatctttagaaaatgctattggaaaaccttttgacaagacaatccgccattatctggatcctttgtggcaccagcttggagccaagactaaatccttagttcaggatttgaagatattacgaactttgctgcagtatctctctcagtatgattgtgtcacatttcttaatcttctggaatctctgagagcaacggaaaaagcttttggtcagaattcaggttggctgtttcttgactccagcacctcgatgtttataaatgctcgagcaagggtttatcatcttccagatgccaaaatgagtaaaaaagaaaaaatatctgaaaaaatggaaattaaagaaggggaagaaacaaaaaaggaactggtcctagaaagcaacccaaagtgggaggcactgactgaagtattaaaagaaattgaggcagaaaataaggagagtgaagctcttggtggtccaggtcaagtactgatttgtgcaagtgatgaccgaacatgttcccagctgagagactatatcactcttggagcggaggccttcttattgaggctctacaggaaaacctttgagaaggatagcaaagctgaagaagtctggatgaaatttaggaaggaagacagttcaaagagaattaggaaatctcacaaaagacctaaagacccccaaaacaaagaacgggcttctaccaaagaaagaaccctcaaaaagaaaaaacggaagttgaccttaactcaaatggtaggaaaacctgaagaactggaagaggaaggagatgtcgaggaaggatatcgtcgagaaataagcagtagcccagaaagctgcccggaagaaattaagcatgaagaatttgatgtaaatttgtcatcggatgctgctttcggaatcctgaaagaacccctcactatcatccatccgcttctgggttgcagcgacccctatgctctgacaagggtactacatgaagtggagccaagatacgtggttctttatgacgcagagctaacctttgttcggcagcttgaaatttacagggcgagtaggcctgggaaacctctgagggtttactttcttatatacggaggttcaactgaggaacaacgctatctcactgctttgcggaaagaaaaggaagcttttgaaaaactcataagggaaaaagcaagcatggttgtccctgaagaaagagaaggcagagatgaaacaaacttagacctagtaagaggcacagcatctgcagatgtttccactgacactcggaaagccggtggccaggaacagaatggtacacagcaaagcatagttgtggatatgcgtgaatttcgaagtgagcttccatctctgatccatcgtcggggcattgacattgaacccgtgactttagaggttggagattacatcctcactccagaaatgtgcgtggagcgcaagagtatcagtgatttaatcggctctttaaataacggccgcctctacagccagtgcatctccatgtcccgctactacaagcgtcccgtgcttctgattgagtttgaccctagcaagcctttctctctcacttcccgaggtgccttgtttcaggagatctccagcaatgacattagttccaaactcactcttcttacacttcacttccccagactacggattctctggtgcccctctcctcatgcaacggcggagttgtttgaggagctgaaacaaagcaagccacagcctgatgcggcgacagcactggccattacagcagattctgaaacccttcccgagtcagagaagtataatcctggtccccaagacttcttgttaaaaatgccaggggtgaatgccaaaaactgccgctccttgatgcaccacgttaagaacatcgcagaattagcagccctgtcacaagacgagctcacgagtattctggggaatgctgcaaatgccaaacagctttatgatttcattcacacctcttttgcagaagtcgtatcaaaaggaaaagggaaaaagtgaacagtgatggctgttttcttatcccatgcctgtacttttcagcggctccttgccagacatcataggtcattattaattattggtttgctatttcattcttttccaatgctcttaatgattgtacggtggaccagaagccaggattcctctctgaactctgcagttaggcatcacttgaacttgcctgtgcctgctctttttcctccctgcaccgtctatgccgggcttagcatgtttctttttaaatgaggtttgtcaggatcaggtaaagttcctacaagtgattacagaaggtagaaactttacctgatcctaacagatctcatttagaaaggaatatgctaagcctggcatggacggtgcagggagggaaaagagcaggcacaagaaagctaccatttttaacagtccttgttatctagtgcaacataaataacagtcttaattgcacttatacccatgtcctgtggctctccaaatctggtctttgctgttgtgtctgctggacgcttgaactgatgtttgtgtaggaaatcatgttctgaccctttgtctacaaaggagccttctggaacactgagaagaaacatctctttgccattcctgaccagttctctctaccacattttcttcagctccatacttctgcctgtctgctctaaggaaatttcatggagccttcctactactaattcaagacagtctcctcaaaaactggttgactagtcttctaatgaccctaacatatgtagcatatactataatttcattgttccaaattagtatttttaaagcaaaatgaattacctgtttgcaaaagttaatgatgaaggagctcttagaattctcaatttttgcacatattcagtctcctaatatcagagatccctaagtccagctggctagttacagagttttttcagacttcctcgtttctcagctcttatatcctaagacaccagcatcatatcctctagaaatacaacctaattggcagtgagccgagatcgcaccactgcacccctgcctgggcgacagagtgagactttgtctctattacaaaaagaaaagaaaagaaatacaacctaagctcacctgcctgtgattcctcatttctcaccatcctgtgccagggtggctacttctctctgtgaggactcaaatacaagccaatgagtggcccactaagcttttaagatttgattttcctgccttgagataaaaaggagtgtaggtaaatgaaagatcaatgtatggaatatataaaaatacgaaagaaatatatacgtttaaaaatccataaagaaaaaaatctcattctaaacctgattaagttggctttttacgtaagtgtacaaataggatattcacagcatctttgtgcagtttttaaacttttatatttaaacattattaagttggcttttgttcacatgttgagtaatgggtagtaaattttctacctcaggagctgatatagacatcagttctgctagccatatcacatattttaatgtttcatcaacatcagctgtttttttgtttgctacactatttgaactaatagacagtggatcatgtaacacaaaattgtcttcaactttaacaaaattgtcattgttatttttttttgagacagagtctccctctgttgcccaggctggagtgcagtggcgcaatctcggctcactgcaacctcgcctgctgggttcaagcagttctcccacctcagcctcccaagtagctgggattataggtgtgcaccaccagacccggctaatttttgtatttttagtagagacggggtttcaccatgttggccaggctggtctcaaactactgacctcaggtgatccacccaccttggcctcccaaagtgctgagataacaggcgtgagccaccgcacccacccaacaaaattatttttaactgtcgtttctgaactgaacctctcacattggcatcttgatttattggtacttaacagtatatatggattttgaactctacacaagggtataaccagaatgaattgaggggtatcaagaaccagattggttacagtagaactctgtaagatgatgtggagagtaaggaaaaggagaagaaataaaaattagtttaagatggaataaagatttgggctgctaattttttcccaggattcaaaatatacccgctagaatggaaaacaaaaatttgaatgattacaacattatcgttaacattcaattttgtatttattgttttattgaatatagttcagagtatattaaaatagacctaccacttcaaatgataatgattattataatgtctcttcaccctattctagcacttctgcttgcagtatgtggtttctatttttttcctcttgtataattccacttgcttttaattgttgtttcattatataaaaggaacatcttcccatagcatattctatgaaaggggtttcattccaagttgagttttcaaaaaaaaggtcttcctaaagctaccattttcaaccgtccttgttatctagtacaacataaataacagtcttaaaaattgcactaataccagtgcccccctggctctccaaatctgttctttgctcttgtatctgctggacgcttgaagacaggtgcactgtctcgtatgtatttgaattatgaacagtaatttctaatgaattctaaaatggtcattgtaagtgaaagcctctcgctaccacttcctcttccaactacataaatatatttcaatgtatttccagttttggaaagttttcaatacatacatcaagtgtttacttagatttttataaaaattttttttacaatctaataatctttggtaaaggaactagagatgcatgcagttgcaaaattaatgtatttattttccagcataattttattaacttcactttttttctctctagtaaatatccagtgtacttatgaactcatgtttggctcttttaaaaccttttctaaaagctagatcagcatttttctattttacaagttttttgtataaaaaggtgaacatatgagatattgtgagaaatcattttaagtttcatttaaatcatggtgcctcttttgatactttcttaaaattgtgcaagaagaaatcatttttagtagtggtcataaatattatccttttggcagtaagctattactaattcagcctgaagctcggtagacaatatgtctacatgtgtttgagtacatcctggatacagtttcccagctcatgagggactgaaaatagtcttattcatcaacccactaggatgtgaagggttaagtctagatttggtcgcattgaaaccccacaatatagaattaataaatggccttcagtaggaaaacctacactaaagcaaatccgaagaagtggggcagggggaaagaggcattactggtctttccttttgttttgcaagcataatttgattttcctttggctcagaaaactcatttggggaaattctcttttgtgttcagtttaacctagaaaggtcctcttgaaaaaccaacattttaggaaagttcttttttcaggatggagtatattaaaattaagccaggctttgacgtgaattatcacttttctttattattttgttttctattttggtttatagctatttctggttcagttctgaacttcagcacttaatcatccttatcaaccaggcttttggtagcctaaaccgctatgctgttgtttttttaatttaaagatgtataagccaaaatttggatgggagtgagacataactgatttatatgaattttaacagagttgtatttgtgtgtgtttaataaaatatatatttattcagtactttcctcagtattttatgggcaaagtaaaaataacaatgcatagtgaaagggcatatattaccagcagtaataattcaaaatcctgaaaatgtttcattttttttgtttttgttatgcagaataaacaaggcagaaatgctctttgaaccactaaaa

SEQ ID NO: 24 - protein, 916 aa, Homo sapiens
MESGQPARRIAMAPLLEYERQLVLELLDTDGLVVCARGLGADRLLYHFLQLHCHPACLVLVLNTQPAEEEYFINQLKIEGVEHLPRRVTNEITSNSRYEVYTQGGVIFATSRILVVDFLTDRIPSDLITGILVYRAHRIIESCQEAFILRLFRQKNKRGFIKAFTDNAVAFDTGFCHVERVMRNLFVRKLYLWPRFHVAVNSFLEQHKPEVVEIHVSMTPTMLAIQTAILDILNACLKELKCHNPSLEVEDLSLENAIGKPFDKTIRHYLDPLWHQLGAKTKSLVQDLKILRTLLQYLSQYDCVTFLNLLESLRATEKAFGQNSGWLFLDSSTSMFINARARVYHLPDAKMSKKEKISEKMEIKEGEETKKELVLESNPKWEALTEVLKEIEAENKESEALGGPGQVLICASDDRTCSQLRDYITLGAEAFLLRLYRKTFEKDSKAEEVWMKFRKEDSSKRIRKSHKRPKDPQNKERASTKERTLKKKKRKLTLTQMVGKPEELEEEGDVEEGYRREISSSPESCPEEIKHEEFDVNLSSDAAFGILKEPLTIIHPLLGCSDPYALTRVLHEVEPRYVVLYDAELTFVRQLEIYRASRPGKPLRVYFLIYGGSTEEQRYLTALRKEKEAFEKLIREKASMVVPEEREGRDETNLDLVRGTASADVSTDTRKAGGQEQNGTQQSIVVDMREFRSELPSLIHRRGIDIEPVTLEVGDYILTPEMCVERKSISDLIGSLNNGRLYSQCISMSRYYKRPVLLIEFDPSKPFSLTSRGALFQEISSNDISSKLTLLTLHFPRLRILWCPSPHATAELFEELKQSKPQPDAATALAITADSETLPESEKYNPGPQDFLLKMPGVNAKNCRSLMHHVKNIAELAALSQDELTSILGNAANAKQLYDFIHTSFAEVVSKGKGKK

SEQ ID NO: 25 - DNA, 4091 bp, Homo sapiens
atttttcatgggtttgcggacccaccagcgaaggcgggaggtgtcgcagggacatcttctggctgtttccgtcgcctgcgtggcccttgcaccccggtcttccattagcggcgcagacgtttgggcctaagcgctgggcgaggcgaggccctgcccctccccgccaacggccattctctggacctgtctttcttccgggaggcggtgacagctgctgagacgtgttgcagccagagtctctccgctttaatgcgctcccattagtgccgtcccccactggaaaaccgtggcttctgtattatttgccatctttgttgtgtaggagcagggagggcttcctcccggggtcctaggcggcggtgcagtccgtcgtagaagaattagagtagaagttgtcggggtccgctcttaggacgcagccgcctcatgggggtccaggggctctggaagctgctggagtgctccgggcggcaggtcagccccgaagcgctggaagggaagatcctggctgttgatattagcatttggttaaaccaagcacttaaaggagtccgggatcgccatgggaactcaatagaaaatcctcatcttctcactttgtttcatcggctctgcaaactcttattttttcgaattcgtcctatttttgtgtttgatggggatgctccactattgaagaaacagactttggtgaagagaaggcagagaaaggacttagcgtccagtgactccaggaaaacgacagagaagcttctgaaaacatttttgaaaagacaagccatcaaaactgccttcagaagcaaaagagatgaagcactacccagtcttacccaagttcgaagagaaaacgacctctatgttttgcctcctttacaagaggaagaaaaacacagttcagaagaggaagatgaaaaagaatggcaagaaagaatgaatcaaaaacaagcattacaggaagagttctttcataatcctcaagcgatagatattgagtctgaggacttcagcagcctgccccctgaagtaaagcatgaaatcttgactgatatgaaagagttcaccaagcgcagaagaacattatttgaagcaatgccagaggagtctgatgacttttcacagtaccaactcaaaggcttgcttaaaaagaactatctgaaccagcatatagaacatgtccaaaaggaaatgaatcagcaacattcaggacacatccgaaggcagtatgaagatgaagggggctttctgaaggaggtagagtcaaggagagtggtctctgaagacacttcacattacatcttgataaaaggtattcaagctaagacagttgcagaagtggattcagagtctcttccttcttccagcaaaatgcacggcatgtcttttgacgtgaagtcatctccatgtgaaaaactgaagacagagaaagagcctgatgctacccctccttctccaagaactttactagctatgcaagctgccctgctgggaagtagctcagaagaggagctggagagtgaaaatcgaaggcaggcccgtgggaggaacgcacctgctgctgtagacgaaggctccatatcaccccggactctttcagccattaagagagctcttgacgatgacgaagatgtaaaagtgtgtgctggggatgatgtgcagacgggagggccaggagcagaagaaatgcgtataaacagctccaccgagaacagtgatgaaggacttaaagtgagagatggaaaaggaataccgtttactgcaacacttgcgtcatctagtgtgaactctgcagaggagcacgtagccagcactaatgaggggagagagcccacagactcagttccaaaagaacaaatgtcacttgttcacgtggggactgaagcctttccgataagtgatgagtctatgattaaggacagaaaagatcggctgcctctggagagtgcagtggttagacatagtgacgcacctgggctcccgaatggaagggaactgacaccggcatctccaacttgtacaaattctgtgtcaaagaatgaaacacatgctgaagtgcttgagcagcagaacgaactttgcccatatgagagtaaattcgattcttctcttctttcaagtgatgatgaaacaaaatgtaaaccgaattctgcttctgaagtcattggccctgtcagtttgcaagaaacaagtagcatagtaagtgtcccttcagaggcagtagataatgtggaaaatgtggtgtcatttaatgctaaagagcatgagaattttctggaaaccatccaagaacagcagaccactgaatctgcaggccaggatttaatttccattccaaaggccgtggaaccaatggaaattgactcggaagaaagtgaatctgatggaagtttcattgaagtgcaaagtgtgattagtgatgaggaacttcaagcagaattccctgaaacttccaaacctccctcagaacaaggcgaagaggaactggtaggaactagggagggagaagcccctgctgagtccgagagcctcctgagggacaactctgagagggacgacgtggatggtgagccacaggaagctgagaaagatgcggaagattcgctccatgaatggcaagatattaatttggaggagttggaaactctggagagcaacctcttagcacagcagaattcactgaaagctcaaaaacagcagcaagaacggatcgctgctactgtcaccggacagatgttcctggaaagccaggaactcctgcgcctgttcggcattccctacatccaggctcccatggaagcagaggcgcagtgcgccatcctggacctgactgatcagacttccggaaccatcactgatgacagtgatatctggctgtttggagcgcggcatgtctatagaaacttttttaataaaaacaagtttgtagaatattatcaatatgtggactttcacaatcaattgggattggaccggaataagttaataaatttggcttatttgcttggaagtgattataccgaaggaataccaactgtgggttgtgtaaccgccatggaaattctcaatgaattccctgggcatggcctggaacctctcctaaaattctcagaatggtggcatgaagctcaaaaaaatccaaagataagacctaatcctcatgacaccaaagtgaaaaaaaaattacggacattgcaactcacccctggctttcctaacccagctgttgccgaggcctacctcaaacccgtggtggatgactcgaagggatcctttctgtgggggaaacctgatctcgacaaaattagagaattttgtcagcggtatttcggctggaacagaacgaagacagatgaatctctgtttcctgtattaaagcaactcgatgcccagcagacacagctccgaattgattccttctttagattagcacaacaggagaaagaagatgctaaacgtattaagagccagagactaaacagagctgtgacatgtatgctaaggaaagagaaagaagcagcagccagcgaaatagaagcagtttctgttgccatggagaaagaatttgagctacttgataaggcaaaacgaaaaacccagaagagaggcataacaaataccttagaagagtcatcaagcctgaaaagaaagaggctttcagattctaaacgaaagaatacatgcggtggatttttgggggagacctgcctctcagaatcatctgatggatcttcaagtgaagatgctgaaagttcatctttaatgaatgtacaaaggagaacagctgcgaaagagccaaaaaccagtgcttcagattcgcagaactcagtgaaggaagctcccgtgaagaatggaggtgcgaccaccagcagctctagtgatagtgatgacgatggagggaaagagaagatggtcctcgtgaccgccagatctgtgtttgggaagaaaagaaggaaactaagacgtgcgaggggaagaaaaaggaaaacctaattaaaaaatatgtatcctctataattagttatgacagccatttgtaatgaatttgtcgcaaagacgtaataaaattaactggtggcacggtctttgtaaaaaaa

SEQ ID NO: 26 - protein, 1186 aa, Homo sapiens
MGVQGLWKLLECSGRQVSPEALEGKILAVDISIWLNQALKGVRDRHGNSIENPHLLTLFHRLCKLLFFRIRPIFVFDGDAPLLKKQTLVKRRQRKDLASSDSRKTTEKLLKTFLKRQAIKTAFRSKRDEALPSLTQVRRENDLYVLPPLQEEEKHSSEEEDEKEWQERMNQKQALQEEFFHNPQAIDIESEDFSSLPPEVKHEILTDMKEFTKRRRTLFEAMPEESDDFSQYQLKGLLKKNYLNQHIEHVQKEMNQQHSGHIRRQYEDEGGFLKEVESRRVVSEDTSHYILIKGIQAKTVAEVDSESLPSSSKMHGMSFDVKSSPCEKLKTEKEPDATPPSPRTLLAMQAALLGSSSEEELESENRRQARGRNAPAAVDEGSISPRTLSAIKRALDDDEDVKVCAGDDVQTGGPGAEEMRINSSTENSDEGLKVRDGKGIPFTATLASSSVNSAEEHVASTNEGREPTDSVPKEQMSLVHVGTEAFPISDESMIKDRKDRLPLESAVVRHSDAPGLPNGRELTPASPTCTNSVSKNETHAEVLEQQNELCPYESKFDSSLLSSDDETKCKPNSASEVIGPVSLQETSSIVSVPSEAVDNVENVVSFNAKEHENFLETIQEQQTTESAGQDLISIPKAVEPMEIDSEESESDGSFIEVQSVISDEELQAEFPETSKPPSEQGEEELVGTREGEAPAESESLLRDNSERDDVDGEPQEAEKDAEDSLHEWQDINLEELETLESNLLAQQNSLKAQKQQQERIAATVTGQMFLESQELLRLFGIPYIQAPMEAEAQCAILDLTDQTSGTITDDSDIWLFGARHVYRNFFNKNKFVEYYQYVDFHNQLGLDRNKLINLAYLLGSDYTEGIPTVGCVTAMEILNEFPGHGLEPLLKFSEWWHEAQKNPKIRPNPHDTKVKKKLRTLQLTPGFPNPAVAEAYLKPVVDDSKGSFLWGKPDLDKIREFCQRYFGWNRTKTDESLFPVLKQLDAQQTQLRIDSFFRLAQQEKEDAKRIKSQRLNRAVTCMLRKEKEAAASEIEAVSVAMEKEFELLDKAKRKTQKRGITNTLEESSSLKRKRLSDSKRKNTCGGFLGETCLSESSDGSSSEDAESSSLMNVQRRTAAKEPKTSASDSQNSVKEAPVKNGGATTSSSSDSDDDGGKEKMVLVTARSVFGKKRRKLRRARGRKRKT

SEQ ID NO: 27 - DNA, 2492 bp, Homo sapiens
cactcagaaaggccgctgggtgcggggagcgcagaggcggtgcagggcggctggctcgcctcggcgtgcagtgcgcgtgcgtggagctgggagctaggtcctcggagtgggccagagatggcggcggccgacggggctttgccggaggcggcggctttagagcaacccgcggagctgcctgcctcggtgcgggcgagtatcgagcggaagcggcagcgggcactgatgctgcgccaggcccggctggctgcccggccctactcggcgacggcggctgcggctactggaggtttgggccgcgtccgcgctttccccttccctctccccgcctccccggtccccagactggctcgtgcaagccgagtcccggggcccgggggtcgcgtcaactccgctggcgtatgtgtgcagattctccccgagtcggagagggaatccgcccagccagccgccttgtcaaagcgtcctgtccacgaccacagagcgttcctctgtcgcacgcgggcctcctgacccccagccccgggccttcttcgctgcacctcggctgctggcagcttcgatttttcgtttagggatgcagccgccccggccgggaggtgtcagccactgccaggtgtcagggcctcagctgtcccggaaagaggagttagactagttcttgattctggcctctatacctagaactagttgatggaagaggcagatcttggtgtttgttagggagagctttcaacaattagagttgccaaaagtgcaatggattgcttctcatgagcttcccgttactagaagcgctcaaataggaactggaagaacgcttacttatgtggaggagaggagattcagcaatcagaatctcctactcagcaatcagaagaagggactggatagtaaacctttaagattctaatccatagattccatgagtctatttcttggacatgtgacctctgcgatttcttggcaaaaactagttgctcaaaacgtgtttattgattgaagtaaattaaggactgatctctcattgcagattattctcttatagaatttgccactggggtcaactaataatctttaacaggatacttaaaatatagtttggttgacaggcagttcttcagggctgcctctataacatgaagtacatgtgttcctaaagctctatactgccctttgtcgagcacagtttagagctgtattactcttttttatcagccagatgtagtgagagtgagaagagtctgaggctggcagcatgtcttgatgttcatactaacaccgaaactgcaaattccagctacttttgatggcatggctaatgtaaaagcagccccaaagataattgacacaggaggaggcttcattttagaagaggaagaagaagaagaacagaaaattggaaaagttgttcatcaaccaggacctgttatggaatttgattatgtaatatgcgaagaatgtgggaaagaatttatggattcttatcttatgaaccactttgatttgccaacttgtgataactgcagagatgctgatgataaacacaagcttataaccaaaacagaggcaaaacaagaatatcttctgaaagactgtgatttagaaaaaagagagccacctcttaaatttattgtgaagaagaatccacatcattcacaatggggtgatatgaaactctacttaaagttacagattgtgaagaggtctcttgaagtttggggtagtcaagaagcattagaagaagcaaaggaagtccgacaggaaaaccgagaaaaaatgaaacagaagaaatttgataaaaaagtaaaagaattgcggcgagcagtaagaagcagcgtgtggaaaagggagacgattgttcatcaacatgagtatggaccagaagaaaacctagaagatgacatgtaccgtaagacttgtactatgtgtggccatgaactgacatatgaaaaaatgtgattttttagttcagtgacctgttttatagaattttatatttaaataaaggaaatttagattggtccttttcaaaattcaaaaaaaaaagcaacatcttcatagatgaatgaaacccttgtataagtaatacttcagtaataattatgtatgttatggcttaaaagcaagtttcagtgaaggtcacctggcctggttgtgtgcacaatgtcatgtctgtgattgccttcttacaacagagatgggagctgagtgctagagtaggtgcagaagtggtaggtcagctacaaatttgaggacaagataccaaggcaaaccctagattggggtagagggaaaagggttcaacaaaggctgaactggattcttaaccaagaaacaaataatagcaatggtggtgcaccactgtaccccaggttctagtcatgtgttttttaggacgatttctgtctccacgatggtggaaacagtggggaactactgctggaaaaagccctaatagcagaaataaacattgagttgtacgagtctga

SEQ ID NO: 28 - protein, 273 aa, Homo sapiens
MAAADGALPEAAALEQPAELPASVRASIERKRQRALMLRQARLAARPYSATAAAATGGMANVKAAPKIIDTGGGFILEEEEEEEQKIGKVVHQPGPVMEFDYVICEECGKEFMDSYLMNHFDLPTCDNCRDADDKHKLITKTEAKQEYLLKDCDLEKREPPLKFIVKKNPHHSQWGDMKLYLKLQIVKRSLEVWGSQEALEEAKEVRQENREKMKQKKFDKKVKELRRAVRSSVWKRETIVHQHEYGPEENLEDDMYRKTCTMCGHELTYEKM

SEQ ID NO: 29 - DNA, 5739 bp, Homo sapiens
gacgtaatgcggtagcgcggggaatttcgagtggtgttggagcgccggaggctagtgggtggctgacccccagcatcctcgggagcgaccatggactccctggccgagtctcggtggcctccgggcctggcagtcatgaagacaatagatgatttgctgcggtgtggaatttgcttcgagtatttcaacattgcaatgataatacctcagtgttcacataactactgctctctctgtataagaaaatttctgtcctataaaactcagtgtccaacttgctgtgtgactgtcacagagccggatctgaaaaataaccgcatattagatgaactggtaaaaagcttgaattttgcacggaatcatctgctgcagtttgctttagagtcaccagccaaatctcctgcttcttcctcttcaaagaatcttgctgtcaaagtatatactcctgtagcctccagacagtctttaaagcaggggagcaggttaatggataatttcttgatcagagaaatgagtggttctacatcagagttgttgataaaagaaaataaaagcaaattcagccctcaaaaagaggcgagccctgctgcaaagaccaaagagacacgttctgtagaagagatcgctccagatccctcagaggctaagcgtcctgagccaccctcgacatccactttgaaacaagttactaaagtggattgtcctgtttgcggggttaacattccagaaagtcacattaataagcatttagacagctgtttatcacgcgaagagaagaaggaaagcctcagaagttctgttcacaaaaggaagccgctgcccaaaactgtatataatttgctctctgatcgtgatttaaagaaaaagctaaaagagcatggattatctattcaaggaaataaacaacagctcattaaaaggcaccaagaatttgtacacatgtacaatgcccaatgcgatgctttgcatcctaaatcagctgctgaaatagttcgagaaatcgaaaatatagagaagactaggatgcgtcttgaagctagtaaactcaatgaaagtgtaatggtttttacaaaggaccaaacagaaaaggaaatagatgaaatccacagtaaatatcgtaaaaaacataagagtgaatttcagcttctggtggatcaggctagaaaaggatacaagaaaattgctggaatgtcacaaaaaacagtaacaataacaaaagaagatgaatctacagaaaagctatcttctgtatgcatgggacaggaagataatatgacctcagtaacaaaccacttttctcaatcaaagctggactccccagaggaattggaacctgacagagaagaggattcttctagctgtattgatattcaagaagttctttcttcatcagaatcagattcatgcaatagttccagttcagacatcataagagatcttttagaagaagaggaagcctgggaagcatcacataaaaacgatcttcaagacacagaaataagtccaagacagaatcgccgcacaagagccgctgaaagtgctgagattgaaccaagaaacaagcgtaataggaattaatgtgggcttttgctgacttttcaaatgcattgattagaataccgtacttttggttgccacagatagattttctatttataaatgcccaaggaaagatgctaaattctaaatattacggttagctgatattcattcttttctgcttttccagaggggaaaaatgttacaaaatatccttacttggtcagttgcctcctgcctctaaaacatctctctctaaaaatactgacatttcacacaggtaccagctttgcagaggaggtagactctttggcactttggcacagggatttggtttggtttggtttggtttgataattaaatttcagaatgtccttaggccattctccttctcttccatggagaatccagcctcacaaaaggattctttcaacttctttattgcaagaaacagttgagttaaatgtttgtttttggaaaggcgggatgtcagttcacatccttggtgtgtgtaagtaccgatgcacgccaccaccatgcctgtgttacagcagctccatgatggttgttgcccgaggttaatgtagttgtttgttagacctgtgtcttacacatttctcagagtaggatattagtattataatttaaagctacgacagtcacaaagtcacaataacttagaaacattgcgcatattcttctgaaatagcacttaaaaatgattagtgtcagtattttttcacttgggtcaatcaaatctgtaacactgaatccaagctattaaacaaaaagtatgcaatgaatgaattttgtaaatgaatagagagtatcagtttacaataatgttcttaaaacagtatcctctggatagttgagtatgggttagaaatcattgaaatggattggtcagaaattgctatctgtgtaaaatgtctaccagtagccagatgcttccagagttcttaatgcctctctggcatttcagagccagcatcccccaactcccacccctctgccatcacccaacccaaacacatcagctttcaaatgagatgatagtaaatgcggcaatgttaagacaagaaatttatgatttgccagattcaacatttatgacctccccttccaaagactgtctccgttgaccttgtctttttggtatgccttggggtttctgataatgtgtggagtctcattatggctgagagtttagtgttttcacagtgaagtgcagacatttgatttctttatgagttccctgtgttagaaatggctatagaaaaatttgtcataataatttcatttgcatgaaatcctgaggggtgcattaaggaaactaaaagcaccacttaccaaatctatcggcagaactgatgtgaggtaagtgagcatgtcaaacaaaataggagctcacatggatatatttatgtcactgagttgtcagaaattatgtcaaaatgaaaactgtttgtttcatgacaaattatatagtctataaattaaactggaagtaattattactttaattgcagcaaaaggagtttgtgagggagcggtgagacccaagattgggaaagtaggcacatgagttcattcagcaaatatttggttatctatgtctgtcactgtgctgacactgggaatacaaaggtggccaaagatcatctagaacaatggttcccagtggggtgggcagaaagattttgccccccaggagacagctggcaatgtgtggagacacttttggaggtggagggtggtgaggggtactaccagtatcaatgggtggaggccagggatgaggctaaacacccaaccctcatggattagtttgccagggctgccgtcacaagatactgcagacggggaagcttacacaacagaaatgtgtattctcagaattctggaggctggaagtccaagatcagtagggtttcttcttcggcctctctccttggcttccactcatggtgtccttgcatggtcttttctctgtgtgcacatgactgtgcaggactggtgtcccgatttcttgtagggacagcagtcattggatcagggcccatgcgtatggcctcattttacttcagttacctcttttttagatagagggccctatctctaaatactgtcacattctgagataccggcagttaagacttccaacatatttagtggtaggggttaaggggcacgctttagactacaacactccacagtaaagaattatccagtctaacatgtcagttgtgccaagactgagaaacctgtaatgtaaaggaactcccaagtctacctgaaaagtaaggtctaaagagcatttattgagcactatctgttagcacttagcatatgtttaatattcatacattgaaagaaatgtatgttcatatccatctgacaaagattaaggaacttagagtaagtaatagatccaaaattgaaactgataaacttctggttctaaaattcaccttttagtgaaaatacagtttctcaccaaacttacagtaattcagagttattaactctttctacctcctcactcccctcaaagttataacatctcccatcaacatcagctcagaatggcagtgatgcttatggtttgtgggggtgcaggtgagctgctggatgcactttagatggcctagtatgccaggccgtcctttcatcctctactctcgtctttctttttcgacctcatgttgaggattactggtctagttgaaaaaagaattcatacacataagaccatgtatataatagagggaggtatgcctttaaaaacaaaattacatggtaaagactgatgtgtcaacagggatagacaacatagagaaggctagaactgtttctggaaaaaaacccaaaaacaatggatttcaaacttcttagcatccgataaaagaaagtagcaattattcaaatgagaaacacttctgtctgttatgtacatattatgaaagtatgaacataagagggaaaaccacaaccattacattttttaccatttcagtaatttttttttggtttttagtctgtttttagacatccttaagaacaactatctgaggctgtaaacaagtatttacattaacacccatgatactgactttatactccctacctgcattgagaccttaaagggggcatttctccattccttctgtgtatttctgggtatccccaggttcagatattcagaatacagatacaagtccatgcttgcatatgttgctgctccccccgacagacttctaccagcatctgccctcctcaccgctgctctgtcacgtgcactgcggctggccctgctggaaagtcctaccttgcctaggacgccatccccgatatagccccaagatgcaaacctgccaagtgctagggcagccctgccttcctgtccatttcagtctcttggccttgctgtgttccaagtggaaatgggagtgtgctttcctggtttgctagtgtactatcacccggaccacagcgtcctgtgcaaaaatttgcttcctctctcttcccctttcactctttctcttttctcttccccacccccttttttttctctttccccttacctttctttcctttccactcttcctgtccttccttccttcaactattaggactatatgtcaagtaatgtgcaaaacaaagacagttcctgccctgatggagcttgtagatcagaagggaagatgagcattaagtaattatatagattaatgtacaactgtgatgagtgcaacaaaagagaggttcatggcactatcaaacatgcaatggacggattttgtttttgcctataaactcttgccatagaaagcttgaaaatcagtccagggggacagcattaatcaccatgttctttccttatccctgtcttccccaaaattcatgtgttgaaacttaacaagaggtgggaactttaggatgtgattaagtcgtgagggcacagctcttatagatggggtcacggtccttctaaaagggcttgagggagtggttttgtttccttccatcccttccgccacatgaggacacagtcttcgttccctctggaggactcagcaacaacacaccatcttggaagcagagagcagtcctcaccagacacggaatctgccagtgccttgatcttggacttaccagcctccatacctgtgagaaataaatttctattgtctataa

SEQ ID NO: 30 - protein, 495 aa, Homo sapiens
MDSLAESRWPPGLAVMKTIDDLLRCGICFEYFNIAMIIPQCSHNYCSLCIRKFLSYKTQCPTCCVTVTEPDLKNNRILDELVKSLNFARNHLLQFALESPAKSPASSSSKNLAVKVYTPVASRQSLKQGSRLMDNFLIREMSGSTSELLIKENKSKFSPQKEASPAAKTKETRSVEEIAPDPSEAKRPEPPSTSTLKQVTKVDCPVCGVNIPESHINKHLDSCLSREEKKESLRSSVHKRKPLPKTVYNLLSDRDLKKKLKEHGLSIQGNKQQLIKRHQEFVHMYNAQCDALHPKSAAEIVREIENIEKTRMRLEASKLNESVMVFTKDQTEKEIDEIHSKYRKKHKSEFQLLVDQARKGYKKIAGMSQKTVTITKEDESTEKLSSVCMGQEDNMTSVTNHFSQSKLDSPEELEPDREEDSSSCIDIQEVLSSSESDSCNSSSSDIIRDLLEEEEAWEASHKNDLQDTEISPRQNRRTRAAESAEIEPRNKRNRN

SEQ ID NO: 31 - DNA, 4263 bp, Homo sapiens
ctctccacggcgcacagagcatgcgcggggcgggagtgagcgaaattcaagctccaaactctaagctccaagctccaagctccaagctccaagctccaaactcccgccggggtaactggaacccaatccgagggtcatggaggcatcccgaaggtttccggaagccgaggccttgagcccagagcaggctgctcattacctaagatatgtgaaagaggccaaagaagcaactaagaatggagacctggaagaagcatttaaacttttcaatttggcaaaggacatttttcccaatgaaaaagtgctgagcagaatccaaaaaatacaggaagccttggaggagttggcagaacagggagatgatgaatttacagatgtgtgcaactctggcttgctactttatcgagaactgcacaaccaactctttgagcaccagaaggaaggcatagctttcctctatagcctgtatagggatggaagaaaaggtggtatattggctgatgatatgggattagggaagactgttcaaatcattgctttcctttccggtatgtttgatgcatcacttgtgaatcatgtgctgctgatcatgccaaccaatcttattaacacatgggtaaaagaattcatcaagtggactccaggaatgagagtcaaaacctttcatggtcctagcaaggatgaacggaccagaaacctcaatcggattcagcaaaggaatggtgttattatcactacataccaaatgttaatcaataactggcagcaactttcaagctttaggggccaagagtttgtgtgggactatgtcatcctcgatgaagcacataaaataaaaacctcatctactaagtcagcaatatgtgctcgtgctattcctgcaagtaatcgcctcctcctcacaggaaccccaatccagaataatttacaagaactatggtccctatttgattttgcttgtcaagggtccctgctgggaacattaaaaacttttaagatggagtatgaaaatcctattactagagcaagagagaaggatgctaccccaggagaaaaagccttgggatttaaaatatctgaaaacttaatggcaatcataaaaccctattttctcaggaggactaaagaagacgtacagaagaaaaagtcaagcaacccagaggccagacttaatgaaaagaatccagatgttgatgccatttgtgaaatgccttccctttccaggaaaaatgatttaattatttggatacgacttgtgcctttacaagaagaaatatacaggaaatttgtgtctttagatcatatcaaggagttgctaatggagacgcgctcacctttggctgagctaggtgtcttaaagaagctgtgtgatcatcctaggctgctgtctgcacgggcttgttgtttgctaaatcttgggacattctctgctcaagatggaaatgagggggaagattccccagatgtggaccatattgatcaagtaactgatgacacattgatggaagaatctggaaaaatgatattcctaatggacctacttaagaggctgcgagatgagggacatcaaactctggtgttttctcaatcgaggcaaattctaaacatcattgaacgcctcttaaagaataggcactttaagacattgcgaatcgatgggacagttactcatcttttggaacgagaaaaaagaattaacttattccagcaaaataaagattactctgtttttctgcttaccactcaagtaggtggtgtcggtttaacattaactgcagcaactagagtggtcatttttgaccctagctggaatcctgcaactgatgctcaagctgtggatagagtttaccgaattggacaaaaagagaatgttgtggtttataggctaatcacttgtgggactgtagaggaaaaaatatacagaagacaggttttcaaggactcattaataagacaaactactggtgaaaaaaagaaccctttccgatattttagtaaacaagaattaagagagctctttacaatcgaggatcttcagaactctgtaacccagctgcagcttcagtctttgcatgctgctcagaggaaatctgatataaaactagatgaacatattgcctacctgcagtctttggggatagctggaatctcagaccatgatttgatgtacacatgtgatctgtctgttaaagaagagcttgatgtggtagaagaatctcactatattcaacaaagggttcagaaagctcaattcctcgttgaattcgagtctcaaaataaagagttcctgatggaacaacaaagaactagaaatgagggggcctggctaagagaacctgtatttccttcttcaacaaagaagaaatgccctaaattgaataaaccacagcctcagccttcacctcttctaagtactcatcatactcaggaagaagatatcagttccaaaatggcaagtgtagtcattgatgatctgcccaaagagggtgagaaacaagatctctccagtataaaggtgaatgttaccaccttgcaagatggtaaaggtacaggtagtgctgactctatagctactttaccaaaggggtttggaagtgtagaagaactttgtactaactcttcattgggaatggaaaaaagctttgcaactaaaaatgaagctgtacaaaaagagacattacaagaggggcctaagcaagaggcactgcaagaggatcctctggaaagttttaattatgtacttagcaaatcaaccaaagctgatattgggccaaatttagatcaactaaaggatgatgagattttacgtcattgcaatccttggcccattatttccataacaaatgaaagtcaaaatgcagaatcaaatgtatccattattgaaatagctgatgacctttcagcatcccatagtgcactgcaggatgctcaagcaagtgaggccaagttggaagaggaaccttcagcatcttcaccacagtatgcatgtgatttcaatcttttcttggaagactcagcagacaacagacaaaatttttccagtcagtctttagagcatgttgagaaagaaaatagcttgtgtggctctgcacctaattccagagcagggtttgtgcatagcaaaacatgtctcagttgggagttttctgagaaagacgatgaaccagaagaagtagtagttaaagcaaaaatcagaagtaaagctagaaggattgtttcagatggcgaagatgaagatgattcttttaaagatacctcaagcataaatccattcaacacatctctctttcaattctcatctgtgaaacaatttgatgcttcaactcccaaaaatgacatcagtccaccaggaaggttcttttcatctcaaatacccagtagtgtaaataagtctatgaactctagaagatctctggcttctaggaggtctcttattaatatggttttagaccacgtggaggacatggaggaaagacttgacgacagcagtgaagcaaagggtcctgaagattatccagaagaaggggtggaggaaagcagtggcgaagcctccaagtatacagaagaggatccttccggagaaacactgtcttcagaaaacaagtccagctggttaatgacgtctaagcctagtgctctagctcaagagacctctcttggtgcccctgagcctttgtctggtgaacagttggttggttctccccaggataaggcggcagaggctacaaatgactatgagactcttgtaaagcgtggaaaagaactaaaagagtgtggaaaaatccaggaggccctaaactgcttagttaaagcgcttgacataaaaagtgcagatcctgaagttatgctcttgactttaagtttgtataagcaacttaataacaattgagaatgtaacctgtttattgtattttaaagtgaaactgaatatgagggaatttttgttcccataattggattctttgggaacatgaagcattcaggcttaaggcaagaaagatctcaaaaagcaacttctgccctgcaacgccccccactccatagtctggtattctgagcactagcttaatatttcttcacttgaatattcttatattttaggcatattctataaatttaactgtgttgtttcttggaaagttttgtaaaattattctggtcattcttaattttactctgaaagtgatcatctttgtatataacagttcagataagaaaattaaagttacttttctcaagtgttttccaaaaaaaaaaaaaaaa

SEQ ID NO: 32 - protein, 1250 aa, Homo sapiens
MEASRRFPEAEALSPEQAAHYLRYVKEAKEATKNGDLEEAFKLFNLAKDIFPNEKVLSRIQKIQEALEELAEQGDDEFTDVCNSGLLLYRELHNQLFEHQKEGIAFLYSLYRDGRKGGILADDMGLGKTVQIIAFLSGMFDASLVNHVLLIMPTNLINTWVKEFIKWTPGMRVKTFHGPSKDERTRNLNRIQQRNGVIITTYQMLINNWQQLSSFRGQEFVWDYVILDEAHKIKTSSTKSAICARAIPASNRLLLTGTPIQNNLQELWSLFDFACQGSLLGTLKTFKMEYENPITRAREKDATPGEKALGFKISENLMAIIKPYFLRRTKEDVQKKKSSNPEARLNEKNPDVDAICEMPSLSRKNDLIIWIRLVPLQEEIYRKFVSLDHIKELLMETRSPLAELGVLKKLCDHPRLLSARACCLLNLGTFSAQDGNEGEDSPDVDHIDQVTDDTLMEESGKMIFLMDLLKRLRDEGHQTLVFSQSRQILNIIERLLKNRHFKTLRIDGTVTHLLEREKRINLFQQNKDYSVFLLTTQVGGVGLTLTAATRVVIFDPSWNPATDAQAVDRVYRIGQKENVVVYRLITCGTVEEKIYRRQVFKDSLIRQTTGEKKNPFRYFSKQELRELFTIEDLQNSVTQLQLQSLHAAQRKSDIKLDEHIAYLQSLGIAGISDHDLMYTCDLSVKEELDVVEESHYIQQRVQKAQFLVEFESQNKEFLMEQQRTRNEGAWLREPVFPSSTKKKCPKLNKPQPQPSPLLSTHHTQEEDISSKMASVVIDDLPKEGEKQDLSSIKVNVTTLQDGKGTGSADSIATLPKGFGSVEELCTNSSLGMEKSFATKNEAVQKETLQEGPKQEALQEDPLESFNYVLSKSTKADIGPNLDQLKDDEILRHCNPWPIISITNESQNAESNVSIIEIADDLSASHSALQDAQASEAKLEEEPSASSPQYACDFNLFLEDSADNRQNFSSQSLEHVEKENSLCGSAPNSRAGFVHSKTCLSWEFSEKDDEPEEVVVKAKIRSKARRIVSDGEDEDDSFKDTSSINPFNTSLFQFSSVKQFDASTPKNDISPPGRFFSSQIPSSVNKSMNSRRSLASRRSLINMVLDHVEDMEERLDDSSEAKGPEDYPEEGVEESSGEASKYTEEDPSGETLSSENKSSWLMTSKPSALAQETSLGAPEPLSGEQLVGSPQDKAAEATNDYETLVKRGKELKECGKIQEALNCLVKALDIKSADPEVMLLTLSLYKQLNNN

SEQ ID NO: 33 - DNA, 10324 bp, Homo sapiens
caattcgggagcccgttctcgcgggattttccaagaccgggttggaatttgcgggggttaggagacggaagtcagagcctaggaagatttgggggtcgccttgccggcctcctgtcctcctccggcggcggcggagcccgagagaactaggtgaacaccgctttgccagcctcacacagcgtcccctggctctgccgccgctccggacgtcgccctcccgttctgcttgggtccccttagtcgctacctttgctgggatccccctcctccatcctgtggcttcgggttgccgaagagcgatgctcggagggcggccggaagtggcgttggccgccattggcctgccggccagccaccttgctgtcctccgccgccttccgggtgttacatgcagccgggctcggcccctccccctggccggatggatccgtcggcgccacagccccgcgcggaaacctcaggcaaagacatatggcatccaggagaaagatgtcttgccccttctccagataatggaaaactttgtgaagcaagcataaaatctatcacagtggatgaaaatggcaagtcatttgcagtcgtcttatatgcagattttcaagaaaggaaaatacctcttaaacagcttcaagaagtgaaatttgttaaagattgccctaggaatcttatatttgatgatgaagatttagaaaaaccttatttcccaaaccgaaaatttccatcatcttctgttgcttttaaattatctgacaatggagactctattccttataccatcaataggtatttgagagactaccaaagagaaggaacccggtttctttatggacactacatccatggaggagggtgcattctgggtgatgacatgggacttggaaaaacagtacaggttatttcatttctggctgcagttttgcataaaaagggaactcgtgaggatattgaaaataacatgccagagtttttactaagaagtatgaaaaaggaacccctttcttctacagcaaaaaagatgttcttaatagttgctcctctttctgtcctctacaactggaaggatgaattggacacctggggatatttcagagtcactgttttacatggaaacagaaaagataatgaattaattcgtgtaaagcagaggaaatgtgaaattgctctaacaacttatgaaacactacgcttatgcctggatgaacttaacagtttggaatggtcagctgtcattgtggatgaagctcatagaatcaagaatccaaaagctagagtaacagaagttatgaaagctttgaaatgtaatgtccgcattggcctcactggaaccatccttcagaacaacatgaaggaactgtggtgtgttatggactgggctgtgccaggccttttagggagtgggacctacttcaagaagcagttttctgacccagtagaacatggtcagagacacacggcaacaaagagagaactagccactggccgaaaggccatgcaaagacttgccaaaaagatgtctggctggtttctcaggcgcaccaagactcttatcaaggatcagttgcctaagaaggaagaccggatggtgtattgttctttgacagatttccagaaagctgtctatcaaacagtgttagaaacagaggacgtgactttgatacttcaatcttctgagccttgtacctgtaggagtggccaaaaaaggagaaattgttgttataagaccaattctcatggtgaaacagtgaaaaccttgtatctcagttaccttacagtccttcagaaggtagctaaccatgtcgcgctactgcaagctgctagtacttccaaacaacaggaaacacttatcaaaaggatatgtgatcaggtattttccagattcccagattttgtgcagaaaagcaaagatgcagcctttgaaacactttctgaccctaaatacagtggaaaaatgaaggtccttcagcagcttttaaatcattgcaggaaaaacagagataaagttcttctcttttctttttccaccaagttgcttgacgtgctacagcagtactgtatggcgtctgggcttgattaccgacgacttgatggaagtacaaaatcagaggaaagactcaagattgtaaaagagttcaacagtacacaagatgttaacatttgccttgtctctacaatggctggtggactaggcctcaattttgtcggtgccaatgttgttgtattatttgatcctacttggaatccagccaatgatcttcaagccattgacagagcatataggattggacaatgtagagatgtcaaagtgcttaggctgatatccttgggaactgtggaggaaatcatgtatttacgacagatatacaagcagcaacttcactgtgtggtggttggaagtgaaaatgccaaacgatattttgaagcagttcaaggatctaaagagcatcaaggagagctttttgggatccataacctcttcaaatttaggtcccaagggtcttgtcttacgaaggacatcctggagagagaaggccaagtagaagcagggatcatgacagccacaacatggttgaaagagggacctccagcacacaaactggaaatgcctagacagcctgactgtcaggaatgcagaggtacagaacaagctgcagagccactggcaaaggaagcatgtgatctctgcagtgacttcagtgatgaagagccagtgggagccacaggaataaagactgccaaaaacaaagcacccgattcaagtaaagcttccagctctccaggacagcttaccttactccagtgtggtttctcgaaattgcttgaaacaaaatgtaaagcagttgaggatagtgatggaaatactgcctctgatgatgaaagttctgatgagcagcccacatgcctttcaacagaagccaaagatgctggttgtgagaaaaatcaggactctcttggtacttcaaaacatcagaaattagataacatcctaaatccaaaagaaaagcatattttttataaaagtgagaagattttagaacagaatatttcttccaagtctgacgagaaaaaaattaaaaatacagataaacattgcattttacagaatgtcacagaatcagaagatagtgatgtcatctgtcctacacaatacacaactgagagattccccgacaatagtataaggtttaagccacccttggaaggatctgaggattctgaaacagaacacactgtaaaaacaagaaataatgataatagtcgaaacactgatgacaaaagaaatggaataatttcaaaaaagttaagtcctgagaacacaaccctgaaatctattttgaaaagaaaaggcaccagtgatatcagtgatgaatctgatgacattgaaatttcttccaagtcaagagtaagaaagagagctagttcattgaggtttaagagaataaaagaaaccaaaaaagaacttcacaattctcccaaaacaatgaacaaaacaaaccaagtgtatgcagcaaatgaggatcataactctcagtttattgatgattattcatcctcagatgagagtttatccgtcagccacttcagtttctctaaacagagccacagaccaagaactataagagacagaactagtttttcttcaaaattgcctagccataataagaaaaatagcacttttattccaagaaaaccaatgaaatgttcaaatgagaaagttgttaatcaagagcagtcgtatgaatcaatggataaatttttagatggcgttcaggaagtggcttatattcactcaaaccagaatgtaattggatcgagcaaagctgaaaatcacatgagccgatgggcagcacatgacgtatttgagttgaagcagttttctcagctgcctgctaacatagctgtttgcagttctaagacatataaagaaaaagtggatgcagatacattgccacacacaaagaaaggccagcaaccgagtgaaggcagcatttcacttcctctttacatttcaaatcctgtaaaccagaagaagaaaaaagtctaccatacaaaccagaccaccttcataattggagaaacaccaaaaggaatccgcagaaaacaatttgaagaaatggcctcttattttaactcgtcttctgtaaacgaatttgctaaacatataaccaatgccacatcagaagaacgacagaaaatgctaagagacttttatgcttctcaatatccagaggtaaaagaattttttgtggattctgtgtcacaattcaacaattcttcctttgagaaaggagagcagcgcacccggaagaaatctgataaaagagaatctcttataaaaccaaggctgtcagattctgaaaccttgtcatttaaagattctaccaacaaaatttctcaagtttgcagcctaaaaacatataaaagaaaatcagttaagtttcagaatcatatttcctatagagaagaggtgttttttaatgatgcagaaactaagaaatcacctgttagttctactcaagagattgacagtgggaaaaacagccaggcatccgaagatactgtgacatcccgttctctgaacagtgagtctgaaacacgtgagagaaggttagaaaataccatgaaagaccaacaggacctcacaagaacgggcatttcaagaaaagaaccccttctcaaattggaaaacaaaaagatagaaaatccagtgctggaaaatacttctgtgataagcttacttggtgatacctctattcttgatgacctttttaaaagtcatgggaacagtcccacacaactgccaaagaaagttctttcagggcccatggaaaaagcaaaacagagaccaaaagatttctgggacatcttgaatgagcagaatgatgagagtcttagtaaactcacagacttggcagtaatagagactctgtgtgaaaaagcacctctagcagcaccctttaaaaggagagaagagccagcaacttctctttggaaatcaaatgagaaatttttatggaagaaatttagcccaagtgatacagatgaaaacgcaaccaatacacagagtaccacataagcatataaatgaattactgcaccagtaaactgctgccatcactgtttacggcactggattccacactgattctattatcttgaacacagttgttgacatatatttttattaaattattgctttaggattttttgaagtctaaagtattgtcatggatctgtttttcttgatatttgatttgatctttcaagaatatgattgtatttatagtataaacctctgttatgaattagaaaagattctaggtttgttaataggagacctgggacatctttcttactatattacataatgatgtgacacttgccccggtgagcattgtttcccagtatgaaagatgaagagtctgtaccgaatcagcatgagtgtccttccagtttaaaaaagctttgcttcgctctcctaatggctcataggctgaatcatgtctgcccctcaaatcaggtgtataccaatgtgttttttactagcacttgggaaagttattaagtattttctttttccctgggcatcatgttctattattattttagaaaaaagtcataattggtactgaatatatggtatatataatattaaaatggtaattttgcaacagctcaaaattaaaaggttaatgttatacactttactatatgagctgtgattactaccattagccacagataccagtgcctcaactttttatgtacctattgtgatttaatgtaaataaaggtttgtatagtacttttgtagttcttaagtatgaagaaatgggtaaactttttattttgttagaaactgttatattttgagtgtaatatttatggtttatagcaaaatgaatgtgcttattgttgaatgcatgtatttagaagcctttactcagcccctgtgttctgtgctaggagcttgagctctacaggtaaggcagagctaccggtgaatgaaaggaaatcatgtcagtgaaaaatcatggtggaaagcccctggcatcacatgtgcatgctgtaggcaggacctgagctgcctccgctgcaggttcagatgcaccgctgcagctgtccttcagttagttcacagggctgcaagaggaggacacatccctccagaaaacagcctgagccgggaactggctgtgctaaagagcactgctatcaagttgaggagagagggcttccgtgtactcaggatgtagagtcattgctcagaagtgaacaaaaaatcaaaaacaaaagtcttctcaagggactgatcggccaagtatgcttttctttagagcaatgttttgccctagagaattgtaaaatttatgtcatgactcagtacatatgtgttcgtacatatatgattggaataaaatgtttatgaaatatttactcataagccatgtaacatactttgacatttttctcttctaggattgtgtttggtagggcagtgggtttgtgtgtgtgttaatcctctcacaacccactgaattgaatttcatggcccatggttaagatccacagtgtgaaaacgctgttttaaattatatgagttcgtcatttgtttgctctgtgcagctgagttgtgtccagacttaccagatggtatgttttgccattgaggggccttctacacaatgagtgcatgatatggtccttgatagacttgacttgtagatgttttcagcctacaatgtgatcagctatctgaggaactccagtaagtagataccacttcatttcagtttatatacaagacaatgtagttcaaacattttaataccttgtaaattatgatattcatataaatattagctctatagtcttcatatatgtacagtttttttttttttttttttttttttgagattgagtctcactctgtcacccaggctggagtacagtggcatgatcttggctcactgcaacctccacctccctcccaaacaactcttatgcctcagcctcctgagtagctaggattacaggtgtgtaccaccacactcagctaaacatttttttttttttttgagacggagtctcactctgtcgccaggctggagtgcagtggctcgatcttggctcactgcagcctccgccccccgagtcaagcaattctcctgcctcagcctcccgagtagctgggactacaggtgcgtgccaccacgcccagctaatttttttgtgtttttagtagggatggggtttcaccatgttggccaggctggtctcaatctcctggctgcaagcgatccacctgccttgtcctcccaaagtgctgggattacaggtgtgagccaccatgcccagccaataaatgctattaaagaaacttttaggccgggcacagtggctcacgcctgtaatcccagcactttgggaggccgaggcaggcggatcacaaggtcatgagatcgagactatcctggctaacgcggtgaaaccccgtctctactaaaaaaaaaaaaaatacaaaaattagccaggcgtggtggtgggcgcctgtagtcccagctactcgggaggctgaggcaggagaatggcgtgaacctgggaggcagagcttgcagtgagccaggattgtgcccctgcaccccagcctgggtgacagagcaagactccatctcaaaaaaggaaacttttatcaatagtagtcaaaatgggagcaaaaatgcagaactggagtttaaaaattagtttccaacagttgtcagtgaaatatttatcactattatgtaggaaagtgtgtcaggtggaatgcagagtccagtatgaaaaggagcctgtttcagaacggaaactgtcaggtggagtggactccctgcaatggagtgatggaaagatttggtacaaccattgatgacctgagaacagacactaggaaggtttgacaagatccttcctacccccactccactggtgatgtgtcaccaagttctgctaactaaatgggtggcctcaagcaaatcccttacctccttttagccttagtttcccctttaaattggtgatggattagatcagtggtggtcagccattttcttaaagcaactgaactgtatcttaatcagaaacttaactagtaaaacaattaaaatgcaagtctgttgcttcaagcaacaccactgtggctccatggagcactaatttgaaaaccacagagatgagatcatttctaagaaaacctttcaactttgtttccatgatgctacttgccacaatcttttttacttaagcaatgataccgtttctggctgaacactcaccacacagctattaatattggaaactgaggcaagataccaagagatttttgcacttgaattcctcagggttctcttacagccctgaaaacacctcttcaaggaaataaataacatctgcaaatggtgcagctgcccctaagtattcaaggcaaagaagccttagtttgcagagatgatgataaacttttcatccttccacagaaaatgagaaagccacaggaaatacacggttattttctaattaaagttcaatgtgtacgcttttaaattctgaagttatccttcttttatgatatcaaaatagccctcttttttgaaatgatggtagatcataccttttggtctttttcattgtccttacataaaagttggtaatcatatgtcagtcccagaagttttatttgacacttactggtctataaaatccaaaggaatggggatcactgcctgccttaaaggtttttttgtgtgtttgtttgtttgtttgtttgcatgtgaaggatttttatgtcacaaatccagctaacagtggatctaggatctaggcctcaccgaggatgtcactgaacctgtcagccccaatgacaggcacacaccttcaaagagcaagagtgcccatcactttctaggctccttgcctgctgctcattccatcatcacggatacagacttgtttctggtttcatcttccaccagagattgcaaagcatcctctgcccagtgcttctaggaggccttactgggatggttcataagccactttcctcttggtgacagcccctgtacactgtggcatgtacggctggctccacttggtatttgttgcaggagggaagaacatctcacttttgcttggctaaagggccaccccaggagagctattttgcctcagggtcttgcagggtttctctaggaaaacagtgcatctgatagttactctctgcccctaggaggaaagacagattcgcccttccttcccaagtcccaggctgtgtggttcccagccccaagggtagcaagtcagaacctccggagaggcttttaagcatgcacatgtccagggtcctcatcaagagactgaatcagggggtctagggctcagcacaggcaccctttttgtttttgcagtttcacaggaattctgatgtgccagtgattgtcaggtttgtccctgggcaggacccacctgcctgaccttctgtccccctgggacacagtatttccagagaggtgcttcagttgccccaccacgacttccagcgccccccatctctgtatgcagctgagctcatgatggagcccactgtgtgctttttgttgttgttacattcctataaaaatgtccacgcatatttgaacatctgtgttcatagtggcattattcacaatggctacaacacgaagaaagcattccaagtacctatcgatgaataagcaaaatattacacacacaggaatattattcagccttgaaaggaaattcggacacgtgctacaacatagatgaatcttgaggacggtatgcaaagtgaaataaatcagacacagaaggacaaatactgtatgattccacttatataaagtacctagattagtcagattcatagagacaaagtagaatggtggttgctagacgctggagggaggggagaaaggggagttattaatgggtgtagagtttctgttacacaggatgcaaagtggcctgaagatggatggtcgtgatggttgcacagcaatgtgaatttaatgacactgaagtgtacacttaaaagtcattaaaatgctaaattttgtatgtgttttacaattttaaaaatggaaaaaaagtaagaccaaaagcaacacctctccagaatgtgtgttatataccaaattttgatgtatgtgagattgctgactatattttacttatcaatttgaaattatattgtttttatgttgacactccatataagccattattttgaaaaaaacattttccttattaaaagattggaaaaaaattcaca

SEQ ID NO: 34 - protein, 1561 aa, Homo sapiens
MQPGSAPPPGRMDPSAPQPRAETSGKDIWHPGERCLAPSPDNGKLCEASIKSITVDENGKSFAVVLYADFQERKIPLKQLQEVKFVKDCPRNLIFDDEDLEKPYFPNRKFPSSSVAFKLSDNGDSIPYTINRYLRDYQREGTRFLYGHYIHGGGCILGDDMGLGKTVQVISFLAAVLHKKGTREDIENNMPEFLLRSMKKEPLSSTAKKMFLIVAPLSVLYNWKDELDTWGYFRVTVLHGNRKDNELIRVKQRKCEIALTTYETLRLCLDELNSLEWSAVIVDEAHRIKNPKARVTEVMKALKCNVRIGLTGTILQNNMKELWCVMDWAVPGLLGSGTYFKKQFSDPVEHGQRHTATKRELATGRKAMQRLAKKMSGWFLRRTKTLIKDQLPKKEDRMVYCSLTDFQKAVYQTVLETEDVTLILQSSEPCTCRSGQKRRNCCYKTNSHGETVKTLYLSYLTVLQKVANHVALLQAASTSKQQETLIKRICDQVFSRFPDFVQKSKDAAFETLSDPKYSGKMKVLQQLLNHCRKNRDKVLLFSFSTKLLDVLQQYCMASGLDYRRLDGSTKSEERLKIVKEFNSTQDVNICLVSTMAGGLGLNFVGANVVVLFDPTWNPANDLQAIDRAYRIGQCRDVKVLRLISLGTVEEIMYLRQIYKQQLHCVVVGSENAKRYFEAVQGSKEHQGELFGIHNLFKFRSQGSCLTKDILEREGQVEAGIMTATTWLKEGPPAHKLEMPRQPDCQECRGTEQAAEPLAKEACDLCSDFSDEEPVGATGIKTAKNKAPDSSKASSSPGQLTLLQCGFSKLLETKCKAVEDSDGNTASDDESSDEQPTCLSTEAKDAGCEKNQDSLGTSKHQKLDNILNPKEKHIFYKSEKILEQNISSKSDEKKIKNTDKHCILQNVTESEDSDVICPTQYTTERFPDNSIRFKPPLEGSEDSETEHTVKTRNNDNSRNTDDKRNGIISKKLSPENTTLKSILKRKGTSDISDESDDIEISSKSRVRKRASSLRFKRIKETKKELHNSPKTMNKTNQVYAANEDHNSQFIDDYSSSDESLSVSHFSFSKQSHRPRTIRDRTSFSSKLPSHNKKNSTFIPRKPMKCSNEKVVNQEQSYESMDKFLDGVQEVAYIHSNQNVIGSSKAENHMSRWAAHDVFELKQFSQLPANIAVCSSKTYKEKVDADTLPHTKKGQQPSEGSISLPLYISNPVNQKKKKVYHTNQTTFIIGETPKGIRRKQFEEMASYFNSSSVNEFAKHITNATSEERQKMLRDFYASQYPEVKEFFVDSVSQFNNSSFEKGEQRTRKKSDKRESLIKPRLSDSETLSFKDSTNKISQVCSLKTYKRKSVKFQNHISYREEVFFNDAETKKSPVSSTQEIDSGKNSQASEDTVTSRSLNSESETRERRLENTMKDQQDLTRTGISRKEPLLKLENKKIENPVLENTSVISLLGDTSILDDLFKSHGNSPTQLPKKVLSGPMEKAKQRPKDFWDILNEQNDESLSKLTDLAVIETLCEKAPLAAPFKRREEPATSLWKSNEKFLWKKFSPSDTDENATNTQSTT

SEQ ID NO: 35 - DNA, 25 bp, Artificial Sequence
  Synthetic polynucleotide
ccttgatcccagatgttgtggcctg

SEQ ID NO: 36 - DNA, 25 bp, Artificial Sequence
  Synthetic polynucleotide
ctgggaaagccctcattgctacagt

SEQ ID NO: 37 - DNA, 25 bp, Artificial Sequence
  Synthetic polynucleotide
tacctcagttgtgaccttcagcaga

SEQ ID NO: 38 - DNA, 25 bp, Artificial Sequence
  Synthetic polynucleotide
gtggaggccatcagtattgactttc

SEQ ID NO: 39 - DNA, 25 bp, Artificial Sequence
  Synthetic polynucleotide
tattgactttctcttacttgctgta

SEQ ID NO: 40 - DNA, 25 bp, Artificial Sequence
  Synthetic polynucleotide
cttgctgtactatcagcctgctcgt

SEQ ID NO: 41 - DNA, 24 bp, Artificial Sequence
  Synthetic polynucleotide
tgctcgtttccacctttaagaatg

SEQ ID NO: 42 - DNA, 25 bp, Artificial Sequence
  Synthetic polynucleotide
ctcaatgtctcctactatccaaaat

SEQ ID NO: 43 - DNA, 25 bp, Artificial Sequence
  Synthetic polynucleotide
atgtgcatcacaggaggctcttaac

SEQ ID NO: 44 - DNA, 25 bp, Artificial Sequence
  Synthetic polynucleotide
ttgcgctaatgcttgaactcttttt

SEQ ID NO: 45 - DNA, 25 bp, Artificial Sequence
  Synthetic polynucleotide
gtatgaccaaatcctgcctcattaa

SEQ ID NO: 46 - DNA, 25 bp, Artificial Sequence
  Synthetic polynucleotide
gctagaaaccacctgattctgccag

SEQ ID NO: 47 - DNA, 25 bp, Artificial Sequence
  Synthetic polynucleotide
tgaaagcgggcacctgcaggaagct

SEQ ID NO: 48 - DNA, 25 bp, Artificial Sequence
  Synthetic polynucleotide
gaacacgatgaccttctggtggaga

SEQ ID NO: 49 - DNA, 25 bp, Artificial Sequence
  Synthetic polynucleotide
tgagaaacttcatcgctttccaggc

SEQ ID NO: 50 - DNA, 25 bp, Artificial Sequence
  Synthetic polynucleotide
tccaggcccacactgatggccaggc

SEQ ID NO: 51 - DNA, 25 bp, Artificial Sequence
  Synthetic polynucleotide
caggccagcaccagggagatactgc

SEQ ID NO: 52 - DNA, 25 bp, Artificial Sequence
  Synthetic polynucleotide
aagttatctgcatcacagtcttgtg

SEQ ID NO: 53 - DNA, 25 bp, Artificial Sequence
  Synthetic polynucleotide
cagtcttgtgtcttccgagaactat

SEQ ID NO: 54 - DNA, 25 bp, Artificial Sequence
  Synthetic polynucleotide
atctgtgcactttccatagaacttc

SEQ ID NO: 55 - DNA, 25 bp, Artificial Sequence
  Synthetic polynucleotide
aacaacattgcttcctaaactttca

SEQ ID NO: 56 - DNA, 25 bp, Artificial Sequence
  Synthetic polynucleotide
ggaagttggctgcacttgatgtttg

SEQ ID NO: 57 - DNA, 25 bp, Artificial Sequence
  Synthetic polynucleotide
gagactgttgctcaaccatcaggaa

SEQ ID NO: 58 - DNA, 25 bp, Artificial Sequence
  Synthetic polynucleotide
gagactgttgctcaaccatcaggaa

SEQ ID NO: 59 - DNA, 25 bp, Artificial Sequence
  Synthetic polynucleotide
gcagaaagtcgcatagggtttttta

SEQ ID NO: 60 - DNA, 25 bp, Artificial Sequence
  Synthetic polynucleotide
gacaatggcgctgcatgtttttctt

SEQ ID NO: 61 - DNA, 25 bp, Artificial Sequence
  Synthetic polynucleotide
tatctccttttctctagtatttgac

SEQ ID NO: 62 - DNA, 25 bp, Artificial Sequence
  Synthetic polynucleotide
tttgactgttactgtccttggcgaa

SEQ ID NO: 63 - DNA, 25 bp, Artificial Sequence
  Synthetic polynucleotide
gttactgtccttggcgaatcgataa

SEQ ID NO: 64 - DNA, 25 bp, Artificial Sequence
  Synthetic polynucleotide
ggcgaatcgataatcattgcatagt

SEQ ID NO: 65 - DNA, 25 bp, Artificial Sequence
  Synthetic polynucleotide
tagtgactgaaaagcctaagtgcaa

SEQ ID NO: 66 - DNA, 25 bp, Artificial Sequence
  Synthetic polynucleotide
ttcttgtttctgaacttcgtgccat

SEQ ID NO: 67 - DNA, 25 bp, Artificial Sequence
  Synthetic polynucleotide
acttcgtgccatattttgttcctga

SEQ ID NO: 68 - DNA, 25 bp, Artificial Sequence
  Synthetic polynucleotide
tctattagagacttaccctcctgac

SEQ ID NO: 69 - DNA, 25 bp, Artificial Sequence
  Synthetic polynucleotide
cttaccctcctgacctgataaaaag

SEQ ID NO: 70 - DNA, 25 bp, Artificial Sequence
  Synthetic polynucleotide
aaagggatacccatgtctctattaa

SEQ ID NO: 71 - DNA, 25 bp, Artificial Sequence
  Synthetic polynucleotide
tacccatgtctctattaacagcttt

SEQ ID NO: 72 - DNA, 25 bp, Artificial Sequence
  Synthetic polynucleotide
ttagttatgcttaaggaggagttct

SEQ ID NO: 73 - DNA, 25 bp, Artificial Sequence
  Synthetic polynucleotide
taatgtaagacagttttggccttta

SEQ ID NO: 74 - DNA, 25 bp, Artificial Sequence
  Synthetic polynucleotide
attatcatgagagatccttctgaat

SEQ ID NO: 75 - DNA, 25 bp, Artificial Sequence
  Synthetic polynucleotide
ccttctgaataggatgtctttctga

SEQ ID NO: 76 - DNA, 25 bp, Artificial Sequence
  Synthetic polynucleotide
tctttctgagttccactattcagtt

SEQ ID NO: 77 - DNA, 25 bp, Artificial Sequence
  Synthetic polynucleotide
cagttacaaaactccttaatgctta

SEQ ID NO: 78 - DNA, 25 bp, Artificial Sequence
  Synthetic polynucleotide
tactgtgtaccttttatatttaata

SEQ ID NO: 79 - DNA, 25 bp, Artificial Sequence
  Synthetic polynucleotide
aagtctgtactgataaaacccattg

SEQ ID NO: 80 - DNA, 25 bp, Artificial Sequence
  Synthetic polynucleotide
actgataaaacccattgtgtacaaa

SEQ ID NO: 81 - DNA, 25 bp, Artificial Sequence
  Synthetic polynucleotide
ttctctttatacaagctgagtcata

SEQ ID NO: 82 - DNA, 25 bp, Artificial Sequence
  Synthetic polynucleotide
gattttatattctggatttgtgttt

SEQ ID NO: 83 - DNA, 25 bp, Artificial Sequence
  Synthetic polynucleotide
agactttggtgatcactttgcaaat

SEQ ID NO: 84 - DNA, 25 bp, Artificial Sequence
  Synthetic polynucleotide
tggtgatcactttgcaaatatttgt

SEQ ID NO: 85 - DNA, 25 bp, Artificial Sequence
  Synthetic polynucleotide
atatttgttaatccttgagtttgag

SEQ ID NO: 86 - DNA, 25 bp, Artificial Sequence
  Synthetic polynucleotide
tgagtttgagaacctgtcttttaaa

SEQ ID NO: 87 - DNA, 25 bp, Artificial Sequence
  Synthetic polynucleotide
atactttcaaacaagctagcaaggc

SEQ ID NO: 88 - DNA, 25 bp, Artificial Sequence
  Synthetic polynucleotide
ttatatatttggttagttctgttta

SEQ ID NO: 89 - DNA, 25 bp, Artificial Sequence
  Synthetic polynucleotide
ctgttgcccttatgagttattttat

SEQ ID NO: 90 - DNA, 25 bp, Artificial Sequence
  Synthetic polynucleotide
attaccgactgtatgcctacacgga

SEQ ID NO: 91 - DNA, 25 bp, Artificial Sequence
  Synthetic polynucleotide
tacacggagtcggagctgcagattg

SEQ ID NO: 92 - DNA, 25 bp, Artificial Sequence
  Synthetic polynucleotide
ttccccaacatggtggtggcgcagg

SEQ ID NO: 93 - DNA, 25 bp, Artificial Sequence
  Synthetic polynucleotide
gcagcaggcaatcgccagtggcatc

SEQ ID NO: 94 - DNA, 25 bp, Artificial Sequence
  Synthetic polynucleotide
cagcccagcagataatccatttcct

SEQ ID NO: 95 - DNA, 25 bp, Artificial Sequence
  Synthetic polynucleotide
cagactccggttcactgagggtgtc

SEQ ID NO: 96 - DNA, 25 bp, Artificial Sequence
  Synthetic polynucleotide
gagggtgtcctgtataaccagttcc

SEQ ID NO: 97 - DNA, 25 bp, Artificial Sequence
  Synthetic polynucleotide
aaccagttcctgtcgcaagtggact

SEQ ID NO: 98 - DNA, 25 bp, Artificial Sequence
  Synthetic polynucleotide
ttcgagaactcggccaagcggctca

SEQ ID NO: 99 - DNA, 25 bp, Artificial Sequence
  Synthetic polynucleotide
ggcacagcgacgtcaagcgcttttg

SEQ ID NO: 100 - DNA, 25 bp, Artificial Sequence
  Synthetic polynucleotide
gctcctgagagcgcgggacttggac

SEQ ID NO: 101 - DNA, 25 bp, Artificial Sequence
  Synthetic polynucleotide
gagcattcttcaggtcatctgaacc

SEQ ID NO: 102 - DNA, 25 bp, Artificial Sequence
  Synthetic polynucleotide
gagaaaacatggtcaacgtcttgaa

SEQ ID NO: 103 - DNA, 25 bp, Artificial Sequence
  Synthetic polynucleotide
gtgcttatagaatgtgatcctgcca

SEQ ID NO: 104 - DNA, 25 bp, Artificial Sequence
  Synthetic polynucleotide
cagtttctgctgtacttggatgagt

SEQ ID NO: 105 - DNA, 25 bp, Artificial Sequence
  Synthetic polynucleotide
ttggatgagtccaatgccctgggga

SEQ ID NO: 106 - DNA, 25 bp, Artificial Sequence
  Synthetic polynucleotide
gatgacactcacgtctttgtaatag

SEQ ID NO: 107 - DNA, 25 bp, Artificial Sequence
  Synthetic polynucleotide
gcagaattggttaatgtcctccagg

SEQ ID NO: 108 - DNA, 25 bp, Artificial Sequence
  Synthetic polynucleotide
tgtcctccaggagcgagtgggtgaa

SEQ ID NO: 109 - DNA, 25 bp, Artificial Sequence
  Synthetic polynucleotide
aactgtgaaagacttgccactcaat

SEQ ID NO: 110 - DNA, 25 bp, Artificial Sequence
  Synthetic polynucleotide
gccactcaatatcttaggtgactga

SEQ ID NO: 111 - DNA, 25 bp, Artificial Sequence
  Synthetic polynucleotide
gggttgttttaggagcatgccacgg

SEQ ID NO: 112 - DNA, 25 bp, Artificial Sequence
  Synthetic polynucleotide
agtccggacagacattgtgggggtc

SEQ ID NO: 113 - DNA, 25 bp, Artificial Sequence
  Synthetic polynucleotide
attaaggtttactctgctgccttgg

SEQ ID NO: 114 - DNA, 25 bp, Artificial Sequence
  Synthetic polynucleotide
gccttggcagacttacgatctcaac

SEQ ID NO: 115 - DNA, 25 bp, Artificial Sequence
  Synthetic polynucleotide
cgatctcaacagttcatacgagcag

SEQ ID NO: 116 - DNA, 25 bp, Artificial Sequence
  Synthetic polynucleotide
gagggcatgctcactagtggttagt

SEQ ID NO: 117 - DNA, 25 bp, Artificial Sequence
  Synthetic polynucleotide
gtggttagtaagctgtcgactttgt

SEQ ID NO: 118 - DNA, 25 bp, Artificial Sequence
  Synthetic polynucleotide
gaacatgtacaatttgccactggga

SEQ ID NO: 119 - DNA, 25 bp, Artificial Sequence
  Synthetic polynucleotide
aatgccagctgcgtgtctagttttg

SEQ ID NO: 120 - DNA, 25 bp, Artificial Sequence
  Synthetic polynucleotide
agcaaatcactcttatttttcatcc

SEQ ID NO: 121 - DNA, 25 bp, Artificial Sequence
  Synthetic polynucleotide
gtgggagcagtgtacaccaactctt

SEQ ID NO: 122 - DNA, 25 bp, Artificial Sequence
  Synthetic polynucleotide
aactcttcctgtatattgccttttt

SEQ ID NO: 123 - DNA, 25 bp, Artificial Sequence
  Synthetic polynucleotide
taacagtaactgactggcccactga

SEQ ID NO: 124 - DNA, 25 bp, Artificial Sequence
  Synthetic polynucleotide
ccacctgggagagaaccacccgagg

SEQ ID NO: 125 - DNA, 25 bp, Artificial Sequence
  Synthetic polynucleotide
gtacccggctctgacgggtggtcat

SEQ ID NO: 126 - DNA, 25 bp, Artificial Sequence
  Synthetic polynucleotide
ttgctgctggacttttcgaagggaa

SEQ ID NO: 127 - DNA, 25 bp, Artificial Sequence
  Synthetic polynucleotide
gagcttgctgatgggcgagttggtc

SEQ ID NO: 128 - DNA, 25 bp, Artificial Sequence
  Synthetic polynucleotide
ggtccatcgcctttagggtatgtcc

SEQ ID NO: 129 - DNA, 25 bp, Artificial Sequence
  Synthetic polynucleotide
ctttagggtatgtccacctctgttc

SEQ ID NO: 130 - DNA, 25 bp, Artificial Sequence
  Synthetic polynucleotide
ctctgttcacttcctccaaggaaaa

SEQ ID NO: 131 - DNA, 25 bp, Artificial Sequence
  Synthetic polynucleotide
caccctcaggcagccagagattcat

SEQ ID NO: 132 - DNA, 25 bp, Artificial Sequence
  Synthetic polynucleotide
aacttcccctcggagggtggagcat

SEQ ID NO: 133 - DNA, 25 bp, Artificial Sequence
  Synthetic polynucleotide
gattattctgtatcctgtgtttgta

SEQ ID NO: 134 - DNA, 25 bp, Artificial Sequence
  Synthetic polynucleotide
ggtgatcacgaaactcgctggcatg

SEQ ID NO: 135 - DNA, 25 bp, Artificial Sequence
  Synthetic polynucleotide
ggaggaagacttggcgttttcgaca

SEQ ID NO: 136 - DNA, 25 bp, Artificial Sequence
  Synthetic polynucleotide
ggctggggaatttggctccagatcc

SEQ ID NO: 137 - DNA, 25 bp, Artificial Sequence
  Synthetic polynucleotide
gcgctttggcaccatgagttctatg

SEQ ID NO: 138 - DNA, 25 bp, Artificial Sequence
  Synthetic polynucleotide
ttctatgtctggggccgacgacact

SEQ ID NO: 139 - DNA, 25 bp, Artificial Sequence
  Synthetic polynucleotide
taccactcatcgcggagcaaggcgc

SEQ ID NO: 140 - DNA, 25 bp, Artificial Sequence
  Synthetic polynucleotide
acccgctcttcaagcgctttaggaa

SEQ ID NO: 141 - DNA, 25 bp, Artificial Sequence
  Synthetic polynucleotide
gcagggtacttcgttcaagaccggc

SEQ ID NO: 142 - DNA, 25 bp, Artificial Sequence
  Synthetic polynucleotide
cctccagcgttggccaaattgtgct

SEQ ID NO: 143 - DNA, 25 bp, Artificial Sequence
  Synthetic polynucleotide
ggctgtgccttcataggtcatctag

SEQ ID NO: 144 - DNA, 25 bp, Artificial Sequence
  Synthetic polynucleotide
ggggagtggggtcatttctgtatat

SEQ ID NO: 145 - DNA, 25 bp, Artificial Sequence
  Synthetic polynucleotide
gaaaccagtgtcgccctggagaagt

SEQ ID NO: 146 - DNA, 25 bp, Artificial Sequence
  Synthetic polynucleotide
aggaggcctgcgagaatggccgcgg

SEQ ID NO: 147 - DNA, 25 bp, Artificial Sequence
  Synthetic polynucleotide
tgctgtcagtggcccggggcaaagt

SEQ ID NO: 148 - DNA, 25 bp, Artificial Sequence
  Synthetic polynucleotide
gagggaatcgactttgtgcaccact

SEQ ID NO: 149 - DNA, 25 bp, Artificial Sequence
  Synthetic polynucleotide
tctacacacagagccgcattctcaa

SEQ ID NO: 150 - DNA, 25 bp, Artificial Sequence
  Synthetic polynucleotide
gcattctcaaggcgcggctggaata

SEQ ID NO: 151 - DNA, 25 bp, Artificial Sequence
  Synthetic polynucleotide
gggaccagttccagattcgtgagaa

SEQ ID NO: 152 - DNA, 25 bp, Artificial Sequence
  Synthetic polynucleotide
agaatgactttcttaccttcgatgc

SEQ ID NO: 153 - DNA, 25 bp, Artificial Sequence
  Synthetic polynucleotide
gtcgggccatcaggggcaagacgga

SEQ ID NO: 154 - DNA, 25 bp, Artificial Sequence
  Synthetic polynucleotide
ggtctttgccgacaagcggtttgcc

SEQ ID NO: 155 - DNA, 25 bp, Artificial Sequence
  Synthetic polynucleotide
tcagcagctctgagtggggcgggtg

SEQ ID NO: 156 - DNA, 25 bp, Artificial Sequence
  Synthetic polynucleotide
ttagttccaaactcactcttcttac

SEQ ID NO: 157 - DNA, 25 bp, Artificial Sequence
  Synthetic polynucleotide
cgacagcactggccattacagcaga

SEQ ID NO: 158 - DNA, 25 bp, Artificial Sequence
  Synthetic polynucleotide
ttacagcagattccgaaacccttcc

SEQ ID NO: 159 - DNA, 25 bp, Artificial Sequence
  Synthetic polynucleotide
gagaagtataatcctggtccccaag

SEQ ID NO: 160 - DNA, 25 bp, Artificial Sequence
  Synthetic polynucleotide
ggtgaatgccaaaaactgccgctcc

SEQ ID NO: 161 - DNA, 25 bp, Artificial Sequence
  Synthetic polynucleotide
gctccttgatgcaccacgttaagaa

SEQ ID NO: 162 - DNA, 25 bp, Artificial Sequence
  Synthetic polynucleotide
tagcagccctgtcacaagacgagct

SEQ ID NO: 163 - DNA, 25 bp, Artificial Sequence
  Synthetic polynucleotide
tatgatttcattcacacctcttttg

SEQ ID NO: 164 - DNA, 25 bp, Artificial Sequence
  Synthetic polynucleotide
tgatggctgttttcttatcccatgc

SEQ ID NO: 165 - DNA, 25 bp, Artificial Sequence
  Synthetic polynucleotide
tcccatgcctgtacttttcagcggc

SEQ ID NO: 166 - DNA, 25 bp, Artificial Sequence
  Synthetic polynucleotide
gctccttgccagacatcataggtca

SEQ ID NO: 167 - DNA, 25 bp, Artificial Sequence
  Synthetic polynucleotide
gaagcagcagccagcgaaatagaag

SEQ ID NO: 168 - DNA, 25 bp, Artificial Sequence
  Synthetic polynucleotide
aagaggctttcagattctaaacgaa

SEQ ID NO: 169 - DNA, 25 bp, Artificial Sequence
  Synthetic polynucleotide
atacatgcggtggatttttggggga

SEQ ID NO: 170 - DNA, 25 bp, Artificial Sequence
  Synthetic polynucleotide
tcatctgatggatcttcaagtgaac

SEQ ID NO: 171 - DNA, 25 bp, Artificial Sequence
  Synthetic polynucleotide
gccaaaaaccagtgcttcagattcg

SEQ ID NO: 172 - DNA, 25 bp, Artificial Sequence
  Synthetic polynucleotide
gcttcagattcgcagaactcagtga

SEQ ID NO: 173 - DNA, 25 bp, Artificial Sequence
  Synthetic polynucleotide
gaatggaggtgcgaccaccagcagc

SEQ ID NO: 174 - DNA, 25 bp, Artificial Sequence
  Synthetic polynucleotide
accagcagctctagtgatagtgatg

SEQ ID NO: 175 - DNA, 25 bp, Artificial Sequence
  Synthetic polynucleotide
agagaagatggtcctcgtgaccgcc

SEQ ID NO: 176 - DNA, 25 bp, Artificial Sequence
  Synthetic polynucleotide
gtgaccgccagatctgtgtttggga

SEQ ID NO: 177 - DNA, 25 bp, Artificial Sequence
  Synthetic polynucleotide
gaaggaaactaagacgtgcgagggg

SEQ ID NO: 178 - DNA, 25 bp, Artificial Sequence
  Synthetic polynucleotide
taagacttgtactatgtgtggccat

SEQ ID NO: 179 - DNA, 25 bp, Artificial Sequence
  Synthetic polynucleotide
gtgtggccatgaactgacatatgaa

SEQ ID NO: 180 - DNA, 25 bp, Artificial Sequence
  Synthetic polynucleotide
tcagtgaaggtcacctggcctggtt

SEQ ID NO: 181 - DNA, 25 bp, Artificial Sequence
  Synthetic polynucleotide
gttgtgtgcacaatgtcatgtctgt

SEQ ID NO: 182 - DNA, 25 bp, Artificial Sequence
  Synthetic polynucleotide
atgtctgtgattgccttcttacaac

SEQ ID NO: 183 - DNA, 25 bp, Artificial Sequence
  Synthetic polynucleotide
aggtgcagaagtggtaggtcagcta

SEQ ID NO: 184 - DNA, 25 bp, Artificial Sequence
  Synthetic polynucleotide
ggacaagataccaaggcaaacccta

SEQ ID NO: 185 - DNA, 25 bp, Artificial Sequence
  Synthetic polynucleotide
ggctgaactggattcttaaccaaga

SEQ ID NO: 186 - DNA, 25 bp, Artificial Sequence
  Synthetic polynucleotide
gcaatggtggtgcaccactgtaccc

SEQ ID NO: 187 - DNA, 25 bp, Artificial Sequence
  Synthetic polynucleotide
actgtaccccaggttctagtcatgt

SEQ ID NO: 188 - DNA, 25 bp, Artificial Sequence
  Synthetic polynucleotide
ttaggacgatttctgtctccacgat

SEQ ID NO: 189 - DNA, 25 bp, Artificial Sequence
  Synthetic polynucleotide
cccttccaaagactgtctccgttga

SEQ ID NO: 190 - DNA, 25 bp, Artificial Sequence
  Synthetic polynucleotide
tccaaagactgtctccgttgacctt

SEQ ID NO: 191 - DNA, 25 bp, Artificial Sequence
  Synthetic polynucleotide
tgaccttgtctttttggtatgcctt

SEQ ID NO: 192 - DNA, 25 bp, Artificial Sequence
  Synthetic polynucleotide
ccttgtctttttggtatgccttggg

SEQ ID NO: 193 - DNA, 25 bp, Artificial Sequence
  Synthetic polynucleotide
ttttggtatgccttggggtttctga

SEQ ID NO: 194 - DNA, 25 bp, Artificial Sequence
  Synthetic polynucleotide
ggtatgccttggggtttctgataat

SEQ ID NO: 195 - DNA, 25 bp, Artificial Sequence
  Synthetic polynucleotide
gccttggggtttctgataatgtgtg

SEQ ID NO: 196 - DNA, 25 bp, Artificial Sequence
  Synthetic polynucleotide
aggtaagtgagcatgtcaaacaaaa

SEQ ID NO: 197 - DNA, 25 bp, Artificial Sequence
  Synthetic polynucleotide
gtcaaacaaaataggagctcacatg

SEQ ID NO: 198 - DNA, 25 bp, Artificial Sequence
  Synthetic polynucleotide
aggagctcacatggatatatttatg

SEQ ID NO: 199 - DNA, 25 bp, Artificial Sequence
  Synthetic polynucleotide
atggatatatttatgtcactgagtt

SEQ ID NO: 200 - DNA, 25 bp, Artificial Sequence
  Synthetic polynucleotide
gagcctttgtctggtgaacagttgg

SEQ ID NO: 201 - DNA, 25 bp, Artificial Sequence
  Synthetic polynucleotide
tctccccaggataaggcggcagagg

SEQ ID NO: 202 - DNA, 25 bp, Artificial Sequence
  Synthetic polynucleotide
ggcggcagaggctacaaatgactat

SEQ ID NO: 203 - DNA, 25 bp, Artificial Sequence
  Synthetic polynucleotide
aatccaggaggccctaaactgctta

SEQ ID NO: 204 - DNA, 25 bp, Artificial Sequence
  Synthetic polynucleotide
gcagatcctgaagttatgctcttga

SEQ ID NO: 205 - DNA, 25 bp, Artificial Sequence
  Synthetic polynucleotide
gttatgctcttgactttaagtttgt

SEQ ID NO: 206 - DNA, 25 bp, Artificial Sequence
  Synthetic polynucleotide
ggaatttttgttcccataattggat

SEQ ID NO: 207 - DNA, 25 bp, Artificial Sequence
  Synthetic polynucleotide
tcaaaaagcaacttctgccctgcaa

SEQ ID NO: 208 - DNA, 25 bp, Artificial Sequence
  Synthetic polynucleotide
ccccactccatagtctggtattctg

SEQ ID NO: 209 - DNA, 25 bp, Artificial Sequence
  Synthetic polynucleotide
gtctggtattctgagcactagctta

SEQ ID NO: 210 - DNA, 25 bp, Artificial Sequence
  Synthetic polynucleotide
gagcactagcttaatatttcttcac

SEQ ID NO: 211 - DNA, 25 bp, Artificial Sequence
  Synthetic polynucleotide
tatttagaagcctttactcagcccc

SEQ ID NO: 212 - DNA, 25 bp, Artificial Sequence
  Synthetic polynucleotide
ggagcttgagctctacaggtaaggc

SEQ ID NO: 213 - DNA, 25 bp, Artificial Sequence
  Synthetic polynucleotide
taaggcagagctaccggtgaatgaa

SEQ ID NO: 214 - DNA, 25 bp, Artificial Sequence
  Synthetic polynucleotide
cccctggcatcacatgtgcatgctg

SEQ ID NO: 215 - DNA, 25 bp, Artificial Sequence
  Synthetic polynucleotide
gcatgctgtaggcaggacctgagct

SEQ ID NO: 216 - DNA, 25 bp, Artificial Sequence
  Synthetic polynucleotide
tccgctgcaggttcagatgcaccgc

SEQ ID NO: 217 - DNA, 25 bp, Artificial Sequence
  Synthetic polynucleotide
tgcagctgtccttcagttagttcac

SEQ ID NO: 218 - DNA, 25 bp, Artificial Sequence
  Synthetic polynucleotide
agcctgagccgggaactggctgtgc

SEQ ID NO: 219 - DNA, 25 bp, Artificial Sequence
  Synthetic polynucleotide
agggcttccgtgtactcaggatgta

SEQ ID NO: 220 - DNA, 25 bp, Artificial Sequence
  Synthetic polynucleotide
gtcttctcaagggactgatcggcca

SEQ ID NO: 221 - DNA, 25 bp, Artificial Sequence
  Synthetic polynucleotide
gatcggccaagtatgcttttcttta

SEQ ID NO: 222 - DNA, 4518 bp, Homo sapiens
ggagtttattcataacgcgctctccaagtatacgtggcaatgcgttgctgggttattttaatcattctaggcatcgttttcctccttatgcctctatcattcctccctatctacactaacatcccacgctctgaacgcgcgcccattaatacccttctttcctccactctccctgggactcttgatcaaagcgcggccctttccccagccttagcgaggcgccctgcagcctggtacgcgcgtggcgtggcggtgggcgcgcagtgcgttctcggtgtggagggcagctgttccgcctgcgatgatttatactcacaggacaaggatgcggtttgtcaaacagtactgctacggaggagcagcagagaaagggagagggtttgagagggagcaaaagaaaatggtaggcgcgcgtagttaattcatgcggctctcttactctgtttacatcctagagctagagtgctcggctgcccggctgagtctcctccccaccttccccaccctccccaccctccccataagcgcccctcccgggttcccaaagcagagggcgtgggggaaaagaaaaaagatcctctctcgctaatctccgcccaccggccctttataatgcgagggtctggacggctgaggacccccgagctgtgctgctcgcggccgccaccgccgggccccggccgtccctggctcccctcctgcctcgagaagggcagggcttctcagaggcttggcgggaaaaagaacggagggagggatcgcgctgagtataaaagccggttttcggggctttatctaactcgctgtagtaattccagcgagaggcagagggagcgagcgggcggccggctagggtggaagagccgggcgagcagagctgcgctgcgggcgtcctgggaagggagatccggagcgaatagggggcttcgcctctggcccagccctcccgctgatcccccagccagcggtccgcaacccttgccgcatccacgaaactttgcccatagcagcgggcgggcactttgcactggaacttacaacacccgagcaaggacgcgactctcccgacgcggggaggctattctgcccatttggggacacttccccgccgctgccaggacccgcttctctgaaaggctctccttgcagctgcttagacgctggatttttttcgggtagtggaaaaccagcagcctcccgcgacgatgcccctcaacgttagcttcaccaacaggaactatgacctcgactacgactcggtgcagccgtatttctactgcgacgaggaggagaacttctaccagcagcagcagcagagcgagctgcagcccccggcgcccagcgaggatatctggaagaaattcgagctgctgcccaccccgcccctgtcccctagccgccgctccgggctctgctcgccctcctacgttgcggtcacacccttctcccttcggggagacaacgacggcggtggcgggagcttctccacggccgaccagctggagatggtgaccgagctgctgggaggagacatggtgaaccagagtttcatctgcgacccggacgacgagaccttcatcaaaaacatcatcatccaggactgtatgtggagcggcttctcggccgccgccaagctcgtctcagagaagctggcctcctaccaggctgcgcgcaaagacagcggcagcccgaaccccgcccgcggccacagcgtctgctccacctccagcttgtacctgcaggatctgagcgccgccgcctcagagtgcatcgacccctcggtggtcttcccctaccctctcaacgacagcagctcgcccaagtcctgcgcctcgcaagactccagcgccttctctccgtcctcggattctctgctctcctcgacggagtcctccccgcagggcagccccgagcccctggtgctccatgaggagacaccgcccaccaccagcagcgactctgaggaggaacaagaagatgaggaagaaatcgatgttgtttctgtggaaaagaggcaggctcctggcaaaaggtcagagtctggatcaccttctgctggaggccacagcaaacctcctcacagcccactggtcctcaagaggtgccacgtctccacacatcagcacaactacgcagcgcctccctccactcggaaggactatcctgctgccaagagggtcaagttggacagtgtcagagtcctgagacagatcagcaacaaccgaaaatgcaccagccccaggtcctcggacaccgaggagaatgtcaagaggcgaacacacaacgtcttggagcgccagaggaggaacgagctaaaacggagcttttttgccctgcgtgaccagatcccggagttggaaaacaatgaaaaggcccccaaggtagttatccttaaaaaagccacagcatacatcctgtccgtccaagcagaggagcaaaagctcatttctgaagaggacttgttgcggaaacgacgagaacagttgaaacacaaacttgaacagctacggaactcttgtgcgtaaggaaaagtaaggaaaacgattccttctaacagaaatgtcctgagcaatcacctatgaacttgtttcaaatgcatgatcaaatgcaacctcacaaccttggctgagtcttgagactgaaagatttagccataatgtaaactgcctcaaattggactttgggcataaaagaacttttttatgcttaccatcttttttttttctttaacagatttgtatttaagaattgtttttaaaaaattttaagatttacacaatgtttctctgtaaatattgccattaaatgtaaataactttaataaaacgtttatagcagttacacagaatttcaatcctagtatatagtacctagtattataggtactataaaccctaattttttttatttaagtacattttgctttttaaagttgatttttttctattgtttttagaaaaaataaaataactggcaaatatatcattgagccaaatcttaagttgtgaatgttttgtttcgtttcttccccctcccaaccaccaccatccctgtttgttttcatcaattgccccttcagagggtggtcttaagaaaggcaagagttttcctctgttgaaatgggtctgggggccttaaggtctttaagttcttggaggttctaagatgcttcctggagactatgataacagccagagttgacagttagaaggaatggcagaaggcaggtgagaaggtgagaggtaggcaaaggagatacaagaggtcaaaggtagcagttaagtacacaaagaggcataaggactggggagttgggaggaaggtgaggaagaaactcctgttactttagttaaccagtgccagtcccctgctcactccaaacccaggaattctgcccagttgatggggacacggtgggaaccagcttctgctgccttcacaaccaggcgccagtcctgtccatgggttatctcgcaaaccccagaggatctctgggaggaatgctactattaaccctatttcacaaacaaggaaatagaagagctcaaagaggttatgtaacttatctgtagccacgcagataatacaaagcagcaatctggacccattctgttcaaaacacttaacccttcgctatcatgccttggttcatctgggtctaatgtgctgagatcaagaaggtttaggacctaatggacagactcaagtcataacaatgctaagctctatttgtgtcccaagcactcctaagcattttatccctaactctacatcaaccccatgaaggagatactgttgatttccccatattagaagtagagagggaagctgaggcacacaaagactcatccacatgcccaagattcactgatagggaaaagtggaagcgagatttgaacccaggctgtttactcctaacctgtccaagccacctctcagacgacggtaggaatcagctggctgcttgtgagtacaggagttacagtccagtgggttatgttttttaagtctcaacatctaagcctggtcaggcatcagttcccctttttttgtgatttattttgtttttattttgttgttcattgtttaatttttccttttacaatgagaaggtcaccatcttgactcctaccttagccatttgttgaatcagactcatgacggctcctgggaagaagccagttcagatcataaaataaaacatatttattctttgtcatgggagtcattattttagaaactacaaactctccttgcttccatccttttttacatactcatgacacatgctcatcctgagtccttgaaaaggtatttttgaacatgtgtattaattataagcctctgaaaacctatggcccaaaccagaaatgatgttgattatataggtaaatgaaggatgctattgctgttctaattacctcattgtctcagtctcaaagtaggtcttcagctccctgtactttgggattttaatctaccaccacccataaatcaataaataattactttctttga

SEQ ID NO: 223 - protein, 454 aa, Homo sapiens
MDFFRVVENQQPPATMPLNVSFTNRNYDLDYDSVQPYFYCDEEENFYQQQQQSELQPPAPSEDIWKKFELLPTPPLSPSRRSGLCSPSYVAVTPFSLRGDNDGGGGSFSTADQLEMVTELLGGDMVNQSFICDPDDETFIKNIIIQDCMWSGFSAAAKLVSEKLASYQAARKDSGSPNPARGHSVCSTSSLYLQDLSAAASECIDPSVVFPYPLNDSSSPKSCASQDSSAFSPSSDSLLSSTESSPQGSPEPLVLHEETPPTTSSDSEEEQEDEEEIDVVSVEKRQAPGKRSESGSPSAGGHSKPPHSPLVLKRCHVSTHQHNYAAPPSTRKDYPAAKRVKLDSVRVLRQISNNRKCTSPRSSDTEENVKRRTHNVLERQRRNELKRSFFALRDQIPELENNEKAPKVVILKKATAYILSVQAEEQKLISEEDLLRKRREQLKHKLEQLRNSCA

SEQ ID NO: 224 - DNA, 25 bp, Artificial Sequence
  Synthetic polynucleotide
gcaacaaccgaaaatgcaccagccc

SEQ ID NO: 225 - DNA, 25 bp, Artificial Sequence
  Synthetic polynucleotide
ccccaggtcctcggacaccgaggag

SEQ ID NO: 226 - DNA, 25 bp, Artificial Sequence
  Synthetic polynucleotide
cgaacacacaacgtcttggagcgcc

SEQ ID NO: 227 - DNA, 25 bp, Artificial Sequence
  Synthetic polynucleotide
ggagcgccagaggaggaacgagcta

SEQ ID NO: 228 - DNA, 25 bp, Artificial Sequence
  Synthetic polynucleotide
gctaaaacggagcttttttgccctg

SEQ ID NO: 229 - DNA, 25 bp, Artificial Sequence
  Synthetic polynucleotide
aaaagccacagcatacatcctgtcc

SEQ ID NO: 230 - DNA, 25 bp, Artificial Sequence
  Synthetic polynucleotide
catcctgtccgtccaagcagaggag

SEQ ID NO: 231 - DNA, 25 bp, Artificial Sequence
  Synthetic polynucleotide
catcctgtccgtccaagcagaggag

SEQ ID NO: 232 - DNA, 25 bp, Artificial Sequence
  Synthetic polynucleotide
gaggacttgttgcggaaacgacgag

SEQ ID NO: 233 - DNA, 25 bp, Artificial Sequence
  Synthetic polynucleotide
gaacagctacggaactcttgtgcgt

SEQ ID NO: 234 - DNA, 25 bp, Artificial Sequence
  Synthetic polynucleotide
gaaatgtcctgagcaatcacctatg

SEQ ID NO: 235 - DNA, 25 bp, Artificial Sequence
  Synthetic polynucleotide
gcaacctcacaaccttggctgagtc

SEQ ID NO: 236 - DNA, 1291 bp, Homo sapiens
gagccgaaggtggaggtcaaaggggcgtggcgttacagagcctctagcgctgggtgttggggacctgacgctatggagctctcggagttttgtgggggacggctgtgagtggggggttcctgctgcgggatgagaacgtagacgccagtggctcactcgctcctggcaccttccctttcaggctccagatggaccctgggaaggacaaagagggggtgccccagccctcagggccgccagcaaggaagaaatttgtgatacccctcgacgaggatgaggtccctcctggagtggccaagcccttattccgatctacacagagccttcccactgtggacacctcggcccaggcggcccctcagacctacgccgaatatgccatctcacagcctctggaaggggctggggccacgtgccccacagggtcagagcccctggcaggagagacgcccaaccaggccctgaaacccggggcaaaatccaacagcatcattgtgagccctcggcagaggggcaatcccgtactgaagttcgtgcgcaatgtgccctgggaatttggcgacgtaattcccgactatgtgctgggccagagcacctgtgccctgttcctcagcctccgctaccacaacctgcacccagactacatccatgggcggctgcagagcctggggaagaacttcgccttgcgggtcctgcttgtccaggtggatgtgaaagatccccagcaggccctcaaggagctggctaagatgtgtatcctggccgactgcacattgatcctcgcctggagccccgaggaagctgggcggtacctggagacctacaaggcctatgagcagaaaccagcggacctcctgatggagaagctagagcaggacttcgtctcccgggtgactgaatgtctgaccaccgtgaagtcagtcaacaaaacggacagtcagaccctcctgaccacatttggatctctggaacagctcatcgccgcatcaagagaagatctggccttatgcccaggcctgggccctcagaaagtaagagctctgggaaagaacccaaggagttgggggaaggagagagccccaaataaacacaacctgagaccccaaagttttaaggtgaaaaaagaaccaaagaccagacacagtggcttccgcctgtaatcccaacattttgggaggccaaggcgggaggactgcttgaggccagaagttggagaccagcctgggcaagtggacacctcatttttactaaaaataaaaaaaactagctgggcaaaaaaaaaaaaaaaaaa

SEQ ID NO: 237 - protein, 323 aa, Homo sapiens
MDPGKDKEGVPQPSGPPARKKFVIPLDEDEVPPGVAKPLFRSTQSLPTVDTSAQAAPQTYAEYAISQPLEGAGATCPTGSEPLAGETPNQALKPGAKSNSIIVSPRQRGNPVLKFVRNVPWEFGDVIPDYVLGQSTCALFLSLRYHNLHPDYIHGRLQSLGKNFALRVLLVQVDVKDPQQALKELAKMCILADCTLILAWSPEEAGRYLETYKAYEQKPADLLMEKLEQDFVSRVTECLTTVKSVNKTDSQTLLTTFGSLEQLIAASREDLALCPGLGPQKVRALGKNPRSWGKERAPNKHNLRPQSFKVKKEPKTRHSGFRL

SEQ ID NO: 238 - DNA, 25 bp, Artificial Sequence
  Synthetic polynucleotide
aagatctggccttatgcccaggcct

SEQ ID NO: 239 - DNA, 25 bp, Artificial Sequence
  Synthetic polynucleotide
ccctcagaaagcccggaggctgttt

SEQ ID NO: 240 - DNA, 25 bp, Artificial Sequence
  Synthetic polynucleotide
ctcagaaagcccggaggctgtttga

SEQ ID NO: 241 - DNA, 25 bp, Artificial Sequence
  Synthetic polynucleotide
gaaagcccggaggctgtttgatgtc

SEQ ID NO: 242 - DNA, 25 bp, Artificial Sequence
  Synthetic polynucleotide
aagcccggaggctgtttgatgtcct

SEQ ID NO: 243 - DNA, 25 bp, Artificial Sequence
  Synthetic polynucleotide
ggctgtttgatgtcctgcacgagcc

SEQ ID NO: 244 - DNA, 25 bp, Artificial Sequence
  Synthetic polynucleotide
tgcacgagcccttcttgaaagtacc

SEQ ID NO: 245 - DNA, 25 bp, Artificial Sequence
  Synthetic polynucleotide
gcccttcttgaaagtaccctgatga

SEQ ID NO: 246 - DNA, 25 bp, Artificial Sequence
  Synthetic polynucleotide
ccttcttgaaagtaccctgatgacc

SEQ ID NO: 247 - DNA, 25 bp, Artificial Sequence
  Synthetic polynucleotide
ttcttgaaagtaccctgatgacccc

SEQ ID NO: 248 - DNA, 25 bp, Artificial Sequence
  Synthetic polynucleotide
tcttgaaagtaccctgatgacccca

SEQ ID NO: 249 - DNA, 1220 bp, Homo sapiens
atgcacacatacgcgcgcgcacatgcacataggcacacagagatacgcgcacacacacacacaaacgcactcagatttcccggaccctggttttcctcctgtgaccctttcggggccgggctctcaccctaaagaagcagccccgccctggggtggccccaccctctcttgggacctgtcataagtcggaccccgggcgcccggctgcgcagtcccagccgccttccccaggcagtggaaccttcgggctcctgagcttcaggatggttcgtactaagacatggaccctgaagaagcactttgttggctatcctactaatagtgactttgagttgaagacagctgagctcccacccttaaaaaatggagaggtcctgcttgaagctttgttcctcaccgtggatccctacatgagagtggcagccaaaagattgaaggaaggtgatacaatgatggggcagcaagtggccaaagttgtggaaagtaaaaatgtagccctaccaaaaggaactattgtactggcttctccaggctggacaacgcactccatttctgatgggaaagatctggaaaagctgctgacagagtggccagacacaataccactgtctttggctctggggacagttggcatgccaggcctgactgcctactttggcctacttgaaatctgtggtgtgaagggtggagaaacagtgatggttaatgcagcagctggagctgtgggctcagtcgtggggcagattgcaaagctcaagggctgcaaagttgttggagcagtagggtctgatgaaaaggttgcctaccttcaaaagcttggatttgatgtcgtctttaactacaagacggtagagtctttggaagaaaccttgaagaaagcgtctcctgatggttatgattgttattttgataatgtaggtggagagttttcaaacactgttatcggccagatgaagaaatttggaaggattgccatatgtggagccatctctacatataacagaaccggcccacttcccccaggcccacccccagagattgttatctatcaggagcttcgcatggaagcttttgtcgtctaccgctggcaaggagatgcccgccaaaaagctctgaaggacttgctgaaatgggtcttagagatcaaaagagaaaatgaagaagattgaagcttcaaagcagaaaaatgaagggaatatgtatcattcaccattacctta

SEQ ID NO: 250 - protein, 301 aa, Homo sapiens
MVRTKTWTLKKHFVGYPTNSDFELKTAELPPLKNGEVLLEALFLTVDPYMRVAAKRLKEGDTMMGQQVAKVVESKNVALPKGTIVLASPGWTTHSISDGKDLEKLLTEWPDTIPLSLALGTVGMPGLTAYFGLLEICGVKGGETVMVNAAAGAVGSVVGQIAKLKGCKVVGAVGSDEKVAYLQKLGFDVVFNYKTVESLEETLKKASPDGYDCYFDNVGGEFSNTVIGQMKKFGRIAICGAISTYNRTGPLPPGPPPEIVIYQELRMEAFVVYRWQGDARQKALKDLLKWVLEIKRENEED

SEQ ID NO: 251 - DNA, 25 bp, Artificial Sequence
  Synthetic polynucleotide
gcttggatttgatgtcgtctttaac

SEQ ID NO: 252 - DNA, 25 bp, Artificial Sequence
  Synthetic polynucleotide
gaaagcgtctcctgatggttatgat

SEQ ID NO: 253 - DNA, 25 bp, Artificial Sequence
  Synthetic polynucleotide
ttcaaacactgttatcggccagatg

SEQ ID NO: 254 - DNA, 25 bp, Artificial Sequence
  Synthetic polynucleotide
atgtggagccatctctacatataac

SEQ ID NO: 255 - DNA, 25 bp, Artificial Sequence
  Synthetic polynucleotide
tacatataacagaaccggcccactt

SEQ ID NO: 256 - DNA, 25 bp, Artificial Sequence
  Synthetic polynucleotide
cccacccccagagattgttatctat

SEQ ID NO: 257 - DNA, 25 bp, Artificial Sequence
  Synthetic polynucleotide
gttatctatcaggagcttcgcatgg

SEQ ID NO: 258 - DNA, 25 bp, Artificial Sequence
  Synthetic polynucleotide
catggaagcttttgtcgtctaccgc

SEQ ID NO: 259 - DNA, 25 bp, Artificial Sequence
  Synthetic polynucleotide
taccgctggcaaggagatgcccgcc

SEQ ID NO: 260 - DNA, 25 bp, Artificial Sequence
  Synthetic polynucleotide
aggatttgaaaacatgccagctgca

SEQ ID NO: 261 - DNA, 25 bp, Artificial Sequence
  Synthetic polynucleotide
gaggacacatggaatctggaggcca

SEQ ID NO: 262 - DNA, 2520 bp, Homo sapiens
gcgcgcctgcgtactgcggtcagagggccgaggcctgggggcgagctggggtcgtgcagtacagcctctttccggcaaatcacgcgagatttcgttcacccgggctccacagggagtattttatacagaaatcttgtgaaaccactgcccaaccagagcaatgattgttcaaagagtggtattgaattctcgacctggaaaaaatggtaatccagtggcagagaatttccgaatggaagaagtctatttaccagataatattaatgaaggacaagtacaagttagaactctttatctttctgtggatccttacatgcgttgtagaatgaatgaagacactggcactgattatataacaccttggcagctatctcaagtcgttgatggaggaggtattggaattatagaagaaagcaaacacacaaatttgactaaaggcgattttgtgacttctttctattggccctggcaaaccaaggttattctggatggaaatagccttgaaaaggtagacccacaacttgtggatggacacctttcatattttcttggagctataggtatgcctggtttgacttccttgattgggatacaggaaaaaggtcatataactgctggatctaataagacaatggttgtcagtggggccgcaggtgcctgtggatctgtggctgggcagattggccatttcttaggttgttccagagtggtgggaatttgtggaacacatgagaaatgcatcctcttgacctcagaactgggctttgatgctgcaattaattataaaaaagacaatgtggcagaacagctccgtgaatcatgcccagctggagtggatgtttattttgacaatgttggtggtaacatcagtgatacagtgataagtcagatgaatgagaacagccacatcatcctgtgtggtcaaatttctcagtacaacaaagatgtgccttatcctcccccgctatcccctgctatagaggcaatccagaaagaaagaaacatcacaagggaaagatttctggtattaaattataaagacaaatttgagcctggcattctacagctgagtcagtggtttaaagaaggaaagctaaagattaaagagacggtaataaatgggttggaaaacatgggagctgcattccagtccatgatgacaggaggtaacattggaaagcagatagtttgcatttcagaagaaatctctttgtaattgctgtaaatgtcatcaaggcaatcatagatttcttttccattttgcatattttcaaagatatgttaaaaaatccttagactatacatagctcttgatttaaatgtgatcataggtgttatttttagttgcatagggtatttgatacaatcattaatggatcatacacaataggtttttaaaaattaataacttttagtaattacttttattaatttaaaatagaacgcttgagaggcactttgtaaagatttgttaaactggaaacgttttacatgatctgatacaaccattaatgaatcatacacaataggttttttaaaattaatattaataacttttattaatttaaaatagaatgcttaaaataaaatagaatgcttgagaggcactgagtaaagatttgttgaactggaaatgttttacatgattcttaaactgaaacttggtgtaaaaatagaattgagatggcctttttttcacattgtagactgaaaagagacttaatggtatgatgtgtacatagggactgggggcaggattgggggtttcggagcttgtgtaacagtttttgggataggagaccagcggttttgggttgggattagtatgggaagataaataacttaggttggttaagttgacaagatttactccagaggatcatctctttgtatttgccaaataatttactgtatagcctaaaaactccatatatattgagaaaagcatatgtttattttaggttagcaggcacatactgtcaagttgtaaagattgagagggcaaacagatgtaaacatcacttgtaggtgattaaaaagattgacagccgggcctgatgtctcaagcctgtaatcctagcactttgggaggcagaggcgggcagatcacttgaggtcaggagttcaagaccagcctggccaacacggtgaaaccccatctctctaaaaatacaaaaattagctgggcgtggtggcacacgcctgtaatcccagctactcaggaggctgaggctggagaatcatttgaacctgggagggggaggttgccgtgagctgagcttgcaccattgcactccagcctgggcgacaagagtgaaattccatctcaaaaaacaaaaacagattgacaacaaagacagtttcagaaaatgacaggactgggcaaattaacaaatgtttgtaaacatgaatgttcaggaactactgatgtacctcaaaagtttgttttattaattgtactcaaccctcgcagaacagtaaaactgaagattattgtttctgaaaaaaaaaaaaaaaaaa

SEQ ID NO: 263 - protein, 351 aa, Homo sapiens
MIVQRVVLNSRPGKNGNPVAENFRMEEVYLPDNINEGQVQVRTLYLSVDPYMRCRMNEDTGTDYITPWQLSQVVDGGGIGIIEESKHTNLTKGDFVTSFYWPWQTKVILDGNSLEKVDPQLVDGHLSYFLGAIGMPGLTSLIGIQEKGHITAGSNKTMVVSGAAGACGSVAGQIGHFLGCSRVVGICGTHEKCILLTSELGFDAAINYKKDNVAEQLRESCPAGVDVYFDNVGGNISDTVISQMNENSHIILCGQISQYNKDVPYPPPLSPAIEAIQKERNITRERFLVLNYKDKFEPGILQLSQWFKEGKLKIKETVINGLENMGAAFQSMMTGGNIGKQIVCISEEISL

SEQ ID NO: 264 - DNA, 25 bp, Artificial Sequence
  Synthetic polynucleotide
ggaaagcagatagtttgcatttcag

SEQ ID NO: 265 - DNA, 25 bp, Artificial Sequence
  Synthetic polynucleotide
aaaatccttagactatacatagctc

SEQ ID NO: 266 - DNA, 25 bp, Artificial Sequence
  Synthetic polynucleotide
agactatacatagctcttgatttaa

SEQ ID NO: 267 - DNA, 25 bp, Artificial Sequence
  Synthetic polynucleotide
gatcataggtgttatttttagttgc

SEQ ID NO: 268 - DNA, 25 bp, Artificial Sequence
  Synthetic polynucleotide
ttagttgcatagggtatttgataca

SEQ ID NO: 269 - DNA, 25 bp, Artificial Sequence
  Synthetic polynucleotide
gatacaatcattaatggatcataca

SEQ ID NO: 270 - DNA, 25 bp, Artificial Sequence
  Synthetic polynucleotide
ggatcatacacaataggtttttaaa

SEQ ID NO: 271 - DNA, 25 bp, Artificial Sequence
  Synthetic polynucleotide
agaacgcttgagaggcactttgtaa

SEQ ID NO: 272 - DNA, 25 bp, Artificial Sequence
  Synthetic polynucleotide
ggaaacgttttacatgatctgatac

SEQ ID NO: 273 - DNA, 25 bp, Artificial Sequence
  Synthetic polynucleotide
tgatctgatacaaccattaatgaat

SEQ ID NO: 274 - DNA, 25 bp, Artificial Sequence
  Synthetic polynucleotide
gaatcatacacaataggttttttaa

SEQ ID NO: 275 - DNA, 20 bp, Artificial Sequence
  Synthetic polynucleotide
gcagtctttcccttgaggct

SEQ ID NO: 276 - DNA, 20 bp, Artificial Sequence
  Synthetic polynucleotide
tcgggaattacgtcgccaaa

SEQ ID NO: 277 - DNA, 23 bp, Artificial Sequence
  Synthetic polynucleotide
taccccgagcagttctcctacat

SEQ ID NO: 278 - DNA, 25 bp, Artificial Sequence
  Synthetic polynucleotide
gccagttccttggacaccaggtctg

SEQ ID NO: 279 - DNA, 20 bp, Artificial Sequence
  Synthetic polynucleotide
gcatccacctggagtaccct

SEQ ID NO: 280 - DNA, 20 bp, Artificial Sequence
  Synthetic polynucleotide
tcccaggaccttttggtggt

SEQ ID NO: 281 - DNA, 25 bp, Artificial Sequence
  Synthetic polynucleotide
tgaggcagaaaataaggagagtgaa

SEQ ID NO: 282 - DNA, 25 bp, Artificial Sequence
  Synthetic polynucleotide
tggggaagtgaagtgtaagaagagt

SEQ ID NO: 283 - DNA, 21 bp, Artificial Sequence
  Synthetic polynucleotide
aggcagaaaataaggagagtg

SEQ ID NO: 284 - DNA, 21 bp, Artificial Sequence
  Synthetic polynucleotide
aagcggatggatgatagtgag

SEQ ID NO: 285 - DNA, 27 bp, Artificial Sequence
  Synthetic polynucleotide
gcgaggtagagtcaaggagagtggtct

SEQ ID NO: 286 - DNA, 26 bp, Artificial Sequence
  Synthetic polynucleotide
gcgcaaagttcgttctgctgctcaag

SEQ ID NO: 287 - DNA, 25 bp, Artificial Sequence
  Synthetic polynucleotide
gccgagatgatggagatgaagatta

SEQ ID NO: 288 - DNA, 25 bp, Artificial Sequence
  Synthetic polynucleotide
gcgcagtaggtatggatttatgtga

SEQ ID NO: 289 - DNA, 27 bp, Artificial Sequence
  Synthetic polynucleotide
gtagtcattgatgatctgcccaaagag

SEQ ID NO: 290 - DNA, 27 bp, Artificial Sequence
  Synthetic polynucleotide
gagccacacaagctattttctttctca

SEQ ID NO: 291 - DNA, 27 bp, Artificial Sequence
  Synthetic polynucleotide
gcagttcaaggatctaaagagcatcaa

SEQ ID NO: 292 - DNA, 27 bp, Artificial Sequence
  Synthetic polynucleotide
aacatctgtatgctgaggatgaacaca

SEQ ID NO: 293 - DNA, 23 bp, Artificial Sequence
  Synthetic polynucleotide
tgatgatgagactaaaacaaaat

SEQ ID NO: 294 - DNA, 23 bp, Artificial Sequence
  Synthetic polynucleotide
tgaagaagaaagaataaaataat

SEQ ID NO: 295 - DNA, 25 bp, Artificial Sequence
  Synthetic polynucleotide
ttttccagtcccattattttcacag

SEQ ID NO: 296 - DNA, 25 bp, Artificial Sequence
  Synthetic polynucleotide
agtcccttctttcctttcagtctcc

SEQ ID NO: 297 - DNA, 25 bp, Artificial Sequence
  Synthetic polynucleotide
tcaaggcaaagagaaaaagagtatt

SEQ ID NO: 298 - DNA, 25 bp, Artificial Sequence
  Synthetic polynucleotide
agacaccaaagtaagaccacagatt

SEQ ID NO: 299 - DNA, 25 bp, Artificial Sequence
  Synthetic polynucleotide
agacttggagacttcttcggagacc

SEQ ID NO: 300 - DNA, 25 bp, Artificial Sequence
  Synthetic polynucleotide
taaaacacaggcatcaatcaaaata

SEQ ID NO: 301 - DNA, 21 bp, Artificial Sequence
  Synthetic polynucleotide
gaactgggtgatgcggatgct

SEQ ID NO: 302 - DNA, 21 bp, Artificial Sequence
  Synthetic polynucleotide
gctggaagaggaaggagagaa

SEQ ID NO: 303 - DNA, 27 bp, Artificial Sequence
  Synthetic polynucleotide
acaaggtgaaaccccgtctctactaaa

SEQ ID NO: 304 - DNA, 27 bp, Artificial Sequence
  Synthetic polynucleotide
ttcttccacctaagctttgccataaat

SEQ ID NO: 305 - DNA, 27 bp, Artificial Sequence
  Synthetic polynucleotide
atcaaaaacatcatcatccaggactgt

SEQ ID NO: 306 - DNA, 27 bp, Artificial Sequence
  Synthetic polynucleotide
tctcaggactctgacactgtccaactt

SEQ ID NO: 307 - DNA, 27 bp, Artificial Sequence
  Synthetic polynucleotide
caggatggttcgtactaagacatggac

SEQ ID NO: 308 - DNA, 27 bp, Artificial Sequence
  Synthetic polynucleotide
gctttcttcaaggtttcttccaaagac

SEQ ID NO: 309 - DNA, 27 bp, Artificial Sequence
  Synthetic polynucleotide
catgcgttgtagaatgaatgaagacac

SEQ ID NO: 310 - DNA, 27 bp, Artificial Sequence
  Synthetic polynucleotide
tgtactgagaaatttgaccacacagga

SEQ ID NO: 311 - DNA, 26 bp, Artificial Sequence
  Synthetic polynucleotide
agcaggttaatggataatttcttgat

SEQ ID NO: 312 - DNA, 26 bp, Artificial Sequence
  Synthetic polynucleotide
ggtcctttgtaaaaaccattacactt

SEQ ID NO: 313 - DNA, 27 bp, Artificial Sequence
  Synthetic polynucleotide
cgtttccttttattttggagctaatgc

SEQ ID NO: 314 - DNA, 27 bp, Artificial Sequence
  Synthetic polynucleotide
aaggaagtcactccaaggtacacactg

SEQ ID NO: 315 - DNA, 27 bp, Artificial Sequence
  Synthetic polynucleotide
atgcaagaaatgtctggagaaattgaa

SEQ ID NO: 316 - DNA, 27 bp, Artificial Sequence
  Synthetic polynucleotide
ccttgtattttctcagtacgagctcca

SEQ ID NO: 317 - DNA, 25 bp, Artificial Sequence
  Synthetic polynucleotide
gcgacggcggctgcggctactggag

SEQ ID NO: 318 - DNA, 25 bp, Artificial Sequence
  Synthetic polynucleotide
ttcttctaatgcttcttgactaccc

SEQ ID NO: 319 - DNA, 25 bp, Artificial Sequence
  Synthetic polynucleotide
tgaaaggaaggagaaggagaaaaag

SEQ ID NO: 320 - DNA, 25 bp, Artificial Sequence
  Synthetic polynucleotide
agaggcagtgagggcagcattagta

SEQ ID NO: 321 - DNA, 25 bp, Artificial Sequence
  Synthetic polynucleotide
taaatggagaggaggtagaagaaac

SEQ ID NO: 322 - DNA, 25 bp, Artificial Sequence
  Synthetic polynucleotide
ggtggtagaaagagaacgaaaagtc

SEQ ID NO: 323 - DNA, 23 bp, Artificial Sequence
  Synthetic polynucleotide
gcgtgacattaaggagaagctgt

SEQ ID NO: 324 - DNA, 23 bp, Artificial Sequence
  Synthetic polynucleotide
cttgttttctgcgcaagttaggt

SEQ ID NO: 325 - DNA, 18 bp, Artificial Sequence
  Synthetic polynucleotide
aggagccaggagaggact

SEQ ID NO: 326 - DNA, 18 bp, Artificial Sequence
  Synthetic polynucleotide
gcagggacgaaaggtatc

SEQ ID NO: 327 - DNA, 23 bp, Artificial Sequence
  Synthetic polynucleotide
gtatcgtggaaggactcatgacc

SEQ ID NO: 328 - DNA, 23 bp, Artificial Sequence
  Synthetic polynucleotide
tctcttcctcttgtgctcttgct

SEQ ID NO: 329 - DNA, 120 bp, Artificial Sequence
  Synthetic polynucleotide
gcacacagaagcgctcagtaagggctttgaaacttaacagtttgggagccagatcctcaggccacatctctctcctcccacgacctccgcggtcctccagaaccatagagagttgtacag

SEQ ID NO: 330 - DNA, 120 bp, Artificial Sequence
  Synthetic polynucleotide
agatcgccctgctctatgctctactctcctggggagcggggccagagaggccggaagtgctgcgagccctgggccacgctggccgtgctggcagtgggccgcctcgatccctctgcagtc

SEQ ID NO: 331 - DNA, 120 bp, Artificial Sequence
  Synthetic polynucleotide
tttcccttgaggctccaagaccagcaggtgaggcctcgcggcgctgaaaccgtgaggcccggaccacaggtgcgggaggcggagactgcgggtggagattggcgccgcggaagccaatca

SEQ ID NO: 332 - DNA, 120 bp, Artificial Sequence
  Synthetic polynucleotide
gcgatgggacttgtggacctgtaaggggcggggcgagccgaaggtggaggtcaaaggggcgtggcgttacagagcctctagcgctgggtgttggggacctgacgctatggagctctcgga

SEQ ID NO: 333 - DNA, 120 bp, Artificial Sequence
  Synthetic polynucleotide
gttttgtgggggacggctgtgagtggggggttcctgctgcgggatgagaacgtagacgccagtggctcactcgctcctggcaccttccctttcaggctccagatggaccctgggaaggac

SEQ ID NO: 334 - DNA, 120 bp, Artificial Sequence
  Synthetic polynucleotide
aaagagggggtgccccagccctcagggccgccagcaaggaagaaatttgtgatacccctcgacgaggatgaggtccctcctggagtggtaggacaaggagatgcggggcccctgggaggc

SEQ ID NO: 335 - DNA, 120 bp, Artificial Sequence
  Synthetic polynucleotide
ttctccccacaggccaagcccttattccgatctacacagagccttcccactgtggacacctcggcccaggcggcccctcagacctacgccgaatatgccatctcacagcctctggaaggg

SEQ ID NO: 336 - DNA, 120 bp, Artificial Sequence
  Synthetic polynucleotide
gctggggccacgtgccccacagggtcagagcccctggcaggagagacgcccaaccaggccctgaaacccggggcaaaatccaacagcatcattgtgagccctcggcaggtgaggagggag

SEQ ID NO: 337 - DNA, 120 bp, Artificial Sequence
  Synthetic polynucleotide
ctccccagaggggcaatcccgtactgaagttcgtgcgcaatgtgccctgggaatttggcgacgtaattcccgactatgtgctgggccagagcacctgtgccctgttcctcaggtgagctc

SEQ ID NO: 338 - DNA, 120 bp, Artificial Sequence
  Synthetic polynucleotide
cccccaccagcctccgctaccacaacctgcacccagactacatccatgggcggctgcagagcctggggaagaacttcgccttgcgggtcctgcttgtccaggtggatgtggtaagcaggg

SEQ ID NO: 339 - DNA, 120 bp, Artificial Sequence
  Synthetic polynucleotide
aattctgattttctcctccagaaagatccccagcaggccctcaaggagctggctaagatgtgtatcctggccgactgcacattgatcctcgcctggaggtgagatgagggcttccctgcc

SEQ ID NO: 340 - DNA, 120 bp, Artificial Sequence
  Synthetic polynucleotide
gttatcccagccccgaggaagctgggcggtacctggagacctacaaggcctatgagcagaaaccagcggacctcctgatggagaagctagagcaggacttcgtctcccgggtgaggccac

SEQ ID NO: 341 - DNA, 120 bp, Artificial Sequence
  Synthetic polynucleotide
cactcctgcctccaccctttccaggtgactgaatgtctgaccaccgtgaagtcagtcaacaaaacggacagtcagaccctcctgaccacatttggagtaaggaatggctcccctgcccca

SEQ ID NO: 342 - DNA, 120 bp, Artificial Sequence
  Synthetic polynucleotide
ggaggcttttgtgctcaactgccctgacccctcgctttcacctttcagtctctggaacagctcatcgccgcatcaagagaagatctggccttatgcccaggcctgggccctcagaaagta

SEQ ID NO: 343 - DNA, 119 bp, Artificial Sequence
  Synthetic polynucleotide
agagctctgggaaagaacccaaggagttgggggaaggagagagccccaaataaacacaacctgagaccccaaagttttaaggtgaaaaaagaaccaaagaccagacacagtggcttccg

SEQ ID NO: 344 - DNA, 120 bp, Artificial Sequence
  Synthetic polynucleotide
ggcgggtcgaccccgctgcacagtccggccggcgccatgaagtgagaagggggctgggggtcgcgctcgctagcgggcgcggggggtcttgaagatggggtcatcggtgggcgcgcctgg

SEQ ID NO: 345 - DNA, 120 bp, Artificial Sequence
  Synthetic polynucleotide
gtccccaagggggcgaggggagggtgaaggggtgggacgggggcagccgcagggagcagcagtgatagcgaggagacactgagggggccccgaggctcctgaggacctgagggttaccgg

SEQ ID NO: 346 - DNA, 120 bp, Artificial Sequence
  Synthetic polynucleotide
gggcgccgggcccgtcacccttctctgggctcgacgaccgggcactgtggaggcgggagaggggctgaggggacgggaactgacccagcagcccctgccgccaggctcaacgtggacggg

SEQ ID NO: 347 - DNA, 120 bp, Artificial Sequence
  Synthetic polynucleotide
ctcctggtctacttcccgtacgactacatctaccccgagcagttctcctacatgcgggagctcaaacgcacgctggacgccaaggtgggtggccggtgggcccgacccgcccactcgacc

SEQ ID NO: 348 - DNA, 120 bp, Artificial Sequence
  Synthetic polynucleotide
cctctggtccccaacatgcagggtcatggagtcctggagatgccctcaggcaccgggaagacagtatccctgttggccctgatcatggcataccagagagtgagtgatgcgctgaacccg

SEQ ID NO: 349 - DNA, 120 bp, Artificial Sequence
  Synthetic polynucleotide
agggactgagtccgcttgttatcggcaggcatatccgctggaggtgaccaaactcatctactgctcaagaactgtgccagagattgagaaggtaagctgggactcatcctggtgctccag

SEQ ID NO: 350 - DNA, 120 bp, Artificial Sequence
  Synthetic polynucleotide
agtaggtgattgaagagcttcgaaagttgctcaacttctatgagaagcaggagggcgagaagctgccgtttctgggactggctctgagctcccgcaaaaacttgtgtattcaccctgagg

SEQ ID NO: 351 - DNA, 120 bp, Artificial Sequence
  Synthetic polynucleotide
aggtgacacccctgcgctttgggaaggacgtcgatgggaaatgccacagcctcacagcctcctatgtgcgggcgcagtaccagcatgacaccagcctgccccactgccgattctatgagg

SEQ ID NO: 352 - DNA, 120 bp, Artificial Sequence
  Synthetic polynucleotide
aggaatttgatgcccatgggcgtgaggtgcccctccccgctggcatctacaacctggatgacctgaaggccctggggcggcgccagggctggtgcccatacttccttgctcgatactcag

SEQ ID NO: 353 - DNA, 120 bp, Artificial Sequence
  Synthetic polynucleotide
ggtaggggtaggggttggggtggcagggccctggtaaccctgctccccggccccccagatcctgcatgccaatgtggtggtttatagctaccactacctcctggaccccaagattgcaga

SEQ ID NO: 354 - DNA, 120 bp, Artificial Sequence
  Synthetic polynucleotide
cctggtgtccaaggaactggcccgcaaggccgtcgtggtcttcgacgaggcccacaacattggtgaggggggcgccaggggccaaagggatgccagcccctctgagtgaggcccctgcag

SEQ ID NO: 355 - DNA, 120 bp, Artificial Sequence
  Synthetic polynucleotide
ccccttctccagacaacgtctgcatcgactccatgagcgtcaacctcacccgccggacccttgaccggtgccagggcaacctggagaccctgcagaagacggtgctcaggtggggccggg

SEQ ID NO: 356 - DNA, 120 bp, Artificial Sequence
  Synthetic polynucleotide
acttgtccccagggttgccagccccctcccagccccagctcatctctccgcaggatcaaagagacagacgagcagcgcctgcgggacgagtaccggcgtctggtggaggggctgcgggag

SEQ ID NO: 357 - DNA, 120 bp, Artificial Sequence
  Synthetic polynucleotide
gccagcgccgcccgggagacggacgcccacctggccaaccccgtgctgcccgacgaagtgctgcagggtgagccccgaccccccgctgccccccagtccctttcccgcctccccgtcgcc

SEQ ID NO: 358 - DNA, 120 bp, Artificial Sequence
  Synthetic polynucleotide
cgcctccccgtcgccgctgatagcgtctcctcgcagaggcagtgcctggctccatccgcacggccgagcatttcctgggcttcctgaggcggctgctggagtacgtgaagtggcggctgc

SEQ ID NO: 359 - DNA, 120 bp, Artificial Sequence
  Synthetic polynucleotide
gtgtgcagcatgtggtgcaggagagcccgcccgccttcctgagcggcctggcccagcgcgtgtgcatccagcgcaagcccctcaggtgcggccccagacagcgcgcggggtgggggcccg

SEQ ID NO: 360 - DNA, 120 bp, Artificial Sequence
  Synthetic polynucleotide
attctgtgctgaacgcctccggtccctgctgcatactctggagatcaccgaccttgctgacttctccccgctcaccctccttgctaactttgccacccttgtcagcacctacgccaaagg

SEQ ID NO: 361 - DNA, 120 bp, Artificial Sequence
  Synthetic polynucleotide
acccctccttgcctgccctctgcaggcttcaccatcatcatcgagccctttgacgacagaaccccgaccattgccaaccccatcctgcacttcaggtgggaccctgcccggtgagggtgt

SEQ ID NO: 362 - DNA, 120 bp, Artificial Sequence
  Synthetic polynucleotide
cctcactgccctcatctctctccagctgcatggacgcctcgctggccatcaaacccgtatttgagcgtttccagtctgtcatcatcacatctggggtaaggacccttccccgtcccctcc

SEQ ID NO: 363 - DNA, 120 bp, Artificial Sequence
  Synthetic polynucleotide
ccgccacagacactgtccccgctggacatctaccccaagatcctggacttccaccccgtcaccatggcaaccttcaccatgacgctggcacgggtctgcctctgccctatggtgagtggg

SEQ ID NO: 364 - DNA, 120 bp, Artificial Sequence
  Synthetic polynucleotide
gcttatcgtgacctctgttgctctccagatcatcggccgtggcaatgaccaggtggccatcagctccaaatttgagacccgggaggatattggtatgctgccagtggggctggtttctgt

SEQ ID NO: 365 - DNA, 120 bp, Artificial Sequence
  Synthetic polynucleotide
agacagagaagggaggaggacctgggccaggagagggcccaacctctgaccccttgcagctgtgatccggaactatgggaacctcctgctggagatgtccgctgtggtccctgatggcat

SEQ ID NO: 366 - DNA, 120 bp, Artificial Sequence
  Synthetic polynucleotide
cgtggccttcttcaccagctaccagtacatggagagcaccgtggcctcctggtatgagcaggtacgcctggccaccccctccctgcacctgctctcctcagtccctggcactgcaccgct

SEQ ID NO: 367 - DNA, 120 bp, Artificial Sequence
  Synthetic polynucleotide
gggtccttccccaggggatccttgagaacatccagaggaacaagctgctctttattgagacccaggatggtgccgaaaccagtgtcgccctggagaagtaccaggaggtgggtgtgcgag

SEQ ID NO: 368 - DNA, 120 bp, Artificial Sequence
  Synthetic polynucleotide
tgcgtctcggtctccccacctcaggcctgcgagaatggccgcggggccatcctgctgtcagtggcccggggcaaagtgtccgagggaatcgactttggtgagtggactgggctcttcctc

SEQ ID NO: 369 - DNA, 120 bp, Artificial Sequence
  Synthetic polynucleotide
cgccccctctcctctgcccaccagtgcaccactacgggcgggccgtcatcatgtttggcgtcccctacgtctacacacagagccgcattctcaaggtgagtagctctgtctcccagggag

SEQ ID NO: 370 - DNA, 120 bp, Artificial Sequence
  Synthetic polynucleotide
aggagtggctcccccacctccccagcttctcatcctccgtatctgcaggcgcggctggaatacctgcgggaccagttccagattcgtgagaatgactttcttaccttcgatgccatgcgc

SEQ ID NO: 371 - DNA, 120 bp, Artificial Sequence
  Synthetic polynucleotide
cacgcggcccagtgtgtgggtcgggccatcaggggcaagacggactacggcctcatggtctttgccgacaaggtgcagcttcaggggtgcccctgtgctcccatcccaggctccaagaac

SEQ ID NO: 372 - DNA, 120 bp, Artificial Sequence
  Synthetic polynucleotide
aggctccccgaatgaccttctgtccctggcctgcgcttctgcccacagcggtttgcccgtggggacaagcgggggaagctgccccgctggatccaggagcacctcacagatgccaacctc

SEQ ID NO: 373 - DNA, 120 bp, Artificial Sequence
  Synthetic polynucleotide
aacctgaccgtggacgagggtgtccaggtggccaagtacttcctgcggcagatggcacagcccttccaccgggtgaggcctgcgtccccctcccggcaccctcccaggctgagcttctcc

SEQ ID NO: 374 - DNA, 120 bp, Artificial Sequence
  Synthetic polynucleotide
tctgttctctgcaggaggatcagctgggcctgtccctgctcagcctggagcagctagaatcagaggagacgctgaagaggatagagcagattgctcagcagctctgagtggggcgggtgg

SEQ ID NO: 375 - DNA, 120 bp, Artificial Sequence
  Synthetic polynucleotide
gagcggggtcatcttctctctgctgctgtagctgccatgggcaaaagagaccgagcggaccgcggtgagacgttgcgcgggcacgctcagccacgactgcccttgccggccctgcccccc

SEQ ID NO: 376 - DNA, 120 bp, Artificial Sequence
  Synthetic polynucleotide
gctctgcctcggagctgctccgggcctctgcgccggccgaccctgctggccctcccgcgcgcaccccgttgggacaggcctttgggcgggagagatgctggacctgggcgcagcccagcg

SEQ ID NO: 377 - DNA, 120 bp, Artificial Sequence
  Synthetic polynucleotide
aactcggcctaggggagacgggtgaggggcgcaacgcctgcgggatgcaggtggctcttagctaggagtttgcggcggcgcaggtgaaatgctgccaagcggtgcggagggaaccctgaa

SEQ ID NO: 378 - DNA, 120 bp, Artificial Sequence
  Synthetic polynucleotide
gtgttggtatcttgcagacaagaagaaatccaggaagcggcactatgaggatgaagaggatgatgaagaggacgccccggggaacgaccctcaggaagcggttccctcggcggcggggaa

SEQ ID NO: 379 - DNA, 120 bp, Artificial Sequence
  Synthetic polynucleotide
gcaggtggatgagtcaggcaccaaagtggatgaatatggagccaaggactacaggctgcaaatgccgctgaaggacgaccacacctccaggcccctctgggtggtaagcatgcccttagc

SEQ ID NO: 380 - DNA, 120 bp, Artificial Sequence
  Synthetic polynucleotide
aggctcccgatggccatatcttcttggaagccttctctccagtttacaaatatgcccaagacttcttggtggctattgcagagccagtgtgccgaccaacccatgtgcatgagtacaaac

SEQ ID NO: 381 - DNA, 120 bp, Artificial Sequence
  Synthetic polynucleotide
taactgcctactccttgtatgcagctgtcagcgttgggctgcaaaccagtgacatcaccgagtacctcaggaagctcagcaagactggagtccctgatggaattatgcagtttattaagg

SEQ ID NO: 382 - DNA, 120 bp, Artificial Sequence
  Synthetic polynucleotide
cacatttacctgttggatgttatctgtatttgcagttgtgtactgtcagctatggaaaagtcaagctggtcttgaagcacaacaggtaagagattccatgacaggcctgtcccaaggcac

SEQ ID NO: 383 - DNA, 120 bp, Artificial Sequence
  Synthetic polynucleotide
tccaggaggtacctgctggtcagtagaccccttcttcctcccctgcttgcagatacttcgttgaaagttgccaccctgatgtaatccagcatcttctccaggaccccgtgatccgagaat

SEQ ID NO: 384 - DNA, 120 bp, Artificial Sequence
  Synthetic polynucleotide
gccgcttaagaaactctgaaggggaggccactgagctcatcacagagactttcacaagcaaatctgccgtatgtggactcctgggccacccttgggtgggggcaggcatttaggatttca

SEQ ID NO: 385 - DNA, 120 bp, Artificial Sequence
  Synthetic polynucleotide
aatgttgtgtgcacgttcagcacctacctctctcacagatttctaagactgctgaaagcagtggtgggccctccacttcccgagtgacagatccacagggtaaatctgacatccccatgg

SEQ ID NO: 386 - DNA, 120 bp, Artificial Sequence
  Synthetic polynucleotide
acctgtttgacttctatgagcaaatggacaaggatgaagaagaagaagaagagacacagacagtgtcttttgaagtcaagcaggttagtgaatgtaccttcctcctggttccttcactga

SEQ ID NO: 387 - DNA, 120 bp, Artificial Sequence
  Synthetic polynucleotide
tttgtgccctctttccaggaaatgattgaggaactccagaaacgttgcatccacctggagtaccctctgttggcagaatatgacttccggaatgattctgtcaaccctgatatcaacatt

SEQ ID NO: 388 - DNA, 120 bp, Artificial Sequence
  Synthetic polynucleotide
gacctaaagcccacagctgtcctcagaccctatcaggagaagagcttgcgaaagatgtttggaaacgggcgtgcacgttcgggggtcattgttcttccctgcggtaagtggtaccagagt

SEQ ID NO: 389 - DNA, 120 bp, Artificial Sequence
  Synthetic polynucleotide
attgcactcttgtttcttgtaggtgctggaaagtccctggttggtgtgactgctgcatgcactgtcagaaaacgctgtctggtgctgggcaactcagctgtttctgtggagcagtggaaa

SEQ ID NO: 390 - DNA, 120 bp, Artificial Sequence
  Synthetic polynucleotide
gcccagttcaagatgtggtccaccattgacgacagccagatctgccggttcacctccgatgccaaggacaagcccatcggctgctccgttgccattagcacctactccatgctgggccac

SEQ ID NO: 391 - DNA, 120 bp, Artificial Sequence
  Synthetic polynucleotide
accaccaaaaggtcctgggaggccgagcgagtcatggagtggctcaagacccaggagtggggcctcatgatcctggatgaagtgcacaccataccaggtaagcaggctggagctgagctg

SEQ ID NO: 392 - DNA, 120 bp, Artificial Sequence
  Synthetic polynucleotide
agtgtgaatgctcccattgtttcctcagccaagatgttccgaagggtgctcaccatcgtgcaggcccactgtaagctgggtttgactgcgaccctcgtccgcgaagatgacaaaattgtg

SEQ ID NO: 393 - DNA, 120 bp, Artificial Sequence
  Synthetic polynucleotide
gatttaaattttctgattgggcctaagctctacgaagccaactggatggagctgcagaataatggctacatcgccaaagtccagtgtgctgaggtagctgggcctgggctgggggcgtct

SEQ ID NO: 394 - DNA, 120 bp, Artificial Sequence
  Synthetic polynucleotide
gttcttactgtattacaggtctggtgccctatgtctcctgaattttaccgggaatatgtggcaatcaaaaccaagaaacgaatcttgctgtacaccatgaaccccaacaaatttagagct

SEQ ID NO: 395 - DNA, 120 bp, Artificial Sequence
  Synthetic polynucleotide
tgccagtttctgatcaagtttcatgaaaggaggaatgacaagattattgtctttgctgacaatgtgtttgccctaaaggaatatgccattcgactgaacaagtaagaattgaaaacttgg

SEQ ID NO: 396 - DNA, 120 bp, Artificial Sequence
  Synthetic polynucleotide
attcttctctagaccctatatctacggacctacgtctcagggggaaaggatgcaaattctccagaatttcaagcacaaccccaaaattaacaccatcttcatatccaaggtttgtgtggc

SEQ ID NO: 397 - DNA, 120 bp, Artificial Sequence
  Synthetic polynucleotide
ggtaggtgacacttcgtttgatctgccggaagcaaatgtcctcattcagatctcatcccatggtggctccaggcgtcaggaagcccaaaggctagggcgggtgcttcgagctaaaaaagg

SEQ ID NO: 398 - DNA, 120 bp, Artificial Sequence
  Synthetic polynucleotide
ggatggttgcagaagagtacaatgcctttttctactcactggtatcccaggacacacaggaaatggcttactcaaccaagcggcagagattcttggtagatcaaggttatagcttcaagg

SEQ ID NO: 399 - DNA, 120 bp, Artificial Sequence
  Synthetic polynucleotide
agagagagcagaaaggggcatgtctgctggcttgggctttgcaggtgatcacgaaactcgctggcatggaggaggaagacttggcgttttcgacaaaagaagagcaacagcagctcttac

SEQ ID NO: 400 - DNA, 120 bp, Artificial Sequence
  Synthetic polynucleotide
agaaagtcctggcagccactgacctggatgccgaggaggaggtggtggctggggaatttggctccagatccagccaggtgagtaaatgggtgaggaggttccaggtgtcagtgctctcac

SEQ ID NO: 401 - DNA, 120 bp, Artificial Sequence
  Synthetic polynucleotide
aggagtatcttttcttctggagactaacatgggctggttcccccttcccggcaggcatctcggcgctttggcaccatgagttctatgtctggggccgacgacactgtgtacatggagtac

SEQ ID NO: 402 - DNA, 120 bp, Artificial Sequence
  Synthetic polynucleotide
cactcatcgcggagcaaggcgcccagcaaacatgtacacccgctcttcaagcgctttaggaaatgatgcttaggcagggtacttcgttcaagaccggcgcttggcacccttgttggaaag

SEQ ID NO: 403 - DNA, 120 bp, Artificial Sequence
  Synthetic polynucleotide
acccggaagagcttccatggagtcagggcagccggctcgacggattgccatggcgccgctgctggagtacgagcgacagctggtgctggaactgctcgacactgacgggctagtagtgtg

SEQ ID NO: 404 - DNA, 120 bp, Artificial Sequence
  Synthetic polynucleotide
cgcccgcgggctcggcgcggaccggctcctctaccactttctccagctgcactgccacccagcctgcctggtgctggtgctcaacacgcagccggccgaggaggtgcggccgcgctggcg

SEQ ID NO: 405 - DNA, 120 bp, Artificial Sequence
  Synthetic polynucleotide
agcctactaatcaagtttgatttgatttaggagtattttatcaatcagctgaagatagaaggagttgaacacctccctcgccgtgtaacaaatgaaatcacaagcaacagtcgctatgaa

SEQ ID NO: 406 - DNA, 120 bp, Artificial Sequence
  Synthetic polynucleotide
gtttacacacaaggtggtgttatatttgcgacaagtaggatacttgtggttgacttcttgactgatagaataccttcagatttaattactggtaagaatttgaaatcttattattagtat

SEQ ID NO: 407 - DNA, 120 bp, Artificial Sequence
  Synthetic polynucleotide
aaattatgtttctccccctcaggcatcttggtgtatagagcccacagaataatcgagtcttgtcaagaagcattcatcttgcgcctctttcgccagaaaaacaaacgtggttttattaaa

SEQ ID NO: 408 - DNA, 120 bp, Artificial Sequence
  Synthetic polynucleotide
gctttcacagacaatgctgttgcctttgatactggtttttgtcatgtggaaagagtgatgagaaatctttttgtgaggaaactgtatctgtggccaaggtaaagaacattatgtgacaaa

SEQ ID NO: 409 - DNA, 120 bp, Artificial Sequence
  Synthetic polynucleotide
atatttgtctctttaggttccatgtagcagtaaactcatttttagaacagcacaaacctgaagttgtagaaatccatgtttctatgacacctaccatgcttgctatacagactgctatac

SEQ ID NO: 410 - DNA, 120 bp, Artificial Sequence
  Synthetic polynucleotide
tggacattttaaatgcatgtctaaaggaactaaaatgccataacccatcgcttgaagtggaagatttatctttagaaaatgctattggaaaaccttttgacaaggtactctttttccttt

SEQ ID NO: 411 - DNA, 120 bp, Artificial Sequence
  Synthetic polynucleotide
tagcaataccaaattttattcttgttttagacaatccgccattatctggatcctttgtggcaccagcttggagccaagactaaatccttagttcaggatttgaagatattacgaactttg

SEQ ID NO: 412 - DNA, 120 bp, Artificial Sequence
  Synthetic polynucleotide
ctgcagtatctctctcagtatgattgtgtcacatttcttaatcttctggaatctctgagagcaacggaaaaagcttttggtcagaattcaggtgggagattaaaatactaataatattct

SEQ ID NO: 413 - DNA, 120 bp, Artificial Sequence
  Synthetic polynucleotide
ctgttttaaattaaccataaattgatggcactttttcttttaacttttcgtattaggttggctgtttcttgactccagcacctcgatgtttataaatgctcgagcaagggtttatcatct

SEQ ID NO: 414 - DNA, 120 bp, Artificial Sequence
  Synthetic polynucleotide
tccagatgccaaaatgagtaaaaaagaaaaaatatctgaaaaaatggaaattaaagaaggggaaggtatcttgtggggttaagtctttaaatgtgttttttatttcggtatttggtatgg

SEQ ID NO: 415 - DNA, 120 bp, Artificial Sequence
  Synthetic polynucleotide
acagaaacaaaaaaggaactggtcctagaaagcaacccaaagtgggaggcactgactgaagtattaaaagaaattgaggcagaaaataaggagagtgaagctcttggtggtccaggtagg

SEQ ID NO: 416 - DNA, 120 bp, Artificial Sequence
  Synthetic polynucleotide
ggtcaagtactgatttgtgcaagtgatgaccgaacatgttcccagctgagagactatatcactcttggagcggaggccttcttattgaggctctacaggaaaacctttgagaaggatagc

SEQ ID NO: 417 - DNA, 120 bp, Artificial Sequence
  Synthetic polynucleotide
aaagctgaagaagtctggatgaaatttaggaaggaagacagttcaaagagaattaggaaatctcacaaaagacctaaagacccccaaaacaaagaacgggcttctaccaaagaaagaacc

SEQ ID NO: 418 - DNA, 120 bp, Artificial Sequence
  Synthetic polynucleotide
ctcaaaaagaaaaaacggaagttgaccttaactcaaatggtaggaaaacctgaagaactggaagaggaaggagatgtcgaggaaggatatcgtcgagaaataagcagtagcccagaaagc

SEQ ID NO: 419 - DNA, 120 bp, Artificial Sequence
  Synthetic polynucleotide
tgcccggaagaaattaagcatgaagaatttgatgtaaatttgtcatcggatgctgctttcggaatcctgaaagaacccctcactatcatccatccgcttctgggttgcagcgacccctat

SEQ ID NO: 420 - DNA, 120 bp, Artificial Sequence
  Synthetic polynucleotide
gctctgacaagggtactacatgaagtggagccaagatacgtggttctttatgacgcagagctaacctttgttcggcagcttgaaatttacagggcgagtaggcctgggaaacctctgagg

SEQ ID NO: 421 - DNA, 120 bp, Artificial Sequence
  Synthetic polynucleotide
gtcttaacatgcagggtttactttcttatatacggaggttcaactgaggaacaacgctatctcactgctttgcggaaagaaaaggaagcttttgaaaaactcataaggtaatacatagaa

SEQ ID NO: 422 - DNA, 120 bp, Artificial Sequence
  Synthetic polynucleotide
acagggaaaaagcaagcatggttgtccctgaagaaagagaaggcagagatgaaacaaacttagacctagtaagaggcacagcatctgcagatgtttccactgacactcggaaagccggtg

SEQ ID NO: 423 - DNA, 120 bp, Artificial Sequence
  Synthetic polynucleotide
attccttctttgagagttcttccccagtgacattacttactttttctctgtaggtggccaggaacagaatggtacacagcaaagcatagttgtggatatgcgtgaatttcgaagtgagct

SEQ ID NO: 424 - DNA, 120 bp, Artificial Sequence
  Synthetic polynucleotide
tccatctctgatccatcgtcggggcattgacattgaacccgtgactttagaggttggagattacatcctcactccagaaatgtgcgtggagcgcaagagtatcagtgatttaatcggctc

SEQ ID NO: 425 - DNA, 120 bp, Artificial Sequence
  Synthetic polynucleotide
tttaaataacggccgcctctacagccagtgcatctccatgtcccgctactacaagcgtcccgtgcttctgattgagtttgaccctagcaagcctttctctctcacttcccgaggtgcctt

SEQ ID NO: 426 - DNA, 120 bp, Artificial Sequence
  Synthetic polynucleotide
gtttcaggagatctccagcaatgacattagttccaaactcactcttcttacacttcacttccccagactacggattctctggtgcccctctcctcatgcaacggcggagttgtttgagga

SEQ ID NO: 427 - DNA, 120 bp, Artificial Sequence
  Synthetic polynucleotide
gctgaaacaaagcaagccacagcctgatgcggcgacagcactggccattacagcagattctgaaacccttcccgagtcagagaagtataatcctggtccccaagacttcttgttaaaaat

SEQ ID NO: 428 - DNA, 120 bp, Artificial Sequence
  Synthetic polynucleotide
gccaggggtgaatgccaaaaactgccgctccttgatgcaccacgttaagaacatcgcagaattagcagccctgtcacaagacgagctcacgagtattctggggaatgctgcaaatgccaa

SEQ ID NO: 429 - DNA, 120 bp, Artificial Sequence
  Synthetic polynucleotide
acagctttatgatttcattcacacctcttttgcagaagtcgtatcaaaaggaaaagggaaaaagtgaacagtgatggctgttttcttatcccatgcctgtacttttcagcggctccttgc

SEQ ID NO: 430 - DNA, 120 bp, Artificial Sequence
  Synthetic polynucleotide
aggacgcagccgcctcatgggggtccaggggctctggaagctgctggagtgctccgggcggcaggtcagccccgaagcgctggaagggaagatcctggctgttggtatccttaacgccgc

SEQ ID NO: 431 - DNA, 120 bp, Artificial Sequence
  Synthetic polynucleotide
cccggagttttttccattaacaattctcccagatattagcatttggttaaaccaagcacttaaaggagtccgggatcgccatgggaactcaatagaaaatcctcatcttctcactttgtt

SEQ ID NO: 432 - DNA, 120 bp, Artificial Sequence
  Synthetic polynucleotide
tcatcggctctgcaaactcttattttttcgaattcgtcctatttttgtgtttgatggggatgctccactattgaagaaacagactttggtaagtgtcgtatagtttttagtaagtgtcaa

SEQ ID NO: 433 - DNA, 120 bp, Artificial Sequence
  Synthetic polynucleotide
aggtgaagagaaggcagagaaaggacttagcgtccagtgactccaggaaaacgacagagaagcttctgaaaacatttttgaaaagacaagccatcaaaactgccttcagaagcaaaaggc

SEQ ID NO: 434 - DNA, 120 bp, Artificial Sequence
  Synthetic polynucleotide
tttgtgtactttccagagatgaagcactacccagtcttacccaagttcgaagagaaaacgacctctatgttttgcctcctttacaagaggaagaaaaacacaggtaaatgtttaactatt

SEQ ID NO: 435 - DNA, 120 bp, Artificial Sequence
  Synthetic polynucleotide
agatatcgtaaaagtatgtttgactttcagttcagaagaggaagatgaaaaagaatggcaagaaagaatgaatcaaaaacaagcattacaggtatttagatcatttttgaattcagaatg

SEQ ID NO: 436 - DNA, 120 bp, Artificial Sequence
  Synthetic polynucleotide
aagtgtatgaaatgtaaatttcatggtgctgtgattttatctttacaggaagagttctttcataatcctcaagcgatagatattgagtctgaggacttcagcagcctgccccctgaagta

SEQ ID NO: 437 - DNA, 120 bp, Artificial Sequence
  Synthetic polynucleotide
aagcatgaaatcttgactgatatgaaagagttcaccaagcgcagaagaacattatttgaagcaatgccagaggtgaaatatgcaacagtacattcatgcttagaattaagaacttcagca

SEQ ID NO: 438 - DNA, 120 bp, Artificial Sequence
  Synthetic polynucleotide
tttattttgcctttaggagtctgatgacttttcacagtaccaactcaaaggcttgcttaaaaagaactatctgaaccagcatatagaacatgtccaaaaggaaatgaatcagcaacattc

SEQ ID NO: 439 - DNA, 120 bp, Artificial Sequence
  Synthetic polynucleotide
aggacacatccgaaggcagtatgaagatgaagggggctttctgaaggaggtagagtcaaggagagtggtctctgaagacacttcacattacatcttgataaaaggtatcaggcaccatca

SEQ ID NO: 440 - DNA, 120 bp, Artificial Sequence
  Synthetic polynucleotide
aaggtattcaagctaagacagttgcagaagtggattcagagtctcttccttcttccagcaaaatgcacggcatgtcttttgacgtgaagtcatctccatgtgaaaaactgaagacagaga

SEQ ID NO: 441-450 - skipped (10 entries)

SEQ ID NO: 451 - DNA, 120 bp, Artificial Sequence
  Synthetic polynucleotide
aagagcctgatgctacccctccttctccaagaactttactagctatgcaagctgccctgctgggaagtagctcagaagaggagctggagagtgaaaatcgaaggcaggcccgtgggagga

SEQ ID NO: 452 - DNA, 120 bp, Artificial Sequence
  Synthetic polynucleotide
acgcacctgctgctgtagacgaaggctccatatcaccccggactctttcagccattaagagagctcttgacgatgacgaagatgtaaaagtgtgtgctggggatgatgtgcagacgggag

SEQ ID NO: 453 - DNA, 120 bp, Artificial Sequence
  Synthetic polynucleotide
ggccaggagcagaagaaatgcgtataaacagctccaccgagaacagtgatgaaggacttaaagtgagagatggaaaaggaataccgtttactgcaacacttgcgtcatctagtgtgaact

SEQ ID NO: 454 - DNA, 120 bp, Artificial Sequence
  Synthetic polynucleotide
ctgcagaggagcacgtagccagcactaatgaggggagagagcccacagactcagttccaaaagaacaaatgtcacttgttcacgtggggactgaagcctttccgataagtgatgagtcta

SEQ ID NO: 455 - DNA, 120 bp, Artificial Sequence
  Synthetic polynucleotide
tgattaaggacagaaaagatcggctgcctctggagagtgcagtggttagacatagtgacgcacctgggctcccgaatggaagggaactgacaccggcatctccaacttgtacaaattctg

SEQ ID NO: 456 - DNA, 120 bp, Artificial Sequence
  Synthetic polynucleotide
tgtcaaagaatgaaacacatgctgaagtgcttgagcagcagaacgaactttgcccatatgagagtaaattcgattcttctcttctttcaagtgatgatgaaacaaaatgtaaaccgaatt

SEQ ID NO: 457 - DNA, 120 bp, Artificial Sequence
  Synthetic polynucleotide
ctgcttctgaagtcattggccctgtcagtttgcaagaaacaagtagcatagtaagtgtcccttcagaggcagtagataatgtggaaaatgtggtgtcatttaatgctaaagagcatgaga

SEQ ID NO: 458 - DNA, 120 bp, Artificial Sequence
  Synthetic polynucleotide
attttctggaaaccatccaagaacagcagaccactgaatctgcaggccaggatttaatttccattccaaaggccgtggaaccaatggaaattgactcggaagaaagtgaatctgatggta

SEQ ID NO: 459 - DNA, 120 bp, Artificial Sequence
  Synthetic polynucleotide
tgcaggatcattttaatgttttgattgtagatgaagtgaccttttaattttggtacaggaagtttcattgaagtgcaaagtgtgattagtgatgaggaacttcaagcagaattccctgaa

SEQ ID NO: 460 - DNA, 120 bp, Artificial Sequence
  Synthetic polynucleotide
acttccaaacctccctcagaacaaggcgaagaggaactggtaggaactagggagggagaagcccctgctgagtccgagagcctcctgagggacaactctgagagggacgacgtggatggt

SEQ ID NO: 461 - DNA, 120 bp, Artificial Sequence
  Synthetic polynucleotide
gagccacaggaagctgagaaagatgcggaagattcgctccatgaatggcaagatattaatttggtaataccgtaacattgtgtttcgacttcttgctgaggaagccaggttaagtaggtt

SEQ ID NO: 462 - DNA, 120 bp, Artificial Sequence
  Synthetic polynucleotide
tgtaaacaaaactcatttggattattaatataaatctataaatgaaaaaacattttataggaggagttggaaactctggagagcaacctcttagcacagcagaattcactgaaagctcaa

SEQ ID NO: 463 - DNA, 120 bp, Artificial Sequence
  Synthetic polynucleotide
aaacagcagcaagaacggatcgctgctactgtcaccggacagatgttcctggaaagccaggtgggtgcaggcagcttgggtttcctttaccaccttcttcagacccctgggggaatgcac

SEQ ID NO: 464 - DNA, 120 bp, Artificial Sequence
  Synthetic polynucleotide
cctcactctgcaggaactcctgcgcctgttcggcattccctacatccaggctcccatggaagcagaggcgcagtgcgccatcctggacctgactgatcagacttccggaaccatcactga

SEQ ID NO: 465 - DNA, 120 bp, Artificial Sequence
  Synthetic polynucleotide
tgacagtgatatctggctgtttggagcgcggcatgtctatagaaacttttttaataaaaacaagtttgtagaatattatcaatatgtggactttcacaatcaattgggtaagacttcaga

SEQ ID NO: 466 - DNA, 120 bp, Artificial Sequence
  Synthetic polynucleotide
tcatataagaaatcttgataaaaattaaaaaatattgttactctttaggattggaccggaataagttaataaatttggcttatttgcttggaagtgattataccgaaggaataccaactg

SEQ ID NO: 467 - DNA, 120 bp, Artificial Sequence
  Synthetic polynucleotide
tgggttgtgtaaccgccatggaaattctcaatgaattccctgggcatggcctggaacctctcctaaaattctcgtaaggtcttttatttctttaatttggataattgtgtaaatacccaa

SEQ ID NO: 468 - DNA, 120 bp, Artificial Sequence
  Synthetic polynucleotide
ttgtttcctttattttacagagaatggtggcatgaagctcaaaaaaatccaaagataagacctaatcctcatgacaccaaagtgaaaaaaaaattacggacattgcaactcacccctggc

SEQ ID NO: 469 - DNA, 120 bp, Artificial Sequence
  Synthetic polynucleotide
tttcctaacccagctgttgccgaggcctacctcaaacccgtggtggatgactcgaagggatcctttctgtgggggaaacctgatctcgacaaaattagagaatatcctttgcttcttaaa

SEQ ID NO: 470 - DNA, 120 bp, Artificial Sequence
  Synthetic polynucleotide
agtcttaactgcatgcatattttgtcagcggtatttcggctggaacagaacgaagacagatgaatctctgtttcctgtattaaagcaactcgatgcccagcaggtaatcatggtggaccc

SEQ ID NO: 471 - DNA, 120 bp, Artificial Sequence
  Synthetic polynucleotide
agacacagctccgaattgattccttctttagattagcacaacaggagaaagaagatgctaaacgtattaagagccagagactaaacagagctgtgacatgtatgctaaggaaagagaaag

SEQ ID NO: 472 - DNA, 120 bp, Artificial Sequence
  Synthetic polynucleotide
aagcagcagccagcgaaatagaagcagtttctgttgccatggagaaagaatttgagctacttgataaggcaaaaggaaaaacccagaagagaggcataacaaataccttagaagagtcat

SEQ ID NO: 473 - DNA, 120 bp, Artificial Sequence
  Synthetic polynucleotide
caagcctgaaaagaaagaggctttcagattctaaaggaaagaatacatgcggtggatttttgggggagacctgcctctcagaatcatctgatggatcttcaagtgaagatgctgaaagtt

SEQ ID NO: 474 - DNA, 120 bp, Artificial Sequence
  Synthetic polynucleotide
catctttaatgaatgtacaaaggagaacagctgcgaaagagccaaaaaccagtgcttcagattcgcagaactcagtgaaggaagctcccgtgaagaatggaggtgcgaccaccagcagct

SEQ ID NO: 475 - DNA, 120 bp, Artificial Sequence
  Synthetic polynucleotide
ctagtgatagtgatgacgatggagggaaagagaagatggtcctcgtgaccgccagatctgtgtttgggaagaaaagaaggaaactaagacgtgcgaggggaagaaaaaggaaaacctaat

SEQ ID NO: 476 - DNA, 120 bp, Artificial Sequence
  Synthetic polynucleotide
tttttttccttttaggtagtctgtagagaatgccaaatgagggaatcccccactcaagtcaaactcaggagcaagactgtttacagagtcaacctgtcagtaataatgaagaaatggcaa

SEQ ID NO: 477 - DNA, 120 bp, Artificial Sequence
  Synthetic polynucleotide
tcaagcaagaaagtggtggtgatggggaggtggaggagtacctctcctttcgttctgtgggtgacgggctgtccacctctgctgtggggtgcgcatcagcagctccgaggagagggccag

SEQ ID NO: 478 - DNA, 120 bp, Artificial Sequence
  Synthetic polynucleotide
ccctgctgcacatcgaccgacatcagatccaggcagtagagcctagcgcccaggcccttgagctgcagggtttgggtgtggacgtctatgaccaggacgtgctggaacagggagtgcttc

SEQ ID NO: 479 - DNA, 120 bp, Artificial Sequence
  Synthetic polynucleotide
agcaggtggacaatgccatccatgaggccagccgtgcctcccagctcgttgacgtggagaaggagtatcggtcggtcctggatgacctcacgtgagtgcagcccatcttcttcctttcaa

SEQ ID NO: 480 - DNA, 120 bp, Artificial Sequence
  Synthetic polynucleotide
tatattatgctataaaaatgttatcagagtgcaaaatagacaatttatcttatttttcaggtcatgtacgacatccctaaggcaaatcaataaaattattgaacagcttagccctcaagc

SEQ ID NO: 481 - DNA, 120 bp, Artificial Sequence
  Synthetic polynucleotide
tgccaccagcagagacatcaacaggaaactagattctgtaaaacgacagaagtataataaggtgattcagaataacattcagtattgcatttttgaaaaagtcatcatttaggggcactt

SEQ ID NO: 482 - DNA, 120 bp, Artificial Sequence
  Synthetic polynucleotide
ttcaaggaacaacagctaaaaaagatcactgcaaaacaaaagcatctccaggccatccttggaggagcagaggtgaaaattgaactagatcacgccagtctggaggaggatgcaggtgag

SEQ ID NO: 483 - DNA, 120 bp, Artificial Sequence
  Synthetic polynucleotide
ggtggagggggcagaggcggacctgtctggagatggtactgactatgagctgaagcctctgcccaagggcgggaaacggcagaagaaagtgccagtgcaggagattgatgatgacttttt

SEQ ID NO: 484 - DNA, 120 bp, Artificial Sequence
  Synthetic polynucleotide
cccaagttctggggaagaagctgaagctgcttctgtaggagaaggaggaggaggaggtcggaaagtgggaagataccgagatgatggagatgaagattattataagcagcggttaaggtc

SEQ ID NO: 485 - DNA, 120 bp, Artificial Sequence
  Synthetic polynucleotide
atttgtagctgcctaatatttcttgaaagagtgagcatttcttttgtaccctcggaaagtttcatgctagtgcgaaacgcattgctattgttctttcagagccggggccatccagtcttg

SEQ ID NO: 486 - DNA, 120 bp, Artificial Sequence
  Synthetic polynucleotide
gcagcatgctcatgcctgtccaggagactgcctgggaagagctcatccgcactggccagatgacaccttttggtacccagatccctcagaaacaggagaaaaagcccagaaaaatcatgc

SEQ ID NO: 487 - DNA, 120 bp, Artificial Sequence
  Synthetic polynucleotide
ttaatgaagcatcaggcttcgaaaagtatttggcagatcaagcaaaactgtcttttgaaaggaagaagcaaggttgtaataaaagagcagctagaaaagctccagccccagtcacgcctc

SEQ ID NO: 488 - DNA, 120 bp, Artificial Sequence
  Synthetic polynucleotide
cagccccagtgcaaaataaaaacaaaccaaacaagaaagccagagttctgtccaaaaaagaggagcgtttgaaaaagcacatcaagaaactccagaagagggctttgcagttccagggga

SEQ ID NO: 489 - DNA, 119 bp, Artificial Sequence
  Synthetic polynucleotide
aagtgggattgccaaaggcaaggagaccttgggagtcagacatgaggccagaggcagagggagactctgagggtgaagagtctgagtatttccccacagaggaggaggaagaggaggaa

SEQ ID NO: 490 - DNA, 120 bp, Artificial Sequence
  Synthetic polynucleotide
tggaacactaggcaaaaccactaccactaggactaataataccttttttccgttttagtcccaagatgcctcgaacactaagtttacatgaaataactgaccttttagagacagatgaca

SEQ ID NO: 491 - DNA, 120 bp, Artificial Sequence
  Synthetic polynucleotide
ttacagaggcacaccctggacaataccattttgtattcaataactttttcaccagtattgcacttcttgataagctcagttcaatgggacatcaggcaacaggtacagtgagaaaggatc

SEQ ID NO: 492 - DNA, 120 bp, Artificial Sequence
  Synthetic polynucleotide
acattgacagagttccactggaatcagatgtagctttaaagaaaaaagaaagaggcacatttgattatcgaattgatggcaaaggcaatattgtctgcagatggaatgataacagtgttg

SEQ ID NO: 493 - DNA, 120 bp, Artificial Sequence
  Synthetic polynucleotide
tcactgttgcctcatctggtgctggtatccatcccctgtgtcttgtcagtcgttactcccagaaactgaaaaagaagatacaagttcagcagccaaacatgatcaaagtgtataaccagt

SEQ ID NO: 494 - DNA, 120 bp, Artificial Sequence
  Synthetic polynucleotide
tcatgggaggcgtagacagagctgatgaaaacattgataagtatcgggcatcaatccgtggaaagaaatggtattcaagccctcttttgttctgtttcgaactggtcttacaaaatgctt

SEQ ID NO: 495 - DNA, 120 bp, Artificial Sequence
  Synthetic polynucleotide
ggcaattgcataaaacatatgatgagaaaccagtggattttctggagtttcgtcgacgtgtggtatgccattatctggagacccatggtcatcctccagaacctggccaaaaaggaagac

SEQ ID NO: 496 - DNA, 120 bp, Artificial Sequence
  Synthetic polynucleotide
ctcagaagcgtaacattgactcacgttatgatggcataaatcatgtgatagtcaaacagggaaagcaaacgcgatgcgctgaatgtcataagaacacaacttttcgatgtgaaaaatgtg

SEQ ID NO: 497 - DNA, 120 bp, Artificial Sequence
  Synthetic polynucleotide
atgttgccttacatgtgaagtgttccgttgaatatcacactgaatagcaggtgtcaccacctcctgagataagaaacatagttttatacattatgtacagtgtagcagtggttttgccta

SEQ ID NO: 498 - DNA, 120 bp, Artificial Sequence
  Synthetic polynucleotide
gtgttccaattttggaacgtcacataacaatggaacataataaatttttttttctcttcaaatttttgttccttgaatttttctaggtaacatatatgaatttcatgcaaaaattcaaaa

SEQ ID NO: 499 - DNA, 120 bp, Artificial Sequence
  Synthetic polynucleotide
gcatagaagcaagtgctatagtgatacaaccacctgaaaatgctacagcacctgtttctgatgaggaatcaggagatgaagaaggtggaacaataaataatctgccaggttctttgttgc

SEQ ID NO: 500 - DNA, 120 bp, Artificial Sequence
  Synthetic polynucleotide
acacagctgcgtatcttattcaagatggctctgatgctgagtctgactcagatgatccctcatacgcacctaaagatgactctcctgatgaagttccatctacgtttactgtgcagcaac

SEQ ID NO: 501 - DNA, 120 bp, Artificial Sequence
  Synthetic polynucleotide
ctccaccatcaaggaggaggaaaatgacaaaaattctttgcaaatggaaaaaagccgacctaactgtacaacccgtagcaggtagagttacagcaccaccaaacgatttcttcaccgtaa

SEQ ID NO: 502 - DNA, 120 bp, Artificial Sequence
  Synthetic polynucleotide
tgagaactcccacagaaattcttgaactttttcttgatgacgaggtcattgaactcattgtcaagtactccaacttatatgcttgcagtaaaggtgtacatcttggcttgactagctctg

SEQ ID NO: 503 - DNA, 120 bp, Artificial Sequence
  Synthetic polynucleotide
aattcaaatgttttctgggaattatttttctgagtggttatgtctcagttcctagaaggcgtatgttttgggaacaaagaacagatgtgcataatgtactggttagtgctgccatgagac

SEQ ID NO: 504 - DNA, 120 bp, Artificial Sequence
  Synthetic polynucleotide
gtgaccggtttgaaactatattttctaatttgcatgttgctgacaatgcaaatttggatccagtggacaaattttccaaattgcgacctctcataagcaaacttaatgagagatgcatga

SEQ ID NO: 505 - DNA, 120 bp, Artificial Sequence
  Synthetic polynucleotide
aatttgttccaaatgaaacatatttcagctttgatgaattcatggttccttattttggtcgtcacgggtgcaaacaatttattcggggaaagcccattcggtttggctataagttttggt

SEQ ID NO: 506 - DNA, 120 bp, Artificial Sequence
  Synthetic polynucleotide
gtggtgccacctgtctgggctacatttgctggtttcagccgtatcagggtaaaaacccaaatactaaacatgaggaatatggtgtcggtgcgtcacttgtccttcagtttagtgaggcac

SEQ ID NO: 507 - DNA, 120 bp, Artificial Sequence
  Synthetic polynucleotide
tttaaatctgtcttgtgatcaaaataatggaaatgtgatttttattttcatggtaggagatggaataaactgagactgcaggacaaagagaaacgtctgaagctggaggacgattctgag

SEQ ID NO: 508 - DNA, 120 bp, Artificial Sequence
  Synthetic polynucleotide
gaaagtgatgctgaatttgacgaaggttttaaagtgccaggttttctgttcaaaaagctttttaagtatgtaccatatgttctttcctttctatttgctatcaagccattatgtacaaat

SEQ ID NO: 509 - DNA, 120 bp, Artificial Sequence
  Synthetic polynucleotide
ttgccattttctcttttcttgttggtgtttgttgtcataggtaccagcagacaggtgttaggtggctgtgggaattgcactgccagcaggcaggaggaattctgggagatgaaatgggat

SEQ ID NO: 510 - DNA, 120 bp, Artificial Sequence
  Synthetic polynucleotide
tgggcaagaccatccagataattgccttcttggcaggtctgagctacagcaagatcaggactcgtggttcaaattacaggcaagtgctcctctgcagactgtcagtctgtggagctcaat

SEQ ID NO: 511 - DNA, 120 bp, Artificial Sequence
  Synthetic polynucleotide
tgactgtatatgctctttcatggttgttttcttcttggacgtttggatgcaggtttgaggggttgggtccaactgtaattgtctgtccaacaacagtgatgcatcagtgggtgaaggaat

SEQ ID NO: 512 - DNA, 120 bp, Artificial Sequence
  Synthetic polynucleotide
ttcacacgtggtggcctccgttcagagtggcaattctacatgaaaccggttcctatacccacaaaaaggtaacacaatatttcagtacctttttgttttgttttaatgccctccatttta

SEQ ID NO: 513 - DNA, 120 bp, Artificial Sequence
  Synthetic polynucleotide
taaaactgactttaccattttattgtggtctcaggagaaactaattcgagatgttgctcattgtcatggaattttgatcacatcttactcctacattcgattgatgcaggatgacattag

SEQ ID NO: 514 - DNA, 120 bp, Artificial Sequence
  Synthetic polynucleotide
caggtatgactggcactatgtgatcttggacgaaggacacaaaattcgaaatccaaatgctgctgtcacccttgcttgcaaacaggtatgacctcttttaacaagggagatttccaagtg

SEQ ID NO: 515 - DNA, 120 bp, Artificial Sequence
  Synthetic polynucleotide
ttaataaaaaggtgcttcctttcctcaaatagtttcgcacccctcatcggatcattctgtctggctcaccgatgcaaaataacctccgagagctgtggtcgctctttgacttcatcttcc

SEQ ID NO: 516 - DNA, 120 bp, Artificial Sequence
  Synthetic polynucleotide
cgggaaagttaggcacgttgcctgtgtttatggagcagttctccgtccccatcaccatggggggatattcaaatgcttccccagtacaggtaaaatattaggatgataatacttttggca

SEQ ID NO: 517 - DNA, 120 bp, Artificial Sequence
  Synthetic polynucleotide
aggtcaaaactgcttacaagtgtgcatgtgtcttacgagataccataaatccatacctactgcggagaatgaagtcagatgtcaagatgagcctttctttgccagataaaaatgaacagg

SEQ ID NO: 518 - DNA, 120 bp, Artificial Sequence
  Synthetic polynucleotide
tcccgtccgtaggtcttattttgccgtcttacagatgagcagcataaagtctaccaaaatttcgttgattccaaagaagtttacaggattctcaatggagagatgcaggtcagctaaaaa

SEQ ID NO: 519 - DNA, 120 bp, Artificial Sequence
  Synthetic polynucleotide
ttcttaccacagattttctccggacttatagccctaagaaaaatttgcaaccaccctgatctcttttctggaggtcccaagaatctcaaaggtcttcctgatgatgaactagaagaagat

SEQ ID NO: 520 - DNA, 120 bp, Artificial Sequence
  Synthetic polynucleotide
cagtttgggtactggaaacgttctgggaaaatgattgttgttgagtctttgttgaaaatatggcacaagcagggtcagcgagtattgctgttttctcagtcaaggcaggtgagtgcacag

SEQ ID NO: 521 - DNA, 120 bp, Artificial Sequence
  Synthetic polynucleotide
acagatgctggacatacttgaagtattccttagagcccaaaagtatacctatctcaagatggatggtaccactacaatagcttcaagacagccactgattacgagatacaatgaggtaac

SEQ ID NO: 522 - DNA, 120 bp, Artificial Sequence
  Synthetic polynucleotide
ggctgagaactgtaactggtcttaagtgtgtgtgctcagtgttgtgtgtcttacctctaggacacatccatatttgtgtttcttctgaccacgcgggtgggcggcttaggtgtcaacctg

SEQ ID NO: 523 - DNA, 120 bp, Artificial Sequence
  Synthetic polynucleotide
acgggggcaaacagagttgtcatctatgacccagactggaacccaagcacggacacgcaggtttgtttttattttttttttaaaagaatgtattagtagaaatatagtttcatggttagc

SEQ ID NO: 524 - DNA, 120 bp, Artificial Sequence
  Synthetic polynucleotide
tctctgttgcaggcccgggagcgagcatggagaataggccagaagaagcaagtgactgtgtacaggctcctgactgcgggcaccattgaagaaaagatctaccaccggtcagtgcacaca

SEQ ID NO: 525 - DNA, 120 bp, Artificial Sequence
  Synthetic polynucleotide
gtagagctacacattgttttataccagcttatcttttatttttttagacaaatcttcaagcagtttttgacaaatagagtgctaaaagacccaaaacaaaggcggtttttcaaatccaat

SEQ ID NO: 526 - DNA, 120 bp, Artificial Sequence
  Synthetic polynucleotide
gatctctatgagctatttactctgactagtcctgatgcatcccagagcactgaaacaagtgcaatttttgcaggtattacataaaatcatttaatttaaagtaatcaattgcacaagatg

SEQ ID NO: 527 - DNA, 120 bp, Artificial Sequence
  Synthetic polynucleotide
ttacaggaactggatcagatgttcagacacccaaatgccatctaaaaagaaggattcaaccagcctttggagcagaccatgatgttccaaaacgcaagaagttccctgcttctaacatat

SEQ ID NO: 528 - DNA, 120 bp, Artificial Sequence
  Synthetic polynucleotide
ctgtaaatgatgccacatcatctgaagagaaatctgaggctaaaggagctgaagtaaatgcagtaacttctaatcgaagtgatcctttgaaagatgaccctcacatgagtagtaatgtaa

SEQ ID NO: 529 - DNA, 120 bp, Artificial Sequence
  Synthetic polynucleotide
ctagcaatgataggcttggagaagagacaaatgcagtatctggaccagaagagttgtcagtgattagtggaaatggggaatgttcaaattcttcaggaacaggcaaaacttctatgccat

SEQ ID NO: 530 - DNA, 120 bp, Artificial Sequence
  Synthetic polynucleotide
ctggtgatgaaagcattgatgaaaagttaggtctttcttacaaaagagaaagacccagccaggctcaaacagaagctttttgggagaataaacaaatggaaaataatttttataagcaca

SEQ ID NO: 531 - DNA, 120 bp, Artificial Sequence
  Synthetic polynucleotide
agtcaaaaacaaaacatcatagtgtggcagaagaagagaccctggagaaacatctgagaccaaagcaaaagcctaagaactctaagcattgcagagacgccaagtttgaaggaactcgaa

SEQ ID NO: 532 - DNA, 120 bp, Artificial Sequence
  Synthetic polynucleotide
ttccacacctggtgaagaaaaggcgttaccagaagcaagacagtgaaaacaagagtgaggccaaggaacagagcaatgacgattatgttttggaaaagcttttcaaaaaatcaggtaatc

SEQ ID NO: 533 - DNA, 120 bp, Artificial Sequence
  Synthetic polynucleotide
tatttcttttcttgctagttggcgtgcacagtgtcatgaagcacgatgccatcatggatggagccagcccagattatgtactggtggaggcagaagccaaccgagtggcccaggatgccc

SEQ ID NO: 534 - DNA, 120 bp, Artificial Sequence
  Synthetic polynucleotide
tgaaagcactgaggctctctcgtcagcggtgtctgggagcagtgtctggtgttcccacctggactggccacagggggatttctggtgcaccagcaggaaaaaagtaagagattgctgcat

SEQ ID NO: 535 - DNA, 120 bp, Artificial Sequence
  Synthetic polynucleotide
tgatgcttttccttttttaggagtagatttggtaagaaaaggaattctaacttctctgtgcagcatccttcatcaacatctccaacagagaagtgccaggtaatatagataacctttttg

SEQ ID NO: 536 - DNA, 120 bp, Artificial Sequence
  Synthetic polynucleotide
tatatcagtatagtggtcttctttttataggatggcatcatgaaaaaggagggaaaagataatgtccctgagcattttagtggaagagcagaagatgcagactcttcatccgggcccctc

SEQ ID NO: 537 - DNA, 120 bp, Artificial Sequence
  Synthetic polynucleotide
gcttcctcctcactcttggctaaaatgagagctagaaaccacctgattctgccagagcgtttagaaagtgaaagcgggcacctgcaggaagcttctgccctgctgcccaccacagaacac

SEQ ID NO: 538 - DNA, 120 bp, Artificial Sequence
  Synthetic polynucleotide
gatgaccttctggtggagatgagaaacttcatcgctttccaggcccacactgatggccaggccagcaccagggagatactgcaggagtttgaatccaagttatctgcatcacagtcttgt

SEQ ID NO: 539 - DNA, 120 bp, Artificial Sequence
  Synthetic polynucleotide
gtcttccgagaactattgagaaatctgtgcactttccatagaacttctggtggtgaaggaatttggaaactcaagccagaatactgctaaacaacattgcttcctaaactttcaagtccc

SEQ ID NO: 540 - DNA, 120 bp, Artificial Sequence
  Synthetic polynucleotide
ggtaactggaacccaatccgagggtcatggaggcatcccgaaggtttccggaagccgaggccttgagcccagagcaggctgctcattacctaaggtatgtctggaccgctgggcgggtct

SEQ ID NO: 541 - DNA, 120 bp, Artificial Sequence
  Synthetic polynucleotide
tctttttttttctatagatatgtgaaagaggccaaagaagcaactaagaatggagacctggaagaagcatttaaacttttcaatttggcaaaggacatttttcccaatgaaaaagtgctg

SEQ ID NO: 542 - DNA, 120 bp, Artificial Sequence
  Synthetic polynucleotide
gaagaaatatacaggaaatttgtgtctttagatcatatcaaggagttgctaatggagacgcgctcacctttggctgagctaggtgtcttaaagaagctgtgtgatcatcctaggctgctg

SEQ ID NO: 543 - DNA, 120 bp, Artificial Sequence
  Synthetic polynucleotide
tctgcacgggcttgttgtttgctaaatcttgggacattctctgctcaagatggaaatgagggggaagattccccagatgtggaccatattgatcaagtaactgatgacacattgatggaa

SEQ ID NO: 544 - DNA, 120 bp, Artificial Sequence
  Synthetic polynucleotide
gaatctggaaaaatgatattcctaatggacctacttaagaggctgcgagatgagggacatcaaactctggtgttttctcaatcgaggcaaattctaaacatcattgaacgcctcttaaag

SEQ ID NO: 545 - DNA, 120 bp, Artificial Sequence
  Synthetic polynucleotide
aataggcactttaagacattgcgaatcgatgggacagttactcatcttttggaacgagaaaaaagaattaacttattccagcaaaataaagattactctgtttttctgcttaccactcaa

SEQ ID NO: 546 - DNA, 120 bp, Artificial Sequence
  Synthetic polynucleotide
gtaggtggtgtcggtttaacattaactgcagcaactagagtggtcatttttgaccctagctggaatcctgcaactgatgctcaagctgtggatagagtttaccgaattggacaaaaagag

SEQ ID NO: 547 - DNA, 120 bp, Artificial Sequence
  Synthetic polynucleotide
aatgttgtggtttataggctaatcacttgtgggactgtagaggaaaaaatatacagaagacaggttttcaaggactcattaataagacaaactactggtgaaaaaaagaaccctttccga

SEQ ID NO: 548 - DNA, 120 bp, Artificial Sequence
  Synthetic polynucleotide
tattttagtaaacaagaattaagagagctctttacaatcgaggatcttcagaactctgtaacccagctgcagcttcagtctttgcatgctgctcagaggaaatctgatataaaactagat

SEQ ID NO: 549 - DNA, 120 bp, Artificial Sequence
  Synthetic polynucleotide
gaacatattgcctacctgcagtctttggggatagctggaatctcagaccatgatttgatgtacacatgtgatctgtctgttaaagaagagcttgatgtggtagaagaatctcactatatt

SEQ ID NO: 550 - DNA, 120 bp, Artificial Sequence
  Synthetic polynucleotide
caacaaagggttcagaaagctcaattcctcgttgaattcgagtctcaaaataaagagttcctgatggaacaacaaagaactagaaatgagggggcctggctaagagaacctgtatttcct

SEQ ID NO: 551 - DNA, 120 bp, Artificial Sequence
  Synthetic polynucleotide
tcttcaacaaagaagaaatgccctaaattgaataaaccacagcctcagccttcacctcttctaagtactcatcatactcaggaagaagatatcagttccaaaatggcaagtgtagtcatt

SEQ ID NO: 552 - DNA, 120 bp, Artificial Sequence
  Synthetic polynucleotide
agcagaatccaaaaaatacaggaagccttggaggagttggcagaacagggagatgatgaatttacagatgtgtgcaactctggcttgctactttatcgagaactgcacaaccaactcttt

SEQ ID NO: 553 - DNA, 120 bp, Artificial Sequence
  Synthetic polynucleotide
gatgatctgcccaaagagggtgagaaacaagatctctccagtataaaggtgaatgttaccaccttgcaagatggtaaaggtacaggtagtgctgactctatagctactttaccaaagggg

SEQ ID NO: 554 - DNA, 120 bp, Artificial Sequence
  Synthetic polynucleotide
tttggaagtgtagaagaactttgtactaactcttcattgggaatggaaaaaagctttgcaactaaaaatgaagctgtacaaaaagagacattacaagaggggcctaagcaagaggcactg

SEQ ID NO: 555 - DNA, 120 bp, Artificial Sequence
  Synthetic polynucleotide
caagaggatcctctggaaagttttaattatgtacttagcaaatcaaccaaagctgatattgggccaaatttagatcaactaaaggatgatgagattttacgtcattgcaatccttggccc

SEQ ID NO: 556 - DNA, 120 bp, Artificial Sequence
  Synthetic polynucleotide
attatttccataacaaatgaaagtcaaaatgcagaatcaaatgtatccattattgaaatagctgatgacctttcagcatcccatagtgcactgcaggatgctcaagcaagtgaggccaag

SEQ ID NO: 557 - DNA, 120 bp, Artificial Sequence
  Synthetic polynucleotide
ttggaagaggaaccttcagcatcttcaccacagtatgcatgtgatttcaatcttttcttggaagactcagcagacaacagacaaaatttttccagtcagtctttagagcatgttgagaaa

SEQ ID NO: 558 - DNA, 120 bp, Artificial Sequence
  Synthetic polynucleotide
gaaaatagcttgtgtggctctgcacctaattccagagcagggtttgtgcatagcaaaacatgtctcagttgggagttttctgagaaagacgatgaaccagaagaagtagtagttaaagca

SEQ ID NO: 559 - DNA, 120 bp, Artificial Sequence
  Synthetic polynucleotide
aaaatcagaagtaaagctagaaggattgtttcagatggcgaagatgaagatgattcttttaaagatacctcaagcataaatccattcaacacatctctctttcaattctcatctgtgaaa

SEQ ID NO: 560 - DNA, 120 bp, Artificial Sequence
  Synthetic polynucleotide
caatttgatgcttcaactcccaaaaatgacatcagtccaccaggaaggttcttttcatctcaaatacccagtagtgtaaataagtctatgaactctagaagatctctggcttctaggagg

SEQ ID NO: 561 - DNA, 120 bp, Artificial Sequence
  Synthetic polynucleotide
tctcttattaatatggttttagaccacgtggaggacatggaggaaagacttgacgacagcagtgaagcaaagggtcctgaagattatccagaagaaggggtggaggaaagcagtggcgaa

SEQ ID NO: 562 - DNA, 120 bp, Artificial Sequence
  Synthetic polynucleotide
gcctccaagtatacagaagaggatccttccggagaaacactgtcttcagaaaacaagtccagctggttaatgacgtctaagcctagtgctctagctcaagagacctctcttggtgcccct

SEQ ID NO: 563 - DNA, 120 bp, Artificial Sequence
  Synthetic polynucleotide
gagcaccagaaggaaggcatagctttcctctatagcctgtatagggatggaagaaaaggtggtatattggctgatgatatgggattagggaagactgttcaaatcattgctttcctttcc

SEQ ID NO: 564 - DNA, 120 bp, Artificial Sequence
  Synthetic polynucleotide
gagcctttgtctggtgaacagttggttggttctccccaggataaggcggcagaggctacaaatgactatgagactcttgtaaagcgtggaaaagaactaaaagagtgtggaaaaatccag

SEQ ID NO: 565 - DNA, 120 bp, Artificial Sequence
  Synthetic polynucleotide
gaggccctaaactgcttagttaaagcgcttgacataaaaagtgcagatcctgaagttatgctcttgactttaagtttgtataagcaacttaataacaattgagaatgtaacctgtttatt

SEQ ID NO: 566 - DNA, 120 bp, Artificial Sequence
  Synthetic polynucleotide
ggtatgtttgatgcatcacttgtgaatcatgtgctgctgatcatgccaaccaatcttattaacacatgggtaaaagaattcatcaagtggactccaggaatgagagtcaaaacctttcat

SEQ ID NO: 567 - DNA, 120 bp, Artificial Sequence
  Synthetic polynucleotide
ggtcctagcaaggatgaacggaccagaaacctcaatcggattcagcaaaggaatggtgttattatcactacataccaaatgttaatcaataactggcagcaactttcaagctttaggggc

SEQ ID NO: 568 - DNA, 120 bp, Artificial Sequence
  Synthetic polynucleotide
caagagtttgtgtgggactatgtcatcctcgatgaagcacataaaataaaaacctcatctactaagtcagcaatatgtgctcgtgctattcctgcaagtaatcgcctcctcctcacagga

SEQ ID NO: 569 - DNA, 120 bp, Artificial Sequence
  Synthetic polynucleotide
accccaatccagaataatttacaagaactatggtccctatttgattttgcttgtcaagggtccctgctgggaacattaaaaacttttaagatggagtatgaaaatcctattactagagca

SEQ ID NO: 570 - DNA, 120 bp, Artificial Sequence
  Synthetic polynucleotide
agagagaaggatgctaccccaggagaaaaagccttgggatttaaaatatctgaaaacttaatggcaatcataaaaccctattttctcaggaggactaaagaagacgtacagaagaaaaag

SEQ ID NO: 571 - DNA, 120 bp, Artificial Sequence
  Synthetic polynucleotide
tcaagcaacccagaggccagacttaatgaaaagaatccagatgttgatgccatttgtgaaatgccttccctttccaggaaaaatgatttaattatttggatacgacttgtgcctttacaa

SEQ ID NO: 572 - DNA, 120 bp, Artificial Sequence
  Synthetic polynucleotide
cgccgccttccgggtgttacatgcagccgggctcggcccctccccctggccggatggatccgtcggcgccacagccccgcgcggaaacctcaggcaaaggtaccagctccgcgctcgccc

SEQ ID NO: 573 - DNA, 120 bp, Artificial Sequence
  Synthetic polynucleotide
ggaaactttattttctttattcttgcagacatatggcatccaggagaaagatgtcttgccccttctccagataatggaaaactttgtgaagcaagcataaaatctatcacagtggatgaa

SEQ ID NO: 574 - DNA, 120 bp, Artificial Sequence
  Synthetic polynucleotide
aatggcaagtcatttgcagtcgtcttatatgcagattttcaagaaaggaaaatacctcttaaacagcttcaagaagtgaaatttgttaaagattgccctaggaatcttatatttgatgat

SEQ ID NO: 575 - DNA, 120 bp, Artificial Sequence
  Synthetic polynucleotide
gaagatttagaaaaaccttatttcccaaaccgaaaatttccatcatcttctgttgcttttaaattatctgacaatggagactctattccttataccatcaataggtatttgagagactac

SEQ ID NO: 576 - DNA, 120 bp, Artificial Sequence
  Synthetic polynucleotide
caaagagaaggaacccggtttctttatggacactacatccatggaggagggtgcattctgggtgatgacatgggacttggaaaaacagtacaggtatttaattatgttataacagtaaag

SEQ ID NO: 577 - DNA, 120 bp, Artificial Sequence
  Synthetic polynucleotide
aaattttgtacgtcatgatacattatacacagtgattgaaaaagtcttttttccccaggttatttcatttctggctgcagttttgcataaaaagggaactcgtgaggatattgaaaataa

SEQ ID NO: 578 - DNA, 120 bp, Artificial Sequence
  Synthetic polynucleotide
catgccagagtttttactaagaagtatgaaaaaggaacccctttcttctacagcaaaaaaggtaaaatctctagacaatgtatattctactcatgatgctggtattacaaaagcatatag

SEQ ID NO: 579 - DNA, 120 bp, Artificial Sequence
  Synthetic polynucleotide
aaatttttttattcttgttttagatgttcttaatagttgctcctctttctgtcctctacaactggaaggatgaattggacacctggggatatttcagagtcactgttttacatggaaaca

SEQ ID NO: 580 - DNA, 120 bp, Artificial Sequence
  Synthetic polynucleotide
gaaaagataatgaattaattcgtgtaaagcagaggaaatgtgaaattgctctaacaacttatgaaacactacgcttatgcctggatgaacttaacaggtaatgggaataataggaatagg

SEQ ID NO: 581 - DNA, 120 bp, Artificial Sequence
  Synthetic polynucleotide
gttttctcaacctcacccttcttttttcttactttatagtttggaatggtcagctgtcattgtggatgaagctcatagaatcaagaatccaaaagctagagtaacagaagttatgaaagc

SEQ ID NO: 582 - DNA, 120 bp, Artificial Sequence
  Synthetic polynucleotide
tttgaaatgtaatgtccgcattggcctcactggaaccatccttcagaacaacatgaaggaactgtggtgtgttatggactggtgagagaaaacactttttaaaaaattgtttaatagttc

SEQ ID NO: 583 - DNA, 120 bp, Artificial Sequence
  Synthetic polynucleotide
tattgtctttataaagggctgtgccaggccttttagggagtgggacctacttcaagaagcagttttctgacccagtagaacatggtcagagacacacggcaacaaagagagaactagcca

SEQ ID NO: 584 - DNA, 120 bp, Artificial Sequence
  Synthetic polynucleotide
ctggccgaaaggccatgcaaagacttgccaaaaagatgtctggctggtttctcaggcgcaccaagactcttatcaaggatcagttgcctaagaaggaagaccgggtaagaaccgcatttg

SEQ ID NO: 585 - DNA, 120 bp, Artificial Sequence
  Synthetic polynucleotide
tattgttataaacaaaatactaataactaccttgtattttatcttggcagatggtgtattgttctttgacagatttccagaaagctgtctatcaaacagtgttagaaacagaggacgtga

SEQ ID NO: 586 - DNA, 120 bp, Artificial Sequence
  Synthetic polynucleotide
ctttgatacttcaatcttctgagccttgtacctgtaggagtggccaaaaaaggagaaattgttgttataaggcaagcatttcaatatatctttataatcatgcttttgattacatagtac

SEQ ID NO: 587 - DNA, 120 bp, Artificial Sequence
  Synthetic polynucleotide
cagaccaattctcatggtgaaacagtgaaaaccttgtatctcagttaccttacagtccttcagaaggtagctaaccatgtcgcgctactgcaagctgctagtacttccaaacaacaggtt

SEQ ID NO: 588 - DNA, 120 bp, Artificial Sequence
  Synthetic polynucleotide
attatttcaatttatacaggtttgaatgtgttaagtggaaatatcttttcttctgccttttcccttcaaggaaacacttatcaaaaggatatgtgatcaggtattttccagattcccaga

SEQ ID NO: 589 - DNA, 119 bp, Artificial Sequence
  Synthetic polynucleotide
ttttgtgcagaaaagcaaagatgcagcctttgaaacactttctgaccctaaatacagtggaaaaatgaaggtaagtgctcctctttcaggttgcatacagacatgatacacaaaatatt

SEQ ID NO: 590 - DNA, 120 bp, Artificial Sequence
  Synthetic polynucleotide
tgattttctgtggttcattttcaggtccttcagcagcttttaaatcattgcaggaaaaacagagataaagttcttctcttttctttttccaccaaggtgagttcatctaaagtatatcct

SEQ ID NO: 591 - DNA, 120 bp, Artificial Sequence
  Synthetic polynucleotide
tacttaaccaagattcatgtttgcccatcttcatacctctcgtctagttgcttgacgtgctacagcagtactgtatggcgtctgggcttgattaccgacgacttgatggaagtacaaaat

SEQ ID NO: 592 - DNA, 120 bp, Artificial Sequence
  Synthetic polynucleotide
cagaggaaagactcaagattgtaaaagagttcaacagtacacaagatgttaacatttgccttgtctctacaatgtaagaaaattaaatttaataactagatttttatccaattgtttttg

SEQ ID NO: 593 - DNA, 120 bp, Artificial Sequence
  Synthetic polynucleotide
tctttcctccagggctggtggactaggcctcaattttgtcggtgccaatgttgttgtattatttgatcctacttggaatccagccaatgatcttcaagccattgacaggtataatactga

SEQ ID NO: 594 - DNA, 120 bp, Artificial Sequence
  Synthetic polynucleotide
ccttttacagagcatataggattggacaatgtagagatgtcaaagtgcttaggctgatatccttgggaactgtggaggaaatcatgtatttacgacagatatacaagcaggtaaatatgt

SEQ ID NO: 595 - DNA, 120 bp, Artificial Sequence
  Synthetic polynucleotide
gcaaacacttcaaaaatgtcttgtgttttttctgttttagcaacttcactgtgtggtggttggaagtgaaaatgccaaacgatattttgaagcagttcaaggatctaaagagcatcaagg

SEQ ID NO: 596 - DNA, 120 bp, Artificial Sequence
  Synthetic polynucleotide
agagctttttgggatccataacctcttcaaatttaggtcccaagggtcttgtcttacgaaggacatcctggaggtgtgaacttcttctctgaccttttcaataatattttaaatacagtt

SEQ ID NO: 597 - DNA, 120 bp, Artificial Sequence
  Synthetic polynucleotide
ttttcttcatcttttttttctctcttagcaccttctagccaccatggcaacctcatctgaagaagttttgctgattgtaaagaaagtgcgtcaaaagaagcaggatggagctctgtacct

SEQ ID NO: 598 - DNA, 120 bp, Artificial Sequence
  Synthetic polynucleotide
catggcagaaagaattgcttgggcacctgaaggcaaagatagatttacaatcagccatatgtatgcagatattaaatgtaagtcagctatactaagttctgatgtatttgtatgtcatag

SEQ ID NO: 599 - DNA, 120 bp, Artificial Sequence
  Synthetic polynucleotide
aactgccctcatgcttctttttaggccagaaaattagtccagaaggaaaagctaaaattcagcttcagctggtcctacatgcaggggacacaactaacttccatttttccaatgaaagca

SEQ ID NO: 600 - DNA, 120 bp, Artificial Sequence
  Synthetic polynucleotide
cagcagtgaaagagcgagatgcagtaaaagaccttcttcagcagctgctgcccaaattcaagaggaaagcaaataaagaactggaagagaagaacaggtgggaggaaaagaatagccttt

SEQ ID NO: 601 - DNA, 120 bp, Artificial Sequence
  Synthetic polynucleotide
agaagttcagttatattcagtatattctgctttacagaatgctgcaagaagatcctgttttgtttcagctttataaagaccttgttgtgagtcaagtgatcagtgctgaggaattctggg

SEQ ID NO: 602 - DNA, 120 bp, Artificial Sequence
  Synthetic polynucleotide
ccaatcgtttaaatgtgaatgcaacagatagttcttccacatccaatcataagcaggatgttggcatttctgctgcatttctggtatgtgagccttctagatttctgaagaaaataaaaa

SEQ ID NO: 603 - DNA, 120 bp, Artificial Sequence
  Synthetic polynucleotide
ggctttgttttaggctgatgtccggccccaaactgatggctgtaacggtctaagatataatttaacttctgatatcattgagtccatatttaggacctatccagcaggtaagaagaatca

SEQ ID NO: 604 - DNA, 120 bp, Artificial Sequence
  Synthetic polynucleotide
aaaatggaaattcagtatataatatttgtgggtttttttccacagtaaaaatgaaatatgcagaaaatgttccccacaacatgacagagaaggaattctggacacgttttttccagtccc

SEQ ID NO: 605 - DNA, 120 bp, Artificial Sequence
  Synthetic polynucleotide
attattttcacagggatcggctgaatacagggtcaaaggatctctttgcagaatgtgccaaaatagatgaaaaaggtaactgtttatctctgatagacactggtatttaacttgccaccc

SEQ ID NO: 606 - DNA, 120 bp, Artificial Sequence
  Synthetic polynucleotide
ttattttgttgattttctaggcctaaaaacaatggtttcattaggagtgaaaaacccactactagatttaacagctttggaagataaaccattagatgaggtaagaagcaataaaagaag

SEQ ID NO: 607 - DNA, 120 bp, Artificial Sequence
  Synthetic polynucleotide
tataataagaaaagcagaacctttttaaaaaatttttaatctattatttctcacagggctatggcatttcctctgtgccatctgcttccaattctaaatccataaaagagaatagtaatg

SEQ ID NO: 608 - DNA, 120 bp, Artificial Sequence
  Synthetic polynucleotide
ctgccatcatcaagagatttaaccatcacagtgccatggtcctggcagctggactcagaaaacagttaagtataaatgcagaggtgcagtaactgggcttttcaggatatccagatggag

SEQ ID NO: 609 - DNA, 120 bp, Artificial Sequence
  Synthetic polynucleotide
tcccctttattttaagagaagcacaaaatgaacaaactagtgagcccagcaacatggatggaaattccggagatgcagactgctttcagccagcagtcaaaagggtatgggcaaaaaaat

SEQ ID NO: 610 - DNA, 120 bp, Artificial Sequence
  Synthetic polynucleotide
gtgttaataattataggcgaaattacaagagtccattgaatatgaagacttggggaaaaataattctgtaaaaacgattgcactaaacctcaagaagtcagataggtaagtttggtcaat

SEQ ID NO: 611 - DNA, 120 bp, Artificial Sequence
  Synthetic polynucleotide
ggtattatcatggtccaactccaatccagtcactacagtatgcaacaagtcaggacattattaattcttttcaaagtattagacaagaaatggaagcttatacacccaagttaactcagg

SEQ ID NO: 612 - DNA, 120 bp, Artificial Sequence
  Synthetic polynucleotide
ttcatttttttcaggttctctcaagtagtgctgccagtagtaccatcacagcactgtcacctggaggggcacttatgcagggaggaacacagcaagccataaaccgtatgtgccgggcca

SEQ ID NO: 613 - DNA, 120 bp, Artificial Sequence
  Synthetic polynucleotide
agagatggtgccaaatgatattcaatctgaattgaaacacttatatgtagctgttggagaacttctacgacatttctggtcctgctttcctgttaatacgccattcctagaagaaaaggt

SEQ ID NO: 614 - DNA, 120 bp, Artificial Sequence
  Synthetic polynucleotide
ctcatcttttttaggtagtgaaaatgaaaagtaatttggaacgattccaagttacgaagctctgtccattccaagaaaagattcggagacagtatttaagcacaaatgtaaggcagcaat

SEQ ID NO: 615 - DNA, 120 bp, Artificial Sequence
  Synthetic polynucleotide
ttgctgtgtttttcagttggtaagtcacatagaagagatgctccagacagcctacaacaagctccacacatggcagtcacggcgtctgatgaagaaaacgtgaggtggccatgatgctta

SEQ ID NO: 616 - DNA, 120 bp, Artificial Sequence
  Synthetic polynucleotide
ttttacagattattgaataataaaatacagttttgaaaaaaatggatgaagaacctgaaagaactaagcgatgggaaggaggctatgaaagaacatggtaaggagagctttattgccctg

SEQ ID NO: 617 - DNA, 120 bp, Artificial Sequence
  Synthetic polynucleotide
aacaaataattatgacttatagggagattcttaaagaagatgaatctggatcacttaaagctacaatagaagacattctattcaaggcaaagagaaaaaggtatgtaaccttcctatgta

SEQ ID NO: 618 - DNA, 120 bp, Artificial Sequence
  Synthetic polynucleotide
agtatatggaattacattaaaatgtttgtataattttaacagagtatttgagcaccatggacaagttcgacttggaatggtatgtcattattttttcttttactagtacagaactagttt

SEQ ID NO: 619 - DNA, 120 bp, Artificial Sequence
  Synthetic polynucleotide
ttcttttttccgatagatgcgccacctttatgtggtagtagatggatcaagaacaatggaagaccaagatttaaagcctaatagactgacgtgtactttaaaggtaaaatttaagtttat

SEQ ID NO: 620 - DNA, 120 bp, Artificial Sequence
  Synthetic polynucleotide
cctttatctagtatgtctttttttgtttaaacagttgttggaatactttgtagaggaatattttgatcaaaatcctattagtcaggtacgtatctaagtgatagaattcagaattagatt

SEQ ID NO: 621 - DNA, 120 bp, Artificial Sequence
  Synthetic polynucleotide
atattaataataatttttgtttttatttcaagattggaataattgtaactaagagtaaaagagctgaaaaattgactgaactttcaggtatgcataaaattacctttacatgactcaagg

SEQ ID NO: 622 - DNA, 120 bp, Artificial Sequence
  Synthetic polynucleotide
attttaggaaacccaagaaaacatataacgtctttgaagaaagctgtggatatgacctgccatggagagccatctctttataattccctaagcatagctatgcagactctaaagttagta

SEQ ID NO: 623 - DNA, 120 bp, Artificial Sequence
  Synthetic polynucleotide
atctttcttttaagacacatgcctggacatacaagtcgagaagtactaatcatctttagcagccttacaacttgcgatccatctaatatttatgatctaatcaaggtagaccaaaaaatc

SEQ ID NO: 624 - DNA, 120 bp, Artificial Sequence
  Synthetic polynucleotide
cttggattttatgaagaccctaaaggcagctaaaattagagtatctgttattggattgtctgcagaagttcgcgtttgcactgtacttgctcgtgaaactggtggtatatatataattta

SEQ ID NO: 625 - DNA, 120 bp, Artificial Sequence
  Synthetic polynucleotide
tgttaggcacgtaccatgttattttagatgaaagccattacaaagagttgctcacacatcatgttagtcctcctcctgctagctcaagttctgaatgctcacttattcgtatgggtaagt

SEQ ID NO: 626 - DNA, 120 bp, Artificial Sequence
  Synthetic polynucleotide
agaaagtaatacattttcttctatgaaggatttcctcagcacaccattgcttctttatctgaccaggatgcaaaaccctctttcagcatggcgtaagtaaagaccttgaaaatatcagtg

SEQ ID NO: 627 - DNA, 120 bp, Artificial Sequence
  Synthetic polynucleotide
ccctacaggcatttggatggcaatactgagccagggcttacattaggaggctatttctgcccacagtgtcgggcaaagtactgtgagctacctgttgagtgtaaaatctgtggtaagaaa

SEQ ID NO: 628 - DNA, 120 bp, Artificial Sequence
  Synthetic polynucleotide
tgtgttaggtcttactttggtgtctgctccccacttggcacggtcttaccatcatttgtttcctttggatgcttttcaagaaattcccctagaagaatataatggagaaaggtatttcag

SEQ ID NO: 629 - DNA, 120 bp, Artificial Sequence
  Synthetic polynucleotide
gtaaattctaagaaaaaacattgttaaacttttttttcagattttgttatggatgtcagggggaattgaaagaccaacatgtaagttctttggctttctaaatattaagtaatgtacaag

SEQ ID NO: 630 - DNA, 120 bp, Artificial Sequence
  Synthetic polynucleotide
tagctgtgctgtaattaacttttggaaactagtttatcacttttcttcttttcactacaggtttatgtttgtgctgtgtgccaaaatgttttctgtgtggactgtgatgtttttgttcat

SEQ ID NO: 631 - DNA, 120 bp, Artificial Sequence
  Synthetic polynucleotide
gattctctacactgttgccctggctgtattcataagattccagctccttcaggtgtttgattccagcatgtagtatacattgtatgtgttaaaaagaaatttgcaactgtgaataaaagg

SEQ ID NO: 632 - DNA, 120 bp, Artificial Sequence
  Synthetic polynucleotide
tttgagacgctcccctgaccaccacttgctctgcgctgaggtgctgggacagccatggtttcagacggtgaggaccctgcagggcgggacttcgactccggggctcggctgtctcggtcc

SEQ ID NO: 633 - DNA, 120 bp, Artificial Sequence
  Synthetic polynucleotide
tttcttgttaatattttcagaagatgaattgaatcttctggttattgtagttgatgccaacccaatttggtggggaaagcaagcattaaaggaatctcaggtaagactgcttgaggaggc

SEQ ID NO: 634 - DNA, 120 bp, Artificial Sequence
  Synthetic polynucleotide
caacagttcactttatccaaatgcatagatgccgtgatggtgctgggaaattcgcatttattcatgaatcgttccaacaaacttgctgtgatagcaagtcacattcaagaaaggtatgac

SEQ ID NO: 635 - DNA, 120 bp, Artificial Sequence
  Synthetic polynucleotide
ggcctggtgtaaccaggttttttcccctgctgtttcagccgattcttatatcctggaaagaatggcagacttggagacttcttcggagaccctggcaaccctcctgaatttaatccctct

SEQ ID NO: 636 - DNA, 120 bp, Artificial Sequence
  Synthetic polynucleotide
gggagtaaagatggaaaatacgaacttttaacctcagcaaatgaagttattgttgaagagattaaagatctaatgaccaaaagtaacaacttttaaacattgttattttgcaaatagtgt

SEQ ID NO: 637 - DNA, 120 bp, Artificial Sequence
  Synthetic polynucleotide
cccttttaatgttttctgttatttgcaggtgacataaagggtcaacatacagaaactttgctggcaggatccctggccaaagccctttgctgtatccttggtgtctgaatcatttagaag

SEQ ID NO: 638 - DNA, 120 bp, Artificial Sequence
  Synthetic polynucleotide
ttatgaagcaaaataatatttttgtattccttaatgttaagaaattaagacattcatagaatgaacaaggaagttaaaggtaagagcctacgttttcctatgagaactgtaatcctactt

SEQ ID NO: 639 - DNA, 120 bp, Artificial Sequence
  Synthetic polynucleotide
ttagtaagatttagttaaatttttttctgcttttttctctttgtagacaatcaggaaatgaaatcaaggatattggtaagataaaaaaatcattacttttttatatgacaactataatta

SEQ ID NO: 640 - DNA, 120 bp, Artificial Sequence
  Synthetic polynucleotide
ttaacatgactgtgatttttaggtgattaaggctgcagaagacagtgcgttgcagtatatgaacttcatgaatgtcatctttgcagcacagaaacaggtgaactgagagcctgccgttta

SEQ ID NO: 641 - DNA, 120 bp, Artificial Sequence
  Synthetic polynucleotide
attcctgtaatattttcaaaatgtttcttttagaatattttgattgatgcctgtgttttagactccgactcagggctcctccaacaggtatgttttaaaaccatgctttgtgtcggtggt

SEQ ID NO: 642 - DNA, 120 bp, Artificial Sequence
  Synthetic polynucleotide
ggcagcaagccgcctgtgtcttgcaggcttgtgacatcacgggaggactgtacctgaaggtgcctcagatgccttctcttctgcagtatttgctggtaaggagacagcagcggcgaccct

SEQ ID NO: 643 - DNA, 120 bp, Artificial Sequence
  Synthetic polynucleotide
atttttttcccatgttttaaataaaagtttcttttgtttgtttgttttacagtgggtgtttcttcccgatcaagatcagagatctcagttaatcctcccacccccagttcatgttgacta

SEQ ID NO: 644 - DNA, 120 bp, Artificial Sequence
  Synthetic polynucleotide
cagggctgcttgcttctgtcatcgaaatctcattgaaattggttatgtctgttctgtgtgtttgtcaagtaagttaatgtacctagtttttcttttttttctatgttggggggcaggaaa

SEQ ID NO: 645 - DNA, 120 bp, Artificial Sequence
  Synthetic polynucleotide
ttttcagccaccctattgtttctttttttttttaatttacagtattctgcaatttcagccccatttgtactacgtgcgagtaagtatctttgagattgtgtgggtggctaatacttcaca

SEQ ID NO: 646 - DNA, 120 bp, Artificial Sequence
  Synthetic polynucleotide
aatgttttcctctctgtaatttcaggacagcctttaaaatttctctgcctccagtgctgaaagccaagaaaaagaaactgaaagtgtctgcctgaggataaaatattttccccatctttt

SEQ ID NO: 647 - DNA, 120 bp, Artificial Sequence
  Synthetic polynucleotide
acactggcatggatggtgaggttgcacttctgacgtttgcattcctcaggtgatggagagcaccccttcaaggggactgaaccgagtacacctacaatgcaggaatctgcaggaattctt

SEQ ID NO: 648 - DNA, 120 bp, Artificial Sequence
  Synthetic polynucleotide
agggggcctgagccctggggtattggaccgattgtatgggcaccctgccacatgtctggctgtcttcaggtgagaagccccttcatggcagggaaatgtaatggggtctgcggagtggaa

SEQ ID NO: 649 - DNA, 120 bp, Artificial Sequence
  Synthetic polynucleotide
ctgtacagggagctcccatccttggctaagaactgggtgatgcggatgctctttctggagcagcctttgccacaggctgctgtagctctgtgggtaaagaaggaattcagcaagtaagtc

SEQ ID NO: 650 - DNA, 120 bp, Artificial Sequence
  Synthetic polynucleotide
gggcctcctttttgttttccaaataccctactcacctctctgcttctgttccagggctcaggaggaaagtacagggctgctgagcggcctccggatctggcacacacagctgctcccagg

SEQ ID NO: 651 - DNA, 120 bp, Artificial Sequence
  Synthetic polynucleotide
cgggctccagggcctcatcctcaaccccattttccgccagaacctccgcattgcccttctgggtgggtatgtcacttctctctcttcctaagctagggcaggggaactgctgcttattaa

SEQ ID NO: 652 - DNA, 120 bp, Artificial Sequence
  Synthetic polynucleotide
cctggccgtagggggaaggcctggtctgatgacacaagtcagctgggaccagacaagcatgcccgggacgttccctcccttgacaagtacgccgaggagcgatgggaggtaagcacttgg

SEQ ID NO: 653 - DNA, 120 bp, Artificial Sequence
  Synthetic polynucleotide
ctcttctgttcttcaggtggtcttgcacttcatggtgggctcccccagtgcagctgtcagccaggacttggctcagctcctcagccaggctgggctcatgaagaggtgaggaagccggag

SEQ ID NO: 654 - DNA, 120 bp, Artificial Sequence
  Synthetic polynucleotide
ctagtactgaacctggagagccgccctgcattacttccgctggcttccagttcctgttgctggacaccccggctcagctctggtactttatgttgcagtatttgcagacagcccaggtga

SEQ ID NO: 655 - DNA, 120 bp, Artificial Sequence
  Synthetic polynucleotide
tttgtctctgcctctttctccctagagccggggcatggacctggtagagattctctccttcctcttccagctcagcttctctactctgggcaaggtaagcagggggctgaaaggtataga

SEQ ID NO: 656 - DNA, 120 bp, Artificial Sequence
  Synthetic polynucleotide
gaaacctctgttcctcaggattactctgtggaaggtatgagtgattctctgttgaacttcctgcaacatctgcgtgagtttgggcttgttttccagaggaaggtatgagcgcctagataa

SEQ ID NO: 657 - DNA, 120 bp, Artificial Sequence
  Synthetic polynucleotide
agatgtaaggcagtgacttctgagacaaggcatctgcctttctattcttttcagaggaaatctcggcgttactaccccacacgcctggccatcaatctctcatcaggtgtctctggagct

SEQ ID NO: 658 - DNA, 120 bp, Artificial Sequence
  Synthetic polynucleotide
gggggcactgtgcatcagccaggtttcattgtcgtggaaaccaattaccgactgtatgcctacacgggtgaggcgggacagagggcccctggaagaggaggttgggggtgagggaatgcc

SEQ ID NO: 659 - DNA, 120 bp, Artificial Sequence
  Synthetic polynucleotide
agggagtctgggtgtgggggtggcctcctcatcctctttctatccctggctcagagtcggagctgcagattgccctcattgccctcttctctgagatgctctatcggttccccaacatgg

SEQ ID NO: 660 - DNA, 120 bp, Artificial Sequence
  Synthetic polynucleotide
tggtggcgcaggtgacccgggagagtgtgcagcaggcaatcgccagtggcatcacagcccagcaggtattcccacttgggagaggtggagcaggaagacaggctgcacttgggctgcggg

SEQ ID NO: 661 - DNA, 120 bp, Artificial Sequence
  Synthetic polynucleotide
tcttgctggagccctcatgccattcttgtctgttttcctagataatccatttcctaaggacaagagcccacccagtgatgctcaaacaggtatagacaggctccaagatgtcagaggctg

SEQ ID NO: 662 - DNA, 120 bp, Artificial Sequence
  Synthetic polynucleotide
gcagctggtgatgacatgatggaaaagaaaaaggggcatccaaatctggggaagaaacagagggccgggttgtctggggcagtattctgagtccctacagtcaacccttgctccttgcag

SEQ ID NO: 663 - DNA, 120 bp, Artificial Sequence
  Synthetic polynucleotide
acacctgtgctgccccccaccatcaccgaccagatccggctctgggagctggaaagggacagactccggttcactgagggtgagtagcttctggtggccaagtcttggtcattggccaga

SEQ ID NO: 664 - DNA, 120 bp, Artificial Sequence
  Synthetic polynucleotide
tctccccgcgcccctcccgtcctgccgaccccaggtgtcctgtataaccagttcctgtcgcaagtggactttgagctgctgctggcccacgcgcgggagctgggcgtgctcgtgttcgag

SEQ ID NO: 665 - DNA, 120 bp, Artificial Sequence
  Synthetic polynucleotide
aactcggccaagcggctcatggtggtgaccccggccgggcacagcgacgtcaagcgcttttggaagcggcagaaacatagctcctgagagcgcgggacttggacacggacctcggcgggc

SEQ ID NO: 666 - DNA, 120 bp, Artificial Sequence
  Synthetic polynucleotide
tttattagcattcttcaggtcatctgaaccttctgagaaaacatggtcaacgtcttgaaaggagtgcttatagaatggttagtagttttgatactgcatgagttttaagtttaaatattg

SEQ ID NO: 667 - DNA, 120 bp, Artificial Sequence
  Synthetic polynucleotide
tgtcttacaatcatgtgtttgtctttacagtgatcctgccatgaagcagtttctgctgtacttggatgagtccaatgccctggggaagaagttcatcattcaagacattgatgacactca

SEQ ID NO: 668 - DNA, 120 bp, Artificial Sequence
  Synthetic polynucleotide
cgtctttgtaatagcagaattggttaatgtcctccaggagcgagtgggtgaattaatggaccaaaatgctttttcccttacccagaaatgaaaatactcaatatggaccatttaggaatt

SEQ ID NO: 669 - DNA, 120 bp, Artificial Sequence
  Synthetic polynucleotide
caggacccgcttctctgaaaggctctccttgcagctgcttagacgctggatttttttcgggtagtggaaaaccaggtaagcaccgaagtccacttgccttttaatttatttttttatcac

SEQ ID NO: 670 - DNA, 120 bp, Artificial Sequence
  Synthetic polynucleotide
aagactgcctcccgctttgtgtgccccgctccagcagcctcccgcgacgatgcccctcaacgttagcttcaccaacaggaactatgacctcgactacgactcggtgcagccgtatttcta

SEQ ID NO: 671 - DNA, 120 bp, Artificial Sequence
  Synthetic polynucleotide
ctgcgacgaggaggagaacttctaccagcagcagcagcagagcgagctgcagcccccggcgcccagcgaggatatctggaagaaattcgagctgctgcccaccccgcccctgtcccctag

SEQ ID NO: 672 - DNA, 120 bp, Artificial Sequence
  Synthetic polynucleotide
ccgccgctccgggctctgctcgccctcctacgttgcggtcacacccttctcccttcggggagacaacgacggcggtggcgggagcttctccacggccgaccagctggagatggtgaccga

SEQ ID NO: 673 - DNA, 120 bp, Artificial Sequence
  Synthetic polynucleotide
gctgctgggaggagacatggtgaaccagagtttcatctgcgacccggacgacgagaccttcatcaaaaacatcatcatccaggactgtatgtggagcggcttctcggccgccgccaagct

SEQ ID NO: 674 - DNA, 120 bp, Artificial Sequence
  Synthetic polynucleotide
cgtctcagagaagctggcctcctaccaggctgcgcgcaaagacagcggcagcccgaaccccgcccgcggccacagcgtctgctccacctccagcttgtacctgcaggatctgagcgccgc

SEQ ID NO: 675 - DNA, 120 bp, Artificial Sequence
  Synthetic polynucleotide
cgcctcagagtgcatcgacccctcggtggtcttcccctaccctctcaacgacagcagctcgcccaagtcctgcgcctcgcaagactccagcgccttctctccgtcctcggattctctgct

SEQ ID NO: 676 - DNA, 120 bp, Artificial Sequence
  Synthetic polynucleotide
ctcctcgacggagtcctccccgcagggcagccccgagcccctggtgctccatgaggagacaccgcccaccaccagcagcgactctggtaagcgaagcccgcccaggcctgtcaaaagtgg

SEQ ID NO: 677 - DNA, 120 bp, Artificial Sequence
  Synthetic polynucleotide
ctatttcctttcttaaagaggaggaacaagaagatgaggaagaaatcgatgttgtttctgtggaaaagaggcaggctcctggcaaaaggtcagagtctggatcaccttctgctggaggcc

SEQ ID NO: 678 - DNA, 120 bp, Artificial Sequence
  Synthetic polynucleotide
acagcaaacctcctcacagcccactggtcctcaagaggtgccacgtctccacacatcagcacaactacgcagcgcctccctccactcggaaggactatcctgctgccaagagggtcaagt

SEQ ID NO: 679 - DNA, 120 bp, Artificial Sequence
  Synthetic polynucleotide
tggacagtgtcagagtcctgagacagatcagcaacaaccgaaaatgcaccagccccaggtcctcggacaccgaggagaatgtcaagaggcgaacacacaacgtcttggagcgccagagga

SEQ ID NO: 680 - DNA, 120 bp, Artificial Sequence
  Synthetic polynucleotide
ggaacgagctaaaacggagcttttttgccctgcgtgaccagatcccggagttggaaaacaatgaaaaggcccccaaggtagttatccttaaaaaagccacagcatacatcctgtccgtcc

SEQ ID NO: 681 - DNA, 120 bp, Artificial Sequence
  Synthetic polynucleotide
aagcagaggagcaaaagctcatttctgaagaggacttgttgcggaaacgacgagaacagttgaaacacaaacttgaacagctacggaactcttgtgcgtaaggaaaagtaaggaaaacga

SEQ ID NO: 682 - DNA, 120 bp, Artificial Sequence
  Synthetic polynucleotide
cttcaggatggttcgtactaagacatggaccctgaagaagcactttgttggctatcctactaatagtgactttgagttgaagacagctgagctcccacccttaaaaaatggaggtaagtc

SEQ ID NO: 683 - DNA, 120 bp, Artificial Sequence
  Synthetic polynucleotide
gagtttctaattgcctatggaatgctttattttgtagaggtcctgcttgaagctttgttcctcaccgtggatccctacatgaggtattatttatttcgcccctcaaaatgctaatgctgt

SEQ ID NO: 684 - DNA, 120 bp, Artificial Sequence
  Synthetic polynucleotide
tttttttttttttttttttttgcagagtggcagccaaaagattgaaggaaggtgatacaatgatggggcagcaagtggccaagtaattatttccatttgtcccagtgcttggaaaatatg

SEQ ID NO: 685 - DNA, 119 bp, Artificial Sequence
  Synthetic polynucleotide
tctcttaaaaaaaccaaacatctcattctttatttttttaaattttgtgtctcaatgactagccagttattataataccattggtagaaatcgtctatggatctttactggaatttcag

SEQ ID NO: 686 - DNA, 120 bp, Artificial Sequence
  Synthetic polynucleotide
acatgccttaatgccttaatgtgctttatctttcagagttgtggaaagtaaaaatgtagccctaccaaaaggaactattgtactggcttctccaggctggacaacgcactccatttctga

SEQ ID NO: 687 - DNA, 120 bp, Artificial Sequence
  Synthetic polynucleotide
tgggaaagatctggaaaagctgctgacagagtggccagacacaataccactgtctttggctctggggacagttggcatgccagggtgagtttcatggatatattccatttgtttgaatgt

SEQ ID NO: 688 - DNA, 120 bp, Artificial Sequence
  Synthetic polynucleotide
gcctgactgcctactttggcctacttgaaatctgtggtgtgaagggtggagaaacagtgatggttaatgcagcagctggagctgtgggctcagtcgtggggcagattgcaaagctcaagg

SEQ ID NO: 689 - DNA, 120 bp, Artificial Sequence
  Synthetic polynucleotide
tgacttattcatggtttcctttttttttttttttctacttagggctgcaaagttgttggagcagtagggtctgatgaaaaggttgcctaccttcaaaagcttggatttgatgtcgtcttt

SEQ ID NO: 690 - DNA, 120 bp, Artificial Sequence
  Synthetic polynucleotide
aactacaagacggtagagtctttggaagaaaccttgaagaaagcgtctcctgatggttatgattgttattttgataatgtaagtacaaactggacttaatatctaatttattatggaagt

SEQ ID NO: 691 - DNA, 120 bp, Artificial Sequence
  Synthetic polynucleotide
gtttaggtaggtggagagttttcaaacactgttatcggccagatgaagaaatttggaaggattgccatatgtggagccatctctacatataacagaaccggcccacttcccccaggtaat

SEQ ID NO: 692 - DNA, 120 bp, Artificial Sequence
  Synthetic polynucleotide
gcccacccccagagattgttatctatcaggagcttcgcatggaagcttttgtcgtctaccgctggcaaggagatgcccgccaaaaagctctgaaggacttgctgaaatgggtcttagagg

SEQ ID NO: 693 - DNA, 120 bp, Artificial Sequence
  Synthetic polynucleotide
ttgagaatattaaattaagttttaaaatttgttgttgctttgatacagggtaaaatccagtacaaggaatatatcattgaaggatttgaaaacatgccagctgcatttatgggaatgctg

SEQ ID NO: 694 - DNA, 120 bp, Artificial Sequence
  Synthetic polynucleotide
aaaggagataatttggggaagacaatagtgaaagcatgaaaaagaggacacatggaatctggaggccatttagatgattagttaatttgtttttcaccatttagcaaaaatgtatactac

SEQ ID NO: 695 - DNA, 120 bp, Artificial Sequence
  Synthetic polynucleotide
cttaaatgtcttaagaaatagtactcataatgagtttgagctacttaataaaatacatttaagtggtatgtaattagtgatggaggatggaagtttcaaagtcaacaacaaccagtcacc

SEQ ID NO: 696 - DNA, 120 bp, Artificial Sequence
  Synthetic polynucleotide
gatcaaaagagaaaatgaagaagattgaagcttcaaagcagaaaaatgaagggaatatgtatcattcaccattaccttagaaggcaagggtccactttacaaaaggactacaaacattta

SEQ ID NO: 697 - DNA, 120 bp, Artificial Sequence
  Synthetic polynucleotide
gggtggctgacccccagcatcctcgggagcgaccatggactccctggccgagtctcggtggcctccgggcctggcagtcatgaaggtgagtgcttcggggagtttgggagctcccgggtg

SEQ ID NO: 698 - DNA, 120 bp, Artificial Sequence
  Synthetic polynucleotide
atgcatatttgcatttcagacaatagatgatttgctgcggtgtggaatttgcttcgagtatttcaacattgcaatgataatacctcagtgttcacataactgtaagtatgttttgttcct

SEQ ID NO: 699 - DNA, 120 bp, Artificial Sequence
  Synthetic polynucleotide
aacattatgttgcactttgtgttttgcagactgctctctctgtataagaaaatttctgtcctataaaactcagtgtccaacttgctgtgtggtgagtttttgtttcctttttttaaaact

SEQ ID NO: 700 - DNA, 120 bp, Artificial Sequence
  Synthetic polynucleotide
ccatctgttgtttgttttttctagactgtcacagagccggatctgaaaaataaccgcatattagatgaactggtaaaaagcttgaattttgcacggtatgatttaattttgtgactaacc

SEQ ID NO: 701 - DNA, 120 bp, Artificial Sequence
  Synthetic polynucleotide
tgtgcttcaaggaatcatctgctgcagtttgctttagagtcaccagccaaatctcctgcttcttcctcttcaaagaatcttgctgtcaaagtatatactcctgtagcctccagacagtct

SEQ ID NO: 702 - DNA, 120 bp, Artificial Sequence
  Synthetic polynucleotide
ttaaagcaggggagcaggttaatggataatttcttgatcagagaaatgagtggttctacatcagagttgttgataaaagaaaataaaagcaaattcagccctcaaaaagaggcgagccct

SEQ ID NO: 703 - DNA, 120 bp, Artificial Sequence
  Synthetic polynucleotide
gctgcaaagaccaaagagacacgttctgtagaagagatcgctccagatccctcagaggctaagcgtcctgagccaccctcgacatccactttgaaacaagttactaaaggtaggaagtta

SEQ ID NO: 704 - DNA, 120 bp, Artificial Sequence
  Synthetic polynucleotide
aaaaatacagtggattgtcctgtttgcggggttaacattccagaaagtcacattaataagcatttagacagctgtttatcacgcgaagagaagaaggaaagcctcagaaggtaaggaagt

SEQ ID NO: 705 - DNA, 120 bp, Artificial Sequence
  Synthetic polynucleotide
atcatcaggtatcttccccccttttcagttctgttcacaaaaggaagccgctgcccaaaactgtatataatttgctctctgatcgtgatttaaagaaaaagctaaaagagcatggattat

SEQ ID NO: 706 - DNA, 120 bp, Artificial Sequence
  Synthetic polynucleotide
ctattcaaggaaataaacaacagctcattaaaaggcaccaagaatttgtacacatgtacaatgcccaatgcgatgctttgcatcctaaatcaggtaaagtaataaaacagtgagttatgc

SEQ ID NO: 707 - DNA, 120 bp, Artificial Sequence
  Synthetic polynucleotide
gttattttcttattttaacagctgctgaaatagttcgagaaatcgaaaatatagagaagactaggatgcgtcttgaagctagtaaactcaatgaaagtgtatgttaatgggctatttcag

SEQ ID NO: 708 - DNA, 120 bp, Artificial Sequence
  Synthetic polynucleotide
tttattaaggtctttttttgattattttaggtaatggtttttacaaaggaccaaacagaaaaggaaatagatgaaatccacagtaaatatcgtaagttgcacgactttatttaatttgta

SEQ ID NO: 709 - DNA, 120 bp, Artificial Sequence
  Synthetic polynucleotide
ggttaactttcatagtcctagctttactgagaagatcttttgaatttcaggtaaaaaacataagagtgaatttcagcttctggtggatcaggctagaaaaggatacaagaaaattgctgg

SEQ ID NO: 710 - DNA, 120 bp, Artificial Sequence
  Synthetic polynucleotide
aatgtcacaaaaaacagtaacaataacaaaagaagatgaatctacagaaaagctatcttctgtatgcatgggtaagagactataattaaaaacagacatatgtcgaatttcattatttac

SEQ ID NO: 711 - DNA, 120 bp, Artificial Sequence
  Synthetic polynucleotide
aagttgtagattttaaggtactcttaaatttattttttcctaggacaggaagataatatgacctcagtaacaaaccacttttctcaatcaaagctggactccccagaggaattggaacct

SEQ ID NO: 712 - DNA, 120 bp, Artificial Sequence
  Synthetic polynucleotide
gacagagaagaggattcttctagctgtattgatattcaagaagttctttcttcatcagaatcagattcatgcaataggtaagaaacatgcagtagttgattattttaaatatctacttca

SEQ ID NO: 713 - DNA, 120 bp, Artificial Sequence
  Synthetic polynucleotide
tgtcaatactgatgtacatatccttttagttccagttcagacatcataagagatcttttagaagaagaggaagcctgggaagcatcacataagtgagttctcataatcatgaaataagca

SEQ ID NO: 714 - DNA, 120 bp, Artificial Sequence
  Synthetic polynucleotide
gtcttcagaaacgatcttcaagacacagaaataagtccaagacagaatcgccgcacaagagccgctgaaagtgctgagattgaaccaagaaacaagcgtaataggaattaatgtgggctt

SEQ ID NO: 715 - DNA, 120 bp, Artificial Sequence
  Synthetic polynucleotide
ttttatacagaaatcttgtgaaaccactgcccaaccagagcaatgattgttcaaagagtggtattgaattctcgacctggtatgtatttgcgatgaatgaacaactctgatctttgataa

SEQ ID NO: 716 - DNA, 120 bp, Artificial Sequence
  Synthetic polynucleotide
gaaaaaatggtaatccagtggcagagaatttccgaatggaagaagtctatttaccagataatattaatgaaggacaagtacaagttagaactctttatctttctgtggatccttacatgg

SEQ ID NO: 717 - DNA, 120 bp, Artificial Sequence
  Synthetic polynucleotide
tatcttaatgttttcttttttcagcgttgtagaatgaatgaagacactggcactgattatataacaccttggcagctatctcaagtcgttgatggaggaggtattggaattatagaagaa

SEQ ID NO: 718 - DNA, 120 bp, Artificial Sequence
  Synthetic polynucleotide
agcaaacacacaaatttgactaaaggcgattttgtgacttctttctattggccctggcaaaccaaggttattctggatggaaatagccttgaaaaggtgatatatatatgaacatatctg

SEQ ID NO: 719 - DNA, 120 bp, Artificial Sequence
  Synthetic polynucleotide
cctagtatttttaaagggtatatattttattttaggtagacccacaacttgtggatggacacctttcatattttcttggagctataggtatgcctggtttgacttccttgattgggatac

SEQ ID NO: 720 - DNA, 120 bp, Artificial Sequence
  Synthetic polynucleotide
aggaaaaaggtcatataactgctggatctaataagacaatggttgtcagtggggccgcaggtgcctgtggatctgtggctgggcaggtaaactttctgagaattatttgattttctgatt

SEQ ID NO: 721 - DNA, 120 bp, Artificial Sequence
  Synthetic polynucleotide
aaatttcccccctagattggccatttcttaggttgttccagagtggtgggaatttgtggaacacatgagaaatgcatcctcttgacctcagaactgggctttgatgctgcaattaattat

SEQ ID NO: 722 - DNA, 120 bp, Artificial Sequence
  Synthetic polynucleotide
aaaaaagacaatgtggcagaacagctccgtgaatcatgcccagctggagtggatgtttattttgacaatgttggtggtaacatcagtgatacagtgataagtcaggttgtttgctgattt

SEQ ID NO: 723 - DNA, 120 bp, Artificial Sequence
  Synthetic polynucleotide
agccataaaatcagtaaacataggaaagggatattttatcattatttttctctgtgcagatgaatgagaacagccacatcatcctgtgtggtcaaatttctcagtacaacaaagatgtgc

SEQ ID NO: 724 - DNA, 120 bp, Artificial Sequence
  Synthetic polynucleotide
cttatcctcccccgctatcccctgctatagaggcaatccagaaagaaagaaacatcacaaggtgtgttcttcctctttgcccttattaccaggttcatggggttttaaatatcatagatg

SEQ ID NO: 725 - DNA, 120 bp, Artificial Sequence
  Synthetic polynucleotide
ttcttcctcactgcagggaaagatttctggtattaaattataaagacaaatttgagcctggcattctacagctgagtcagtggtttaaagaaggaaagctaaaggtagaacttctattct

SEQ ID NO: 726 - DNA, 120 bp, Artificial Sequence
  Synthetic polynucleotide
aagtttaaagactattaaatctagctattttgatttacagattaaagagacggtaataaatgggttggaaaacatgggaggtaagatgaatgtagacttattatatacacatgctcagca

SEQ ID NO: 727 - DNA, 120 bp, Artificial Sequence
  Synthetic polynucleotide
aacctactttctctttttccagctgcattccagtccatgatgacaggaggtaacattggaaagcagatagtttgcatttcagaagaaatctctttgtaattgctgtaaatgtcatcaagg

SEQ ID NO: 728 - DNA, 120 bp, Artificial Sequence
  Synthetic polynucleotide
gagctgggagctaggtcctcggagtgggccagagatggcggcggccgacggggctttgccggaggcggcggctttagagcaacccgcggagctgcctgcctcggtgcgggcgagtatcga

SEQ ID NO: 729 - DNA, 120 bp, Artificial Sequence
  Synthetic polynucleotide
gcggaagcggcagcgggcactgatgctgcgccaggcccggctggctgcccggccctactcggcgacggcggctgcggctactggaggtttgggccgcgtccgcgctttccccttccctct

SEQ ID NO: 730 - DNA, 120 bp, Artificial Sequence
  Synthetic polynucleotide
gtaggcatggctaatgtaaaagcagccccaaagataattgacacaggaggaggcttcattttagaagaggaagaagaagaagaacagaaaattggaaaagttgttcatcaaccaggtaaa

SEQ ID NO: 731 - DNA, 120 bp, Artificial Sequence
  Synthetic polynucleotide
ttcttaggacctgttatggaatttgattatgtaatatgcgaagaatgtgggaaagaatttatggattcttatcttatgaaccactttgatttgccaacttgtgataactgcaggtactta

SEQ ID NO: 732 - DNA, 120 bp, Artificial Sequence
  Synthetic polynucleotide
ataactaatttatataatggacttaatctgttttcagagatgctgatgataaacacaagcttataaccaaaacagaggcaaaacaagaatatcttctgaaagactgtgatttagaaaaaa

SEQ ID NO: 733 - DNA, 120 bp, Artificial Sequence
  Synthetic polynucleotide
gagagccacctcttaaatttattgtgaagaagaatccacatcattcacaatggggtgatatgaaactctacttaaagttacaggtctctaataagttgtatttattatttttcactctgg

SEQ ID NO: 734 - DNA, 120 bp, Artificial Sequence
  Synthetic polynucleotide
gattgtgaagaggtctcttgaagtttggggtagtcaagaagcattagaagaagcaaaggaagtccgacaggaaaaccgagaaaaaatgaaacagaagaaatttgataaaaaagtaaaagg

SEQ ID NO: 735 - DNA, 120 bp, Artificial Sequence
  Synthetic polynucleotide
cctgaatagcaccactgaaaagatgactttaaaatttttttttcagaattgcggcgagcagtaagaagcagcgtgtggaaaagggagacgattgttcatcaacatgagtatggaccagaa

SEQ ID NO: 736 - DNA, 120 bp, Artificial Sequence
  Synthetic polynucleotide
gaaaacctagaagatgacatgtaccgtaagacttgtactatgtgtggccatgaactgacatatgaaaaaatgtgattttttagttcagtgacctgttttatagaattttatatttaaata

SEQ ID NO: 737 - DNA, 120 bp, Artificial Sequence
  Synthetic polynucleotide
caagcaacatggctcggaaacgcgcggccggcggggagccgcggggacgcgaactgcgcagccagaaatccaaggccaagagcaaggcccggcgtgaggaggaggaggagggtgagagcg

SEQ ID NO: 738 - DNA, 120 bp, Artificial Sequence
  Synthetic polynucleotide
tatgttctgtgttgtcacctagatgcctttgaagatgagaaacccccaaagaagagccttctctccaaagtttcacaaggaaagaggaaaagaggctgcagtcatcctgggggttcagca

SEQ ID NO: 739 - DNA, 120 bp, Artificial Sequence
  Synthetic polynucleotide
gatggtccagcaaaaaagaaagtggccaaggtgactgttaaatctgaaaacctcaaggttataaaggatgaagccctcagcgatggggatgacctcaggtgagatgtctgcaaagctttg

SEQ ID NO: 740 - DNA, 120 bp, Artificial Sequence
  Synthetic polynucleotide
acagggactttccaagtgacctcaagaaggcacaccatctgaagagaggggctaccatgaatgaagacagcaatgaagaagaggaagaaagtgaaaatgattgggaagaggttgaaggtg

SEQ ID NO: 741 - DNA, 120 bp, Artificial Sequence
  Synthetic polynucleotide
acagtagctattattattgttattactattactgatttttaaaaatgcttgttgatagaacttagtgagcctgtgctgggtgacgtgagagaaagtacagccttctctcgatctcttctg

SEQ ID NO: 742 - DNA, 120 bp, Artificial Sequence
  Synthetic polynucleotide
cctgtgaagccagtggagatagagattgaaacgccagagcaggcgaagacaagagaaagaaggtaagcttaggcccttgcttctaggctcctgtcacatgcagtaggcaacagctgctgc

SEQ ID NO: 743 - DNA, 120 bp, Artificial Sequence
  Synthetic polynucleotide
tttcactatttgttgcagtgaaaagataaaactggagtttgagacatatcttcggagggcgatgaaacgtttcaataaaggggtccatgaggacacacacaaggtaagggcaaggaatga

SEQ ID NO: 744 - DNA, 120 bp, Artificial Sequence
  Synthetic polynucleotide
ccttccttccatgctgccccttcctcctttcctcttcacaggttcaccttctctgcctgctagcaaatggcttctatcgaaataacatctgcagccagccagatctgcatgctattggcc

SEQ ID NO: 745 - DNA, 120 bp, Artificial Sequence
  Synthetic polynucleotide
tgtccatcatcccagcccgctttaccagagtgctgcctcgagatgtggacacctactacctctcaaacctggtgaagtggtaaggccctccgcttgtcctgcagagctggggagtgtagg

SEQ ID NO: 746 - DNA, 120 bp, Artificial Sequence
  Synthetic polynucleotide
gaaatgaaaattcccctttgccctgacctctgacacaaggaatgcctgctttctccccaggttcattggaacatttacagttaatgcagaactttcagccagtgaacaagataacctgca

SEQ ID NO: 747 - DNA, 120 bp, Artificial Sequence
  Synthetic polynucleotide
gactacattggaaaggagatttgctatttactctgctcgagatgatgaggaattggtccatgtaagtgatcctcccggatcactgttttttatcagtactgttaactaatgataatggca

SEQ ID NO: 748 - DNA, 120 bp, Artificial Sequence
  Synthetic polynucleotide
tccttttcatcatagatattcttactgattctccgggctctgcagctcttgacccggctggtattgtctctacagccaattcctctgaagtcagcaacagcaaaggtgaggtgcgcaggg

SEQ ID NO: 749 - DNA, 120 bp, Artificial Sequence
  Synthetic polynucleotide
gggggagaaaaaaaagcaaaatttcttattctgtttaagggaaagaaaccttccaaggaaagattgactgcggatccaggaggctcctcagaaacttccagccaagttctagaaaaccac

SEQ ID NO: 750 - DNA, 120 bp, Artificial Sequence
  Synthetic polynucleotide
accaaaccaaagaccagcaaaggaaccaaacaagaggaaacctttgctaagggcacctgcaggccaagtgccaaagggaagaggaacaagggaggcagaaagaaacggagcaagccctcc

SEQ ID NO: 751 - DNA, 120 bp, Artificial Sequence
  Synthetic polynucleotide
tccagcgaggaagatgagggcccaggagacaagcaggagaaggcaacccagcgacgtccgcatggccgggagcggcgggtggcctccagggtgtcttataaagaggagagtgggagtgat

SEQ ID NO: 752 - DNA, 120 bp, Artificial Sequence
  Synthetic polynucleotide
gaggctggcagcggctctgattttgagctctccagtggagaagcctctgatccctctgatgaggattccgaacctggccctccaaagcagaggaaagcccccgctcctcagaggacaaag

SEQ ID NO: 753 - DNA, 120 bp, Artificial Sequence
  Synthetic polynucleotide
gctgggtccaagagtgcctccaggacccatcgtgggagccatcgtaaggacccaagcttgccagcggcatcctcaagctcttcaagcagtaaaagaggcaagaaaatgtgcagcgatggt

SEQ ID NO: 754 - DNA, 120 bp, Artificial Sequence
  Synthetic polynucleotide
gagaaggcagaaaaaagaagcatagctggtatagaccagtggctagaggtgttctgtgagcaggaggaaaagtgggtatgtgtagactgtgtgcacggtgtggtgggccagcctctgacc

SEQ ID NO: 755 - DNA, 120 bp, Artificial Sequence
  Synthetic polynucleotide
tgttacaagtacgccaccaagcccatgacctatgtggtgggcattgacagtgacggctgggtccgagatgtcacacagaggtacgacccagtctggatgacagtgacccgcaagtgccgg

SEQ ID NO: 756 - DNA, 120 bp, Artificial Sequence
  Synthetic polynucleotide
gttgatgctgagtggtgggccgagaccttgagaccataccagagcccatttatggacagggagaagaaagaagacttggaggtaaggccttggctgccaggggctccaagacacagtcag

SEQ ID NO: 757 - DNA, 120 bp, Artificial Sequence
  Synthetic polynucleotide
ctaaataacatgctcaaccttgtctgtctggcctttgcagtttcaggctaaacacatggaccagcctttgcccactgccattggcttatataagaaccaccctctgtatgccctgaagcg

SEQ ID NO: 758 - DNA, 120 bp, Artificial Sequence
  Synthetic polynucleotide
gcatctcctgaaatatgaggccatctatcccgagacagctgccatccttgggtattgtcgtggagaagcggtctactccaggtgcgtgaggcagcctggttggcctcaggggcttcctga

SEQ ID NO: 759 - DNA, 120 bp, Artificial Sequence
  Synthetic polynucleotide
tcctgtgttggttccacagggattgtgtgcacactctgcattccagggacacgtggctgaagaaagcaagagtggtgaggcttggagaagtaccctacaaggtaactggagctggggggt

SEQ ID NO: 760 - DNA, 120 bp, Artificial Sequence
  Synthetic polynucleotide
ctgaggaactggatgcctttgttgtaaacggtggccgtgtcctctggtgcagatggtgaaaggcttttctaaccgtgctcggaaagcccgacttgctgagccccagctgcgggaagaaaa

SEQ ID NO: 761 - DNA, 120 bp, Artificial Sequence
  Synthetic polynucleotide
tgacctgggcctgtttggctactggcagacagaggagtatcagcccccagtggccgtggacgggaaggtaagggcagcatcagaagggctcaggaccaggccgccttgttcccctgctgg

SEQ ID NO: 762 - DNA, 120 bp, Artificial Sequence
  Synthetic polynucleotide
tgctggccaaatgctgacttgctcacccgacacaggtgccccggaacgagtttgggaatgtgtacctcttcctgcccagcatgatgcctattggctgtgtccagctgaacctgcccaatc

SEQ ID NO: 763 - DNA, 120 bp, Artificial Sequence
  Synthetic polynucleotide
tacaccgcgtggcccgcaagctggacatcgactgtgtccaggccatcactggctttgatttccatggcggctactcccatcccgtgtgcgtgaggggccttcgatggaggctaaacacag

SEQ ID NO: 764 - DNA, 120 bp, Artificial Sequence
  Synthetic polynucleotide
tgtgtccccacaggactgatggatacatcgtctgcgaggaattcaaagacgtgctcctgactgcctgggaaaatgagcaggcagtcattgaaaggaaggagaaggaggtaagcgcatatg

SEQ ID NO: 765 - DNA, 120 bp, Artificial Sequence
  Synthetic polynucleotide
catttttgcctgcagaaaaaggagaagcgggctctagggaactggaagttgctggccaaaggtctgctcatcagggagaggctgaagcgtcgctacgggcccaaggtcagtgcaggttct

SEQ ID NO: 766 - DNA, 120 bp, Artificial Sequence
  Synthetic polynucleotide
acctgtccagagtgaggcagcagctccccacacagatgcaggaggtggactctcttctgatgaagaggaggggaccagctctcaagcagaagcggccaggatactggctgcctcctggcc

SEQ ID NO: 767 - DNA, 120 bp, Artificial Sequence
  Synthetic polynucleotide
tcaaaaccgagaagatgaagaaaagcagaagctgaagggtgggcccaagaagaccaaaagggaaaagaaagcagcagcttcccacctgttcccatttgagcagctgtgagctgagcgccc

SEQ ID NO: 768 - DNA, 120 bp, Artificial Sequence
  Synthetic polynucleotide
cagaaagcgggcgagcagcagttgagcgagcccgaggacatggagatggaaggtgaggcccgagggccggccgcggcggggccggggggcgcctttcattgtggccgggggagccgcggg

SEQ ID NO: 769 - DNA, 120 bp, Artificial Sequence
  Synthetic polynucleotide
tgaatgtttctggtcctaaagacaaggcttctgtgggatgctttaaaaaataaaaaagaatgctgaggtagagctcctagagattctatgcagtcactctgatgtgggtgagagaacctc

SEQ ID NO: 770 - DNA, 120 bp, Artificial Sequence
  Synthetic polynucleotide
ccccatcccccagcagaggccactgcagagccatgcagagatggctgggaaccacaggcttgggctggaaggtgagtcaggttttcaggttgagctccttatgctggtgatggatggaga

SEQ ID NO: 771 - DNA, 120 bp, Artificial Sequence
  Synthetic polynucleotide
ctttaaagcgggagatacagatgacccaccaagaattactcagaaccctgtgatcaatgggaatgtggccctgagtgatggacacaacaccgcggaggaggacatggaggatggtaagtg

SEQ ID NO: 772 - DNA, 120 bp, Artificial Sequence
  Synthetic polynucleotide
atgatgtgttttttttgcagacaccagttggcgctccgaggcaacctttcagttcactgtggagcgcttcagcagactgagtgagtcggtccttagccctccgtgttttgtgcgaaatct

SEQ ID NO: 773 - DNA, 120 bp, Artificial Sequence
  Synthetic polynucleotide
gccatggaagattatggtgatgccacgcttttatccagacagaccacaccaaaaaagcgtaggattctttctccagtgcaatgctgaatctgattccacgtaagacagtatttcattact

SEQ ID NO: 774 - DNA, 120 bp, Artificial Sequence
  Synthetic polynucleotide
aacatctggtaaataatgtcaactaaggctcagattattcttttaaacaggtcatggtcttgccatgcacaagcagtgctgaagataataaattacagagatgatgaaaagtcgttcagt

SEQ ID NO: 775 - DNA, 120 bp, Artificial Sequence
  Synthetic polynucleotide
cgtcgtattagtcatttgttcttccataaagaaaatgattggggattttccaattttatggcctggagtgtaagtaacagtgtatttagtctgaacaattggtgcattactgcttgttgt

SEQ ID NO: 776 - DNA, 120 bp, Artificial Sequence
  Synthetic polynucleotide
tatttatgttttataggaagtgaccgatcctgagaaaggatttatagatgatgacaaagttacctttgaagtctttgtacaggcggatgctccccatggagttgcgtaagtttttcttta

SEQ ID NO: 777 - DNA, 120 bp, Artificial Sequence
  Synthetic polynucleotide
tttcaggtgggattcaaagaagcacacaggctacgtcggcttaaagaatcagggagcgacttgttacatgaacagcctgctacagacgttatttttcacgaatcagctacgaaaggtaaa

SEQ ID NO: 778 - DNA, 120 bp, Artificial Sequence
  Synthetic polynucleotide
taaattcccctgcatcttctcagagtaaaaattcttatttcttaattgtttcaggctgtgtacatgatgccaaccgagggggatgattcgtctaaaagcgtccctttagcattacaaaga

SEQ ID NO: 779 - DNA, 120 bp, Artificial Sequence
  Synthetic polynucleotide
gtgttctatgaattacagcatagtgataaacctgtaggaacaaaaaagttaacaaagtcatttgggtatgtattagacatctgcctttgccattctgcttcctctttttttttttttttt

SEQ ID NO: 780 - DNA, 120 bp, Artificial Sequence
  Synthetic polynucleotide
ttaaatggagttgtttgttttatctttgaaaggtgggaaactttagatagcttcatgcaacatgatgttcaggagctttgtcgagtggtaagtttcaagcaatacttgtatatttcttac

SEQ ID NO: 781 - DNA, 120 bp, Artificial Sequence
  Synthetic polynucleotide
gccaaaacattctttttcagttgctcgataatgtggaaaataagatgaaaggcacctgtgtagagggcaccatacccaaattattccgcggcaaaatggtggtatgtggctaccagttct

SEQ ID NO: 782 - DNA, 120 bp, Artificial Sequence
  Synthetic polynucleotide
ttccttatttgcagtcctatatccagtgtaaagaagtagactatcggtctgatagaagagaagattattatgatatccagctaagtatcaaaggaaagaaaaatagtaagtgttgtgtgt

SEQ ID NO: 783 - DNA, 120 bp, Artificial Sequence
  Synthetic polynucleotide
ctctctctctctttaaagtatttgaatcatttgtggattatgtggcagtagaacagctcgatggggacaataaatacgacgctggggaacatggcttacaggtaaattgagtgttttgtg

SEQ ID NO: 784 - DNA, 120 bp, Artificial Sequence
  Synthetic polynucleotide
tttaggaagcagagaaaggtgtgaaattcctaacattgccaccagtgttacatctacaactgatgagatttatgtatgaccctcagacggaccaaaatatcaagatcaatgataggtaat

SEQ ID NO: 785 - DNA, 120 bp, Artificial Sequence
  Synthetic polynucleotide
tgtaaattaatactgaatttcttttaaaatgttttctaataggtttgaattcccagagcagttaccacttgatgaatttttgcaaaaaacagatcctaaggaccctgcaaattatattct

SEQ ID NO: 786 - DNA, 120 bp, Artificial Sequence
  Synthetic polynucleotide
tcatgcagtcctggttcatagtggagataatcatggtggacattatgtggtttatctaaaccccaaaggggatggcaaagtaagtggtgggacccagggctgaatgcaagctcatcagaa

SEQ ID NO: 787 - DNA, 120 bp, Artificial Sequence
  Synthetic polynucleotide
cttgtcacagtgcttgatcgctgctggtgtgtgttgttttccttgcagtggtgtaaatttgatgacgacgtggtgtcaaggtgtactaaagaggaagcaattgagcacaattatgggggt

SEQ ID NO: 788 - DNA, 120 bp, Artificial Sequence
  Synthetic polynucleotide
cacgatgacgacctgtctgttcgacactgcactaatgcttacatgttagtctacatcagggaatcaaaactgagtgagtagtgttcacttttgttctgttctttactgtggtggacttgg

SEQ ID NO: 789 - DNA, 120 bp, Artificial Sequence
  Synthetic polynucleotide
ctaagaggggaaagtccatctgcaggggtcaaagaggatgcctttgtcctgcaggtgaagttttacaggcggtcaccgaccatgatattcctcagcagttggtggagcgattacaagaag

SEQ ID NO: 790 - DNA, 120 bp, Artificial Sequence
  Synthetic polynucleotide
agaaaaggatcgaggctcagaagcggaaggagcggcaggaagcccatctctatatgcaagtgcaggtcagcccccgcccttctgggactccgggtcaccatgcagccgggcacccatctc

SEQ ID NO: 791 - DNA, 120 bp, Artificial Sequence
  Synthetic polynucleotide
tcattttttgtcagttgtcaagtcttttctgtgctttcatacatattttcagatagtcgcagaggaccagttttgtggccaccaagggaatgacatgtacgatgaagaaaaagtgaaata

SEQ ID NO: 792 - DNA, 120 bp, Artificial Sequence
  Synthetic polynucleotide
cactgtgttcaaagtattgaagaactcctcgcttgctgagtttgttcagagcctctctcagaccatggtgcgtaccggtcccgtggatataccccaccgtggctcccaacgtccaccttc

SEQ ID NO: 793 - DNA, 120 bp, Artificial Sequence
  Synthetic polynucleotide
ttttttcagggatttccacaagatcaaattcgattgtggcccatgcaagcaaggagtaatggaacaaaacgaccagcaatgttagataatgaagccgacggcaataaaacagtaaatatt

SEQ ID NO: 794 - DNA, 120 bp, Artificial Sequence
  Synthetic polynucleotide
gaaatagatgattgagctcagtgataatgaaaacccttggacaatattcctggaaacagttgatcccgagctggctgctagtggagcgaccttacccaagtttgataaagatcgtaagtg

SEQ ID NO: 795 - DNA, 120 bp, Artificial Sequence
  Synthetic polynucleotide
tattaaccttgtagatgatgtaatgttatttttgaagatgtatgatcccaaaacgcggagcttgaattactgtgggcatatctacacaccaatatcctgtaaaatacgtaagtccttcgt

SEQ ID NO: 796 - DNA, 120 bp, Artificial Sequence
  Synthetic polynucleotide
catttaaaatatcttctttctcctaggtgacttgctcccagttatgtgtgacagagcaggatttattcaagatactagccttatcctctatgaggtttggatggtttatttttccataat

SEQ ID NO: 797 - DNA, 120 bp, Artificial Sequence
  Synthetic polynucleotide
ttcactgtaggaagttaaaccgaatttaacagagagaattcaggactatgacgtgtctcttgataaagcccttgatgaactaatggatggtgacatcatagtatttcagaagtatgtact

SEQ ID NO: 798 - DNA, 120 bp, Artificial Sequence
  Synthetic polynucleotide
ccatggactttgattcagactgcaaactttctccctccaccagggatgaccctgaaaatgataacagtgaattacccaccgcaaaggagtatttccgagatctctaccaccgcgttgatg

SEQ ID NO: 799 - DNA, 120 bp, Artificial Sequence
  Synthetic polynucleotide
tcattttctgtgataaaacaatccctaatgatcctggatttgtggttacgttatcaaatagaatgaattattttcaggtatttaataaatgctcctttcctcttcagatcccactccaga

SEQ ID NO: 800 - DNA, 120 bp, Artificial Sequence
  Synthetic polynucleotide
tgtgaaccttcctttctgtgtcttaggttgcaaagacagttgcacagaggctcaacacagatccaatgttgctgcagtttttcaagtctcaagggtaggtcacatgtgtggacacttgct

SEQ ID NO: 801 - DNA, 120 bp, Artificial Sequence
  Synthetic polynucleotide
gtgtagttatagggatggcccaggtaatcctcttagacataattatgaaggtactttaagagatcttctacagttcttcaagcctagacaacctaagaaactttactatcagcaggtatg

SEQ ID NO: 802 - DNA, 120 bp, Artificial Sequence
  Synthetic polynucleotide
gaatctttcttttcttaatagcttaagatgaaaatcacagactttgagaacaggcgaagttttaaatgtatatggttaaacagccaatttagggaagaggtaagtttttttaatactatg

SEQ ID NO: 803 - DNA, 120 bp, Artificial Sequence
  Synthetic polynucleotide
cattacttaggaaataacactatatccagacaagcatgggtgtgtccgggacctgttagaagaatgtaaaaaggccgtggagcttggggagaaagcatcagggaaacttaggcaagtatt

SEQ ID NO: 804 - DNA, 120 bp, Artificial Sequence
  Synthetic polynucleotide
ctctgttcaggctgctagaaattgtaagctacaaaatcattggtgttcatcaagaagatgaactattagaatgtttatctcctgcaacgagccggacgtttcgaatagaggtatctgtcc

SEQ ID NO: 805 - DNA, 120 bp, Artificial Sequence
  Synthetic polynucleotide
tggacactttgaccacatcacttgcacttacagaactgtgtctgttgtccgtgtccccaggaaatccctttggaccaggtggacatagacaaagagaatgagatgcttgtcacagtggcg

SEQ ID NO: 806 - DNA, 120 bp, Artificial Sequence
  Synthetic polynucleotide
catttccacaaagaggtcttcggaacgttcggaatcccgtttttgctgaggatacaccaggtatgctgttgtggttggccgagtggctcacgtcaaaacctggagcctttgagtggccgc

SEQ ID NO: 807 - DNA, 120 bp, Artificial Sequence
  Synthetic polynucleotide
agcacatgtcctttgccattctagggcgagcattttcgagaagtgatgaagcgaatccagagcctgctggacatccaggagaaggagtttgagaaggtgtgcagctggggcctcctgggg

SEQ ID NO: 808 - DNA, 120 bp, Artificial Sequence
  Synthetic polynucleotide
gtttaaatttgcaattgtaatgatgggccgacaccagtacataaatgaagacgagtatgaagtaaatttgaaagactttgagccacagcccggtaagggttctcccccccccgggggctg

SEQ ID NO: 809 - DNA, 120 bp, Artificial Sequence
  Synthetic polynucleotide
caccaggtaatatgtctcatcctcggccttggctagggctcgaccacttcaacaaagccccaaagaggagtcgctacacttaccttgaaaaggccattaaaatccataactgatttccaa

SEQ ID NO: 810 - DNA, 120 bp, Artificial Sequence
  Synthetic polynucleotide
tatttctagatatggatcagaaactttcgaagttggtagaagagctcacaacttcaggagaaccccgactaaatcctgagaaaatgaaggaactgaagaaaatttgcaagtatgtcttag

SEQ ID NO: 811 - DNA, 120 bp, Artificial Sequence
  Synthetic polynucleotide
gctcgcatccccaggtcttcagaggagcagctgagccgcgcctaccgcctgctgatagcacagctgacccaggagcacgccgagatccgtctctcagccttccagattgtggaggaactc

SEQ ID NO: 812 - DNA, 120 bp, Artificial Sequence
  Synthetic polynucleotide
ttcgtcaggtctcaccagttccggatgctggttgtttccaacttccaggagttcctggagctcacgctgggcacagaccccgcacagcctctgccgccccccagggaggcggcacagagg

SEQ ID NO: 813 - DNA, 120 bp, Artificial Sequence
  Synthetic polynucleotide
ctgaggcaggcgaccacccgggccgtggaagggtggaatgagaagtttggggaggcctacaagaagcttgccttgggctaccacttcttaagacacaacaaaaaggtaggtgggcctggc

SEQ ID NO: 814 - DNA, 120 bp, Artificial Sequence
  Synthetic polynucleotide
gtgagccaccgcgcctgtcccctagtctttattttcaattgctcaggtggattttcaagacacgaatgctcggagtctggcagaaaggaagagagaagaggagaagcagaagcacttgga

SEQ ID NO: 815 - DNA, 120 bp, Artificial Sequence
  Synthetic polynucleotide
taaaatttatcaagaaagagccagccaggcggagagggagatgcaaggcaagtgtccaggacggagggaggggcccacgcctctgagggttgcccgtggtccagcagttcatcctcctgg

SEQ ID NO: 816 - DNA, 120 bp, Artificial Sequence
  Synthetic polynucleotide
cttttgctccacatagcgcagcaaacaggtgtcttgatcttccggcagaaatgtctggagaaattgaatcctgcttgacggaggtagagagctgctttaggctgctggtgccttttgact

SEQ ID NO: 817 - DNA, 120 bp, Artificial Sequence
  Synthetic polynucleotide
ttgacccgaacccggagacggaatcccttggcatggcttctggcatgtccgatgcccttcgctcctcctgcgcgggccaggtgggcccctgccggtctggcacccctgacccccgggacg

SEQ ID NO: 818 - DNA, 120 bp, Artificial Sequence
  Synthetic polynucleotide
gggagcagccctgctgcagtagagacctgcctgcctctgcaggccaccccagagcgggcggcggggcacagccatcccagacagccacaggtgacccctcagatgaggacgaggacagcg

SEQ ID NO: 819 - DNA, 120 bp, Artificial Sequence
  Synthetic polynucleotide
acctcgaggagtttgtgcggagccacgggctgggctcgcacaagtacacgctggatgtggagctctgctcaggtaactgccttcgcggggtctctgtggcgccaccctgccccggctccc

SEQ ID NO: 820 - DNA, 120 bp, Artificial Sequence
  Synthetic polynucleotide
ccagagggcctgaaggtgcaggagaacgaggacaaccttgctctcatccacgccgcccgcgacacactcaagctcatccggaacaagttcctgccggctgtgtgctcgtggatccaggtg

SEQ ID NO: 821 - DNA, 120 bp, Artificial Sequence
  Synthetic polynucleotide
gtgtgccagggaccccccgggccagtggacctggcatgtgcctcccagcaggacagcttcccaggtcctgcccggccggcccctgagctgttcgcacccccgtttcgcagcgcttcaccc

SEQ ID NO: 822 - DNA, 120 bp, Artificial Sequence
  Synthetic polynucleotide
gcgtcgggacccacggtggatgtttaaagcgtgccattgacctgaaggctgaattggagctcgtactgagaaaatacaaggagctggacatcgagcctgagggaggggaaaggcgcaggg

SEQ ID NO: 823 - DNA, 120 bp, Artificial Sequence
  Synthetic polynucleotide
acagacagaagccctgggggatgcggaggaagatgaggacgatgaggactttgtggaggtccctgagaaggaggggtatgagccacacatccccgaccacttgcggcctgagtatggtga

SEQ ID NO: 824 - DNA, 120 bp, Artificial Sequence
  Synthetic polynucleotide
ggcgggttgtgggagtggtggcagggagtggacacgtgtctgtttcagggctggaggcagcaccagagaaagacacagttgtgcggtgcttgcggacgaggacgaggatggacgaggagg

SEQ ID NO: 825 - DNA, 120 bp, Artificial Sequence
  Synthetic polynucleotide
tgtcggaccccacctctgcggctgctcagctgcggcagctccgggaccacttgcctccaccctcatctgccaggtgactcccagtgtcctgtgtgctgagccccctgcccggcgctgcca

SEQ ID NO: 826 - DNA, 120 bp, Artificial Sequence
  Synthetic polynucleotide
gctgtgggtggcaccagcagcaccgtcaggctgtcccactctgctcctgtagcccctccagagcgttgccagagccacaggaggcccagaagctggcagcagagcgggcccgggcgcctg

SEQ ID NO: 827 - DNA, 120 bp, Artificial Sequence
  Synthetic polynucleotide
tggtgccctacggcgtggacctgcactactggggccaggagctccccacagccgggaagattgtcaagtgagtccccatgtgtctgaagtcggccagggcacacaaccagggtcccagcc

SEQ ID NO: 828 - DNA, 120 bp, Artificial Sequence
  Synthetic polynucleotide
ctatgagggcctctggctgtgtctgcaggtctgactcccagcaccgcttctggaagcccagcgaggtggaggaggaagtggtcaatgccgacatctccgagatgctccggagccgccaca

SEQ ID NO: 829 - DNA, 120 bp, Artificial Sequence
  Synthetic polynucleotide
tcacttttgccgggaagtttgagcctgtgcagcactggtgccgtgccccgaggccagacggccggctctgtgagcgccaagaccggctgaaggtgaggccgtggcccgagggcgggggtg

SEQ ID NO: 830 - DNA, 120 bp, Artificial Sequence
  Synthetic polynucleotide
gactttccacagctgcccaagaccttccggctccagaggagggacggagccatccccacgtccctgtggctctcaggacgccctcctctgaggggcgcgtgattccaggttgtgtacact

SEQ ID NO: 831 - DNA, 120 bp, Artificial Sequence
  Synthetic polynucleotide
ttggctctgtgataccacccaccctggtcgctgtttgtgcccaagtcgtggtggtggggggaggtggtcaaggcaagcggacccctccccgccatcagccaccgtgtcctcgctgtgcag

SEQ ID NO: 832 - DNA, 120 bp, Artificial Sequence
  Synthetic polynucleotide
tgccctttccatgggaagattgttccacgggacgacgaaggacggccgctcgacccggaagacagggctcgtgagcagcggcggcagctgcagaagcaggagcgcccgggtaggtctggg

SEQ ID NO: 833 - DNA, 120 bp, Artificial Sequence
  Synthetic polynucleotide
cgtctcctgaagtgcttgagttttgtttgcagaatggcaggaccctgagttgatgagagacgtggaagcagccacagggcaggatctcggctcatccaggtacagcgggaaaggcagggg

SEQ ID NO: 834 - DNA, 120 bp, Artificial Sequence
  Synthetic polynucleotide
gaagaagaggaggtaccccagcctcaccaacctgaaggctcaggctgataccgcccgcgctcgcattgggagaaaagtcttcgccaagtaagagtggctgctgggtcacctcccaccgcg

SEQ ID NO: 835 - DNA, 120 bp, Artificial Sequence
  Synthetic polynucleotide
tgtttccccacagggcagctgtgcggagggtagtggcagccatgaaccggatggaccagaagaagcacgagaagttttcaaaccagtttaactacgcactgaactagagagcggggccca

SEQ ID NO: 836 - DNA, 120 bp, Artificial Sequence
  Synthetic polynucleotide
tttttctttatcttttttttttttagactacaacaaaatcacaattaaatccggcctttgaagatgcctggagcagcagtgatgaagaaggatgaatatcatctttagtacctttttgtc

SEQ ID NO: 837 - DNA, 120 bp, Artificial Sequence
  Synthetic polynucleotide
ctttgccttctatgttataggaactttatagtggtagcagagactgcaacattctggcttgggttccatccttatatgaaccagttcctgatgatgatgaggtaaatattattttcacaa

SEQ ID NO: 838 - DNA, 120 bp, Artificial Sequence
  Synthetic polynucleotide
accattgctgtttatacagtttactcaggagaacagataactatgcttaagggacattataaaactgttgactgctgtgtatttcagtcaaatttccaggtaagagtgatacaggaattt

SEQ ID NO: 839 - DNA, 120 bp, Artificial Sequence
  Synthetic polynucleotide
cttattattttaatcctacaggtgaactatggaaaagtttgtaataacagtaaaaaaggattgaaattcactgtctcctgtggctgcagttcagaatttgtttttgtaccatatggtagc

SEQ ID NO: 840 - DNA, 120 bp, Artificial Sequence
  Synthetic polynucleotide
ctcactgttggtacagataatcgaatgaggctctggaatagttccaatggagaaaacacacttgtaagagatttttaagtatatatttgggtataaattaagaaatggatctgtgacata

SEQ ID NO: 841 - DNA, 120 bp, Artificial Sequence
  Synthetic polynucleotide
acattaaatatgtcctgaatacaagaacagataaactgaactatgtttttcattgcagcaaacactgctcataatgggaaagttaatggcttatgttttacaagtgatggacttcacctc

SEQ ID NO: 842 - DNA, 120 bp, Artificial Sequence
  Synthetic polynucleotide
ttcttctcagtgctgacagtagagtaaaattatgggatgtgagaagagcatcaggatgtttgattactcttgatcaacataatgggaaaaagtcacaagctgttgaatcaggtaaggaag

SEQ ID NO: 843 - DNA, 120 bp, Artificial Sequence
  Synthetic polynucleotide
gacttttcatatagttgtatttgcaggtcacagacaagaaatattagcagtttcctggtctccacgttatgactatatcttggcaacagcaaggtaaaatttaacttatttgcttttgaa

SEQ ID NO: 844 - DNA, 120 bp, Artificial Sequence
  Synthetic polynucleotide
aatgtcttttgattaccagactgcagatgtatttaattttgaggaaacagtttatagtcatcatatgtctccagtctccaccaagcactgtttggtagcaggtttgtaagtgtattcttt

SEQ ID NO: 845 - DNA, 120 bp, Artificial Sequence
  Synthetic polynucleotide
tttatttttaagagttttgggactggaattaaataaagacagagatgttgaaagaatccacggcggtggaattaacacccttgacattgaacctgttgaagggagatagtaagtttatta

SEQ ID NO: 846 - DNA, 120 bp, Artificial Sequence
  Synthetic polynucleotide
ccagccggtgtgaggacacgatatgctggggtttttgtccgcacgccaaacgggtttggaggaccctcttcgccttcggagagcagagtcaacacggaggtaaagaaaaccttacttttt

SEQ ID NO: 847 - DNA, 120 bp, Artificial Sequence
  Synthetic polynucleotide
gcatgttcacatcaagctcatttgataaaactctgaaagtatgggatacaaatacattacaagtaagtacattaaaacatttgcagattgctttgtaggataaaggagaatttaatccta

SEQ ID NO: 848 - DNA, 120 bp, Artificial Sequence
  Synthetic polynucleotide
taccagttttgaaactcacataagtcagttaatgtaaattttgattgctgttttgtagagatcatcctgatgttcacagatacagtgtggagactgtacagtggtatcctcatgacactg

SEQ ID NO: 849 - DNA, 120 bp, Artificial Sequence
  Synthetic polynucleotide
tattatcagcatgttatcaggtggttcagatggtgtgattgtactttatgaccttgagaactccagcagacaatcttattacacatgtaaagcagtgtgttccattggcaggtatgtatt

SEQ ID NO: 850 - DNA, 120 bp, Artificial Sequence
  Synthetic polynucleotide
ggtatttttattttatttcaaacggcaactactttgagtaaacgattcaataaaaagaaacgttactaacagtgtattctttgtaagtgacatgactaatgtactttgtgctggttgttg

SEQ ID NO: 851 - DNA, 120 bp, Artificial Sequence
  Synthetic polynucleotide
ttttgatgatgacttatgataaaattatcttaaaccggttctgtttttacagttggtactagaggacccaaagtacaactttgtgacttgaagtctggatcctgttctcacattctacag

SEQ ID NO: 852 - DNA, 21 bp, Artificial Sequence
  Synthetic polynucleotide
aatttgtgatacccctcgacg

SEQ ID NO: 853 - DNA, 24 bp, Artificial Sequence
  Synthetic polynucleotide
tgggaaggctctgtgtagatcgga

SEQ ID NO: 854 - DNA, 20 bp, Artificial Sequence
  Synthetic polynucleotide
tgtgagatggcatattcggc

SEQ ID NO: 855 - DNA, 20 bp, Artificial Sequence
  Synthetic polynucleotide
tccttgctaactttgccacc

SEQ ID NO: 856 - DNA, 21 bp, Artificial Sequence
  Synthetic polynucleotide
tgcttccacagtgctgagcct

SEQ ID NO: 857 - DNA, 22 bp, Artificial Sequence
  Synthetic polynucleotide
catctttgctactggttttccc

SEQ ID NO: 858 - DNA, 22 bp, Artificial Sequence
  Synthetic polynucleotide
gtccgcgaagatgacaaaattg

SEQ ID NO: 859 - DNA, 24 bp, Artificial Sequence
  Synthetic polynucleotide
agcacactggactttggcgatgta

SEQ ID NO: 860 - DNA, 21 bp, Artificial Sequence
  Synthetic polynucleotide
aattcaggagacatagggcac

SEQ ID NO: 861 - DNA, 22 bp, Artificial Sequence
  Synthetic polynucleotide
tctttatgacgcagagctaacc

SEQ ID NO: 862 - DNA, 25 bp, Artificial Sequence
  Synthetic polynucleotide
ttcggcagcttgaaatttacagggc

SEQ ID NO: 863 - DNA, 20 bp, Artificial Sequence
  Synthetic polynucleotide
tccgcaaagcagtgagatag

SEQ ID NO: 864 - DNA, 21 bp, Artificial Sequence
  Synthetic polynucleotide
gactccaggaaaacgacagag

SEQ ID NO: 865 - DNA, 28 bp, Artificial Sequence
  Synthetic polynucleotide
agcaaaagagatgaagcactacccagtc

SEQ ID NO: 866 - DNA, 21 bp, Artificial Sequence
  Synthetic polynucleotide
ggaggcaaaacatagaggtcg

SEQ ID NO: 867 - DNA, 21 bp, Artificial Sequence
  Synthetic polynucleotide
ggaaagtgggaagataccgag

SEQ ID NO: 868 - DNA, 27 bp, Artificial Sequence
  Synthetic polynucleotide
tgcaggacaaagagaaacgtctgaagc

SEQ ID NO: 869 - DNA, 22 bp, Artificial Sequence
  Synthetic polynucleotide
ccttcgtcaaattcagcatcac

SEQ ID NO: 870 - DNA, 20 bp, Artificial Sequence
  Synthetic polynucleotide
agtagaaatacggctgcacc

SEQ ID NO: 871 - DNA, 20 bp, Artificial Sequence
  Synthetic polynucleotide
tccggaaggccgaggccttg

SEQ ID NO: 872 - DNA, 22 bp, Artificial Sequence
  Synthetic polynucleotide
ccaggtctccattcttagttgc

SEQ ID NO: 873 - DNA, 22 bp, Artificial Sequence
  Synthetic polynucleotide
agccattgacagagcatatagg

SEQ ID NO: 874 - DNA, 26 bp, Artificial Sequence
  Synthetic polynucleotide
cctccacagttcccaaggatatcagc

SEQ ID NO: 875 - DNA, 21 bp, Artificial Sequence
  Synthetic polynucleotide
ggcattttcacttccaaccac

SEQ ID NO: 876 - DNA, 20 bp, Artificial Sequence
  Synthetic polynucleotide
gtgaggacacgatatgctgg

SEQ ID NO: 877 - DNA, 26 bp, Artificial Sequence
  Synthetic polynucleotide
aacacggagagttttgggactggaat

SEQ ID NO: 878 - DNA, 21 bp, Artificial Sequence
  Synthetic polynucleotide
gccgtggattctttcaacatc

SEQ ID NO: 879 - DNA, 22 bp, Artificial Sequence
  Synthetic polynucleotide
tccacatccaatcataagcagg

SEQ ID NO: 880 - DNA, 23 bp, Artificial Sequence
  Synthetic polynucleotide
cggacatcagccagaaatgcagc

SEQ ID NO: 881 - DNA, 22 bp, Artificial Sequence
  Synthetic polynucleotide
cttagaccgttacagccatcag

SEQ ID NO: 882 - DNA, 21 bp, Artificial Sequence
  Synthetic polynucleotide
caaaaccctctttcagcatgg

SEQ ID NO: 883 - DNA, 25 bp, Artificial Sequence
  Synthetic polynucleotide
tggctcagtgttgctatccagatgc

SEQ ID NO: 884 - DNA, 21 bp, Artificial Sequence
  Synthetic polynucleotide
agcagacaccaaagtaagacc

SEQ ID NO: 885 - DNA, 20 bp, Artificial Sequence
  Synthetic polynucleotide
agccatggtttcagacgaag

SEQ ID NO: 886 - DNA, 26 bp, Artificial Sequence
  Synthetic polynucleotide
ttcctttaatgcttgctttccccacc

SEQ ID NO: 887 - DNA, 18 bp, Artificial Sequence
  Synthetic polynucleotide
tttcccagcaccatcacg

SEQ ID NO: 888 - DNA, 22 bp, Artificial Sequence
  Synthetic polynucleotide
ccatctttccctcaatctccag

SEQ ID NO: 889 - DNA, 25 bp, Artificial Sequence
  Synthetic polynucleotide
cgtcgcttaatcggagccaaagtct

SEQ ID NO: 890 - DNA, 21 bp, Artificial Sequence
  Synthetic polynucleotide
ctgcattgtaggtgtactcgg

SEQ ID NO: 891 - DNA, 21 bp, Artificial Sequence
  Synthetic polynucleotide
tggtcaacgtcttgaaaggag

SEQ ID NO: 892 - DNA, 26 bp, Artificial Sequence
  Synthetic polynucleotide
tgaatgatgaacttcttccccagggc

SEQ ID NO: 893 - DNA, 25 bp, Artificial Sequence
  Synthetic polynucleotide
aaccaattctgctattacaaagacg

SEQ ID NO: 894 - DNA, 20 bp, Artificial Sequence
  Synthetic polynucleotide
ttcgggtagtggaaaaccag

SEQ ID NO: 895 - DNA, 25 bp, Artificial Sequence
  Synthetic polynucleotide
cccctcaacgttagcttcaccaaca

SEQ ID NO: 896 - DNA, 20 bp, Artificial Sequence
  Synthetic polynucleotide
agtagaaatacggctgcacc

SEQ ID NO: 897 - DNA, 20 bp, Artificial Sequence
  Synthetic polynucleotide
atataacagaaccggcccac

SEQ ID NO: 898 - DNA, 23 bp, Artificial Sequence
  Synthetic polynucleotide
catctccttgccagcggtagacg

SEQ ID NO: 899 - DNA, 21 bp, Artificial Sequence
  Synthetic polynucleotide
ccctctaagacccatttcagc

SEQ ID NO: 900 - DNA, 21 bp, Artificial Sequence
  Synthetic polynucleotide
ccctctaagacccatttcagc

SEQ ID NO: 901 - DNA, 24 bp, Artificial Sequence
  Synthetic polynucleotide
tcttgtgaaaccactgcccaacca

SEQ ID NO: 902 - DNA, 21 bp, Artificial Sequence
  Synthetic polynucleotide
attctctgccactggattacc

SEQ ID NO: 903 - DNA, 20 bp, Artificial Sequence
  Synthetic polynucleotide
gcaaagaccaaagagacacg

SEQ ID NO: 904 - DNA, 23 bp, Artificial Sequence
  Synthetic polynucleotide
tcaaagtggatgtcgagggtggc

SEQ ID NO: 905 - DNA, 20 bp, Artificial Sequence
  Synthetic polynucleotide
ggaatgttaaccccgcaaac

SEQ ID NO: 906 - DNA, 22 bp, Artificial Sequence
  Synthetic polynucleotide
ccaggagaaggagtttgagaag

SEQ ID NO: 907 - DNA, 25 bp, Artificial Sequence
  Synthetic polynucleotide
tttgaaagactttgagccacagccc

SEQ ID NO: 908 - DNA, 22 bp, Artificial Sequence
  Synthetic polynucleotide
ggccgaggatgagacatattac

SEQ ID NO: 909 - DNA, 22 bp, Artificial Sequence
  Synthetic polynucleotide
gatgaggacgatgaggactttg

SEQ ID NO: 910 - DNA, 23 bp, Artificial Sequence
  Synthetic polynucleotide
cgaccacttgcggcctgagtatg

SEQ ID NO: 911 - DNA, 20 bp, Artificial Sequence
  Synthetic polynucleotide
tgtgtctttctctggtgctg

SEQ ID NO: 912 - DNA, 18 bp, Artificial Sequence
  Synthetic polynucleotide
gagtatcgagcggaagcg

SEQ ID NO: 913 - DNA, 23 bp, Artificial Sequence
  Synthetic polynucleotide
attagccatgcctccagtagccg

SEQ ID NO: 914 - DNA, 23 bp, Artificial Sequence
  Synthetic polynucleotide
ctcctgtgtcaattatctttggg

SEQ ID NO: 915 - DNA, 22 bp, Artificial Sequence
  Synthetic polynucleotide
gtctctacagccaattcctctg

SEQ ID NO: 916 - DNA, 26 bp, Artificial Sequence
  Synthetic polynucleotide
tggatccgcagtcaatctttccttgg

SEQ ID NO: 917 - DNA, 21 bp, Artificial Sequence
  Synthetic polynucleotide
cctttgctggtctttggtttg

SEQ ID NO: 918 - DNA, 20 bp, Artificial Sequence
  Synthetic polynucleotide
accttctacaatgagctgcg

SEQ ID NO: 919 - DNA, 24 bp, Artificial Sequence
  Synthetic polynucleotide
atctgggtcatcttctcgcggttg

SEQ ID NO: 920 - DNA, 21 bp, Artificial Sequence
  Synthetic polynucleotide
cctggatagcaacgtacatgg

SEQ ID NO: 921 - DNA, 20 bp, Artificial Sequence
  Synthetic polynucleotide
acttgcccagatgttctcag

SEQ ID NO: 922 - DNA, 24 bp, Artificial Sequence
  Synthetic polynucleotide
accaaccgatccaaagtctccagc

SEQ ID NO: 923 - DNA, 22 bp, Artificial Sequence
  Synthetic polynucleotide
gtatccctctagccattcagtg

SEQ ID NO: 924 - DNA, 19 bp, Artificial Sequence
  Synthetic polynucleotide
acatcgctcagacaccatg

SEQ ID NO: 925 - DNA, 25 bp, Artificial Sequence
  Synthetic polynucleotide
aaggtcggagtcaacggatttggtc

SEQ ID NO: 926 - DNA, 22 bp, Artificial Sequence
  Synthetic polynucleotide
tgtagttgaggtcaatgaaggg